European Patent Specification EP 3 775 195 B1, published September 3, 2025. Title: Engineered Decarboxylase Polypeptides and Their uses in Preparing Tyramine and Dopamine. Applicant: Enzymaster (Ningbo) Bio-Engineering Co., Ltd. The sequence listing filed with the application follows.

SEQUENCE LISTING (104 sequences)

SEQ ID NO: 1 - DNA, 1863 bp, Artificial sequence
  Engineered sequence
atgagcaacaccagtttcagcgcaaaagataccgatctgagtgcactgtttatcggtgacaaagcagaaaatggtcagctgtataaggacctgctgggcaaactggttgatgaacatctgggttggcgccagaattatatgccgcaggataaaccgatgatcagcgccgaacagcagaccagcccggaatttcgtggtaccgtgaataatatgaaggacgttctggatgagctgagcagtcgcctgcgtagtcagagcgttccgtggcataatgccggtcgttattggggccacatgaatagcgaaaccctgatgccggcaattctggcctataattatgcaatgctgtggaatggtaacaacgtggcctatgaaagcagcccggcaaccagccagatggaagaagaagttggtctggaatttgccaccctgatgggctataccaatggttggggccatattgttgcagatggtagcctggcaaatctggaaggcctgtggtatgcacgcaatattaagagcctgccgtttgccatgaaagccgttgatccgaccattgttgccggcaaaaccgattgggaactgagtaatatgagcaccaaagaaatcatggacctggttgaagccaatggtgacaaaattgatgagatcaaggccaaaagcgcccgcggcggtaaagatctggataaactgggtaaatggctggttccgcagaccaaacattatagttggctgaaagccgcagatattatcggcattggcctggatcaggttattccggttccggttgatagcaattatcgtatggatatcaacgagctggagaaaattatccgcgaactggcaagtaccgaaaccccgattctgggcgttgtgggcgttgtgggtagtaccgaagaaggtgccgttgatggcattaatgaaattgcagaactgcgtaacaagctggtgaaagaaggtatctatttctacttccacatcgacgccgcctatggtggctatggtcgcgcaattctgctggatgaagataataagctgatcccgtataaggaccttcagagtaaattcgccgaatataacgtgttcaccgaagaagaaaacctggtgagtgaacatacctataacgcctatgccgcatttccggaagccgaaagtgttaccattgatccgcataaaatgggctatatcccgtatagtgcaggcggcattgccattcaggatattcgcatgcgtgatgttatcagctatttcgcaacctatgtgttcgaaaagggcgcagatattccggcactgctgggtgcttatattctggaaggcagtaaagcaggcgcaaccgcagccagtgtttgggcagcacataaaaccctgccgctgaatgttaccggttatggtaaactggttggtgcaagcattgaaggcgcccgccgtttttataattttctgagcggcctggaattcaaggtgggcgataaaaccattgaagttcatccgctgaccgatccggattttaatatggttgattacgtgttccaggagaagggcaataataatctggtggaaatgaacgagctgaaccatgaattttacaaccaggcaagctacgttaccggtagcatctatggcaatgaatatctgaccagccataccgatttcgcaattccggattatggtaatagcccgtttaagtttgtgaacaacctgggcgtgaccgaagaaggctggaaagaagcaggtaaagtgaccgttctgcgcgccgctgtgatgacaccttatatgaataaggcagagaacttcgactacttcgccccgaaaattaagcaggccatgcaggaaaaactggaagccatctatgaagatcgtaag

SEQ ID NO: 2 - protein, 621 aa, Streptococcus thermophilus
MSNTSFSAKDTDLSALFIGDKAENGQLYKDLLGKLVDEHLGWRQNYMPQDKPMISAEQQTSPEFRGTVNNMKDVLDELSSRLRSQSVPWHNAGRYWGHMNSETLMPAILAYNYAMLWNGNNVAYESSPATSQMEEEVGLEFATLMGYTNGWGHIVADGSLANLEGLWYARNIKSLPFAMKAVDPTIVAGKTDWELSNMSTKEIMDLVEANGDKIDEIKAKSARGGKDLDKLGKWLVPQTKHYSWLKAADIIGIGLDQVIPVPVDSNYRMDINELEKIIRELASTETPILGVVGVVGSTEEGAVDGINEIAELRNKLVKEGIYFYFHIDAAYGGYGRAILLDEDNKLIPYKDLQSKFAEYNVFTEEENLVSEHTYNAYAAFPEAESVTIDPHKMGYIPYSAGGIAIQDIRMRDVISYFATYVFEKGADIPALLGAYILEGSKAGATAASVWAAHKTLPLNVTGYGKLVGASIEGARRFYNFLSGLEFKVGDKTIEVHPLTDPDFNMVDYVFQEKGNNNLVEMNELNHEFYNQASYVTGSIYGNEYLTSHTDFAIPDYGNSPFKFVNNLGVTEEGWKEAGKVTVLRAAVMTPYMNKAENFDYFAPKIKQAMQEKLEAIYEDRK

SEQ ID NO: 3 - DNA, 1863 bp, Artificial sequence
  Engineered sequence
atgagcaacaccagtttcagcgcaaaagataccgatctgagtgcactgtttatcggtgacaaagcagaaaatggtcagctgtataaggacctgctgggcaaactggttgatgaacatctgggttggcgccagaattatatgccgcaggataaaccgatgatcagcgccgaacagcagaccagcccggaatttcgtggtaccgtgaataatatgaaggacgttctggatgagctgagcagtcgcctgcgtagtcagagcgttccgtggcataatgccggtcgttattggggccacatgaatagcgaaaccctgatgccggcaattctggcctataattatgcaatgctgtggaatggtaacaacgtggcctatgaaagcagcccggcaaccagccagatggaagaagaagttggtctggaatttgccaccctgatgggctataccaatggttggggccatattgttgcagatggtagcctggcaaatctggaaggcctgtggtatgcacgcaatattaagagcctgccgtttgccatgaaagccgttgatccgaccattgttgccggcaaaaccgattgggaactgagtaatatgagcaccaaagaaatcatggacctggttgaagccaatggtgacaaaattgatgagatcaaggccaaaagcgcccgcggcggtaaagatctggataaactgggtaaatggctggttccgcagaccaaacattatagttggctgaaagccgcagatattatcggcattggcctggatcaggttattccggttccggttgatagcaattatcgtatggatatcaacgagctggagaaaattatccgcgaactggcaagtaccgaaaccccgattctgggcgttgtgggcgttgtgggtagtaccgaagaaggtgccgttgatggcattaatgaaattgcagaactgcgtaacaagctggtgaaagaaggtatctatttctacttccacatcgacgccgcctatggtggctatggtcgcgcaattctgctggatgaagataataagctgatcccgtataaggaccttcagagtaaattcgccgaatataacgtgttcaccgaagaagaaaacctggtgagtgaacatacctataacgcctatgccgcatttccggaagccgaaagtgttaccattgatccgcataaaatgggctatatcccgtatagtgcaggcggcattgccattcaggatattcgcatgcgtgatgttatcagctatttcgcaacctatgtgttcgaaaagggcgcagatattccggcactgctgggtgcttatattctggaaggcagtaaagcaggcgcaaccgcagccagtgtttgggcagcacataaaaccctgccgctgaatgttaccggttatggtaaactggttggtgcaagcattgaaggcgcccgccgtttttataattttctgagcggcctggaattcaaggtgggcgataaaaccattgaagttcatccgctgaccgatccggattttaatatggttgattacgtgttccaggagaagggcaataatgatctggtggaaatgaacgagctgaaccatgaattttacaaccaggcaagctacgttaccggtagcatctatggcaatgaatatctgaccagccataccgatttcgcaattccggattatggtaatagcccgtttaagtttgtgaacaacctgggcgtgaccgaagaaggctggaaagaagcaggtaaagtgaccgttctgcgcgccgctgtgatgacaccttatatgaataaggcagagaacttcgactacttcgccccgaaaattaagcaggccatgcaggaaaaactggaagccatctatgaagatcgtaag

SEQ ID NO: 4 - protein, 621 aa, Artificial sequence
  Engineered sequence
MSNTSFSAKDTDLSALFIGDKAENGQLYKDLLGKLVDEHLGWRQNYMPQDKPMISAEQQTSPEFRGTVNNMKDVLDELSSRLRSQSVPWHNAGRYWGHMNSETLMPAILAYNYAMLWNGNNVAYESSPATSQMEEEVGLEFATLMGYTNGWGHIVADGSLANLEGLWYARNIKSLPFAMKAVDPTIVAGKTDWELSNMSTKEIMDLVEANGDKIDEIKAKSARGGKDLDKLGKWLVPQTKHYSWLKAADIIGIGLDQVIPVPVDSNYRMDINELEKIIRELASTETPILGVVGVVGSTEEGAVDGINEIAELRNKLVKEGIYFYFHIDAAYGGYGRAILLDEDNKLIPYKDLQSKFAEYNVFTEEENLVSEHTYNAYAAFPEAESVTIDPHKMGYIPYSAGGIAIQDIRMRDVISYFATYVFEKGADIPALLGAYILEGSKAGATAASVWAAHKTLPLNVTGYGKLVGASIEGARRFYNFLSGLEFKVGDKTIEVHPLTDPDFNMVDYVFQEKGNNDLVEMNELNHEFYNQASYVTGSIYGNEYLTSHTDFAIPDYGNSPFKFVNNLGVTEEGWKEAGKVTVLRAAVMTPYMNKAENFDYFAPKIKQAMQEKLEAIYEDRK

SEQ ID NO: 5 - DNA, 1863 bp, Artificial sequence
  Engineered sequence
atgagcaacaccagtttcagcgcaaaagataccgatctgagtgcactgtttatcggtgacaaagcagaaaatggtcagctgtataaggacctgctgggcaaactggttgatgaacatctgggttggcgccagaattatatgccgcaggataaaccgatgatcagcgccgaacagcagaccagcccggaatttcgtggtaccgtgaataatatgaaggacgttctggatgagctgagcagtcgcctgcgtagtcagagcgttccgtggcataatgccggtcgttattggggccacatgaatagcgaaaccctgatgccggcaattctggcctataattatgcaatgctgtggaatggtaacaacgtggcctatgaaagcagcccggcaaccagccagatggaagaagaagttggtctggaatttgccaccctgatgggctataccaatggttggggccatattgttgcagatggtagcctggcaaatctggaaggcctgtggtatgcacgcaatattaagagcctgccgtttgccatgaaagccgttgatccgaccattgttgccggcaaaaccgattgggaactgagtaatatgagcaccaaagaaatcatggacctggttgaagccctgggtgacaaaattgatgagatcaaggccaaaagcgcccgcggcggtaaagatctggataaactgggtaaatggctggttccgcagaccaaacattatagttggctgaaagccgcagatattatcggcattggcctggatcaggttattccggttccggttgatagcaattatcgtatggatatcaacgagctggagaaaattatccgcgaactggcaagtaccgaaaccccgattctgggcgttgtgggcgttgtgggtagtaccgaagaaggtgccgttgatggcattaatgaaattgcagaactgcgtaacaagctggtgaaagaaggtatctatttctacttccacatcgacgccgcctatggtggctatggtcgcgcaattctgctggatgaagataataagctgatcccgtataaggaccttcagagtaaattcgccgaatataacgtgttcaccgaagaagaaaacctggtgagtgaacatacctataacgcctatgccgcatttccggaagccgaaagtgttaccattgatccgcataaaatgggctatatcccgtatagtgcaggcggcattgccattcaggatattcgcatgcgtgatgttatcagctatttcgcaacctatgtgttcgaaaagggcgcagatattccggcactgctgggtgcttatattctggaaggcagtaaagcaggcgcaaccgcagccagtgtttgggcagcacataaaaccctgccgctgaatgttaccggttatggtaaactggttggtgcaagcattgaaggcgcccgccgtttttataattttctgagcggcctggaattcaaggtgggcgataaaaccattgaagttcatccgctgaccgatccggattttaatatggttgattacgtgttccaggagaagggcaataataatctggtggaaatgaacgagctgaaccatgaattttacaaccaggcaagctacgttaccggtagcatctatggcaatgaatatctgaccagccataccgatttcgcaattccggattatggtaatagcccgtttaagtttgtgaacaacctgggcgtgaccgaagaaggctggaaagaagcaggtaaagtgaccgttctgcgcgccgctgtgatgacaccttatatgaataaggcagagaacttcgactacttcgccccgaaaattaagcaggccatgcaggaaaaactggaagccatctatgaagatcgtaag

SEQ ID NO: 6 - protein, 621 aa, Artificial sequence
  Engineered sequence
MSNTSFSAKDTDLSALFIGDKAENGQLYKDLLGKLVDEHLGWRQNYMPQDKPMISAEQQTSPEFRGTVNNMKDVLDELSSRLRSQSVPWHNAGRYWGHMNSETLMPAILAYNYAMLWNGNNVAYESSPATSQMEEEVGLEFATLMGYTNGWGHIVADGSLANLEGLWYARNIKSLPFAMKAVDPTIVAGKTDWELSNMSTKEIMDLVEALGDKIDEIKAKSARGGKDLDKLGKWLVPQTKHYSWLKAADIIGIGLDQVIPVPVDSNYRMDINELEKIIRELASTETPILGVVGVVGSTEEGAVDGINEIAELRNKLVKEGIYFYFHIDAAYGGYGRAILLDEDNKLIPYKDLQSKFAEYNVFTEEENLVSEHTYNAYAAFPEAESVTIDPHKMGYIPYSAGGIAIQDIRMRDVISYFATYVFEKGADIPALLGAYILEGSKAGATAASVWAAHKTLPLNVTGYGKLVGASIEGARRFYNFLSGLEFKVGDKTIEVHPLTDPDFNMVDYVFQEKGNNNLVEMNELNHEFYNQASYVTGSIYGNEYLTSHTDFAIPDYGNSPFKFVNNLGVTEEGWKEAGKVTVLRAAVMTPYMNKAENFDYFAPKIKQAMQEKLEAIYEDRK

SEQ ID NO: 7 - DNA, 1863 bp, Artificial sequence
  Engineered sequence
atgagcaacaccagtttcagcgcaaaagataccgatctgagtgcactgtttatcggtgacaaagcagaaaatggtcagctgtataaggacctgctgggcaaactggttgatgaacatctgggttggcgccagaattatatgccgcaggataaaccgatgatcagcgccgaacagcagaccagcccggaatttcgtggtaccgtgaataatatgaaggacgttctggatgagctgagcagtcgcctgcgtagtcagagcgttccgtggcataatgccggtcgttattggggccacatgaatagcgaaaccctgatgccggcaattctggcctataattatgcaatgctgtggaatggtaacaacgtggcctatgaaagcagcccggcaaccagccagatggaagaagaagttggtctggaatttgccaccctgatgggctataccaatggttggggccatattgttgcagatggtagcctggcaaatctggaaggcctgtggtatgcacgcaatattaagagcctgccgtttgccatgaaagaagttgatccgaccattgttgccggcaaaaccgattgggaactgagtaatatgagcaccaaagaaatcatggacctggttgaagccaatggtgacaaaattgatgagatcaaggccaaaagcgcccgcggcggtaaagatctggataaactgggtaaatggctggttccgcagaccaaacattatagttggctgaaagccgcagatattatcggcattggcctggatcaggttattccggttccggttgatagcaattatcgtatggatatcaacgagctggagaaaattatccgcgaactggcaagtaccgaaaccccgattctgggcgttgtgggcgttgtgggtagtaccgaagaaggtgccgttgatggcattaatgaaattgcagaactgcgtaacaagctggtgaaagaaggtatctatttctacttccacatcgacgccgcctatggtggctatggtcgcgcaattctgctggatgaagataataagctgatcccgtataaggaccttcagagtaaattcgccgaatataacgtgttcaccgaagaagaaaacctggtgagtgaacatacctataacgcctatgccgcatttccggaagccgaaagtgttaccattgatccgcataaaatgggctatatcccgtatagtgcaggcggcattgccattcaggatattcgcatgcgtgatgttatcagctatttcgcaacctatgtgttcgaaaagggcgcagatattccggcactgctgggtgcttatattctggaaggcagtaaagcaggcgcaaccgcagccagtgtttgggcagcacataaaaccctgccgctgaatgttaccggttatggtaaactggttggtgcaagcattgaaggcgcccgccgtttttataattttctgagcggcctggaattcaaggtgggcgataaaaccattgaagttcatccgctgaccgatccggattttaatatggttgattacgtgttccaggagaagggcaataataatctggtggaaatgaacgagctgaaccatgaattttacaaccaggcaagctacgttaccggtagcatctatggcaatgaatatctgaccagccataccgatttcgcaattccggattatggtaatagcccgtttaagtttgtgaacaacctgggcgtgaccgaagaaggctggaaagaagcaggtaaagtgaccgttctgcgcgccgctgtgatgacaccttatatgaataaggcagagaacttcgactacttcgccccgaaaattaagcaggccatgcaggaaaaactggaagccatctatgaagatcgtaag

SEQ ID NO: 8 - protein, 621 aa, Artificial sequence
  Engineered sequence
MSNTSFSAKDTDLSALFIGDKAENGQLYKDLLGKLVDEHLGWRQNYMPQDKPMISAEQQTSPEFRGTVNNMKDVLDELSSRLRSQSVPWHNAGRYWGHMNSETLMPAILAYNYAMLWNGNNVAYESSPATSQMEEEVGLEFATLMGYTNGWGHIVADGSLANLEGLWYARNIKSLPFAMKEVDPTIVAGKTDWELSNMSTKEIMDLVEANGDKIDEIKAKSARGGKDLDKLGKWLVPQTKHYSWLKAADIIGIGLDQVIPVPVDSNYRMDINELEKIIRELASTETPILGVVGVVGSTEEGAVDGINEIAELRNKLVKEGIYFYFHIDAAYGGYGRAILLDEDNKLIPYKDLQSKFAEYNVFTEEENLVSEHTYNAYAAFPEAESVTIDPHKMGYIPYSAGGIAIQDIRMRDVISYFATYVFEKGADIPALLGAYILEGSKAGATAASVWAAHKTLPLNVTGYGKLVGASIEGARRFYNFLSGLEFKVGDKTIEVHPLTDPDFNMVDYVFQEKGNNNLVEMNELNHEFYNQASYVTGSIYGNEYLTSHTDFAIPDYGNSPFKFVNNLGVTEEGWKEAGKVTVLRAAVMTPYMNKAENFDYFAPKIKQAMQEKLEAIYEDRK

SEQ ID NO: 9 - DNA, 1863 bp, Artificial sequence
  Engineered sequence
atgagcaacaccagtttcagcgcaaaagataccgatctgagtgcactgtttatcggtgacaaagcagaaaatggtcagctgtataaggacctgctgggcaaactggttgatgaacatctgggttggcgccagaattatatgccgcaggataaaccgatgatcagcgccgaacagcagaccagcccggaatttcgtggtaccgtgaataatatgaaggacgttctggatgagctgagcagtcgcctgcgtagtcagagcgttccgtggcataatgccggtcgttattggggccacatgaatagcgaaaccctgatgccggcaattctggcctataattatgcaatgctgtggaatggtaacaacgtggcctatgaaagcagcccggcaaccagccagatggaagaagaagttggtctggaatttgccaccctgatgggctataccaatggttggggccatattgttgcagatggtagcctggcaaatctggaaggcctgtggtatgcacgcaatattaagagcctgccgtttgccatgaaagccgttgatccgaccattgttgccggcaaaaccgattgggaactgagtaatatgagcaccaaagaaatcatggacctggttgaagccaatggtgacaaaattgatgagatcaaggccaaaagcgcccgcggcggtaaagatctggataaactgggtaaatggctggttccgcagaccaaacattatagttggctgaaagccgcagatattatcggcattggcctggatcaggttattccggttccggttgatagcaattatcgtatggatatcaacgagctggagaaaattatccgcgaactggcaagtaccgaaaccccgattctgggcgttgtgggcgttgtgggtagtaccgaagaaggtgccgttgatggcattaatgaaattgcagaactgcgtaacaagctggaaaaagaaggtatctatttctacttccacatcgacgccgcctatggtggctatggtcgcgcaattctgctggatgaagataataagctgatcccgtataaggaccttcagagtaaattcgccgaatataacgtgttcaccgaagaagaaaacctggtgagtgaacatacctataacgcctatgccgcatttccggaagccgaaagtgttaccattgatccgcataaaatgggctatatcccgtatagtgcaggcggcattgccattcaggatattcgcatgcgtgatgttatcagctatttcgcaacctatgtgttcgaaaagggcgcagatattccggcactgctgggtgcttatattctggaaggcagtaaagcaggcgcaaccgcagccagtgtttgggcagcacataaaaccctgccgctgaatgttaccggttatggtaaactggttggtgcaagcattgaaggcgcccgccgtttttataattttctgagcggcctggaattcaaggtgggcgataaaaccattgaagttcatccgctgaccgatccggattttaatatggttgattacgtgttccaggagaagggcaataataatctggtggaaatgaacgagctgaaccatgaattttacaaccaggcaagctacgttaccggtagcatctatggcaatgaatatctgaccagccataccgatttcgcaattccggattatggtaatagcccgtttaagtttgtgaacaacctgggcgtgaccgaagaaggctggaaagaagcaggtaaagtgaccgttctgcgcgccgctgtgatgacaccttatatgaataaggcagagaacttcgactacttcgccccgaaaattaagcaggccatgcaggaaaaactggaagccatctatgaagatcgtaag

SEQ ID NO: 10 - protein, 621 aa, Artificial sequence
  Engineered sequence
MSNTSFSAKDTDLSALFIGDKAENGQLYKDLLGKLVDEHLGWRQNYMPQDKPMISAEQQTSPEFRGTVNNMKDVLDELSSRLRSQSVPWHNAGRYWGHMNSETLMPAILAYNYAMLWNGNNVAYESSPATSQMEEEVGLEFATLMGYTNGWGHIVADGSLANLEGLWYARNIKSLPFAMKAVDPTIVAGKTDWELSNMSTKEIMDLVEANGDKIDEIKAKSARGGKDLDKLGKWLVPQTKHYSWLKAADIIGIGLDQVIPVPVDSNYRMDINELEKIIRELASTETPILGVVGVVGSTEEGAVDGINEIAELRNKLEKEGIYFYFHIDAAYGGYGRAILLDEDNKLIPYKDLQSKFAEYNVFTEEENLVSEHTYNAYAAFPEAESVTIDPHKMGYIPYSAGGIAIQDIRMRDVISYFATYVFEKGADIPALLGAYILEGSKAGATAASVWAAHKTLPLNVTGYGKLVGASIEGARRFYNFLSGLEFKVGDKTIEVHPLTDPDFNMVDYVFQEKGNNNLVEMNELNHEFYNQASYVTGSIYGNEYLTSHTDFAIPDYGNSPFKFVNNLGVTEEGWKEAGKVTVLRAAVMTPYMNKAENFDYFAPKIKQAMQEKLEAIYEDRK

SEQ ID NO: 11 - DNA, 1863 bp, Artificial sequence
  Engineered sequence
atgagcaacaccagtttcagcgcaaaagataccgatctgagtgcactgtttatcggtgacaaagcagaaaatggtcagctgtataaggacctgctgggcaaactggttgatgaacatctgggttggcgccagaattatatgccgcaggataaaccgatgatcagcgccgaacagcagaccagcccggaatttcgtggtaccgtgaataatatgaaggacgttctggatgagctgagcagtcgcctgcgtagtcagagcgttccgtggcataatgccggtcgttattggggccacatgaatagcgaaaccctgatgccggcaattctggcctataattatgcaatgctgtggaatggtaacaacgtggcctatgaaagcagcccggcaaccagccagatggaagaagaagttggtctggaatttgccaccctgatgggctataccaatggttggggccatattgttgcagatggtagcctggcaaatctggaaggcctgtggtatgcacgcaatattaagagcctgccgtttgccatgaaagccgttgatccgaccattgttgccggcaaaaccgattgggaactgagtaatatgagcaccaaagaaatcatggacctggttgaagccaatggtgacaaaattgatgagatcaaggccaaaagcgcccgcggcggtaaagatctggataaactgggtaaatggctggttccgcagaccaaacattatagttggctgaaagccgcagatattatcggcattggcctggatcaggttattccggttccggttgatagcaattatcgtatggatatcaacgagctggagaaaattatccgcgaactggcaagtaccgaaaccccgattctgggcgttgtgggcgttgtgggtagtaccgaagaaggtgccgttgatggcattaatgaaattgcagaactgcgtaacaagctggtgaaagaaggtatctatttctacttccacatcgacgccgcctatggtggctatggtcgcgcaattctgctggatgaagataataagctgatcccgtataaggaccttcagagtaaattcgccgaatataacgtgttcaccgaagaagaaaacctggtgagtgaacatacctataacgcctatgccgcatttccggaagccgaaagtgttaccattgatccgcataaaatgggctatatcccgtatagtgcaggcggcattgccattcaggatattcgcatgcgtgatgttatcagctatttcgcaacctatgtgttcgaaaagggcgcagatattccggcactgctgggtgcttatattctggaaggcagtaaagcaggcgcaaccgcagccagtgtttgggcagcacataaaaccctgccgctgaatgttaccggttatggtaaactggttggtgcaagcattgaaggcgcccgccgtttttataattttctgagcggcctggaattcaaggtgggcgataaaaccattgaagttcatccgctgaccgatccggattttaatatggttgattacgtgttccaggagaagggcaataataatctggtggaaatgaacgagctgaaccatgaattttacaaccaggcaagctacgttaccggtagcatctatggcaatgaatatctgaccagccataccgatttcgcaattccggattatggtaatagcccgtttaagtttgtgaacaacctgggcgtgaccgaagaaggctggaaaaaagcaggtaaagtgaccgttctgcgcgccgctgtgatgacaccttatatgaataaggcagagaacttcgactacttcgccccgaaaattaagcaggccatgcaggaaaaactggaagccatctatgaagatcgtaag

SEQ ID NO: 12 - protein, 621 aa, Artificial sequence
  Engineered sequence
MSNTSFSAKDTDLSALFIGDKAENGQLYKDLLGKLVDEHLGWRQNYMPQDKPMISAEQQTSPEFRGTVNNMKDVLDELSSRLRSQSVPWHNAGRYWGHMNSETLMPAILAYNYAMLWNGNNVAYESSPATSQMEEEVGLEFATLMGYTNGWGHIVADGSLANLEGLWYARNIKSLPFAMKAVDPTIVAGKTDWELSNMSTKEIMDLVEANGDKIDEIKAKSARGGKDLDKLGKWLVPQTKHYSWLKAADIIGIGLDQVIPVPVDSNYRMDINELEKIIRELASTETPILGVVGVVGSTEEGAVDGINEIAELRNKLVKEGIYFYFHIDAAYGGYGRAILLDEDNKLIPYKDLQSKFAEYNVFTEEENLVSEHTYNAYAAFPEAESVTIDPHKMGYIPYSAGGIAIQDIRMRDVISYFATYVFEKGADIPALLGAYILEGSKAGATAASVWAAHKTLPLNVTGYGKLVGASIEGARRFYNFLSGLEFKVGDKTIEVHPLTDPDFNMVDYVFQEKGNNNLVEMNELNHEFYNQASYVTGSIYGNEYLTSHTDFAIPDYGNSPFKFVNNLGVTEEGWKKAGKVTVLRAAVMTPYMNKAENFDYFAPKIKQAMQEKLEAIYEDRK

SEQ ID NO: 13 - DNA, 1863 bp, Artificial sequence
  Engineered sequence
atgagcaacaccagtttcagcgcaaaagataccgatctgagtgcactgtttatcggtgacaaagcagaaaatggtcagctgtataaggacctgctgggcaaactggttgatgaacatctgggttggcgccagaattatatgccgcaggataaaccgatgatcagcgccgaacagcagaccagcccggaatttcgtggtaccgtgaataatatgaaggacgttctggatgagctgagcagtcgcctgcgtagtcagagcgttccgtggcataatgccggtcgttattggggccacatgaatagcgaaaccctgatgccggcaattctggcctataattatgcaatgctgtggaatggtaacaacgtggcctatgaaagcagcccggcaaccagccagatggaagaagaagttggtctggaatttgccaccctgatgggctataccaatggttggggccatattgttgcagatggtagcctggcaaatctggaaggcctgtggtatgcacgcaatattaagagcctgccgtttgccatgaaagccgttgatccgaccattgttgccggcaaaaccgattgggaactgagtaatatgagcaccaaagaaatcatggacctggttgaagccaatggtgacaaaattgatgagatcaaggccaaaagcgcccgcggcggtaaagatctggataaactgggtaaatggctggttccgcagaccaaacattatagttggctgaaagccgcagatattatcggcattggcctggatcaggttattccggttccggttgatagcaattatcgtatggatatcaacgagctggagaaaattatccgcgaactggcaagtaccgaaaccccgattctgggcgttgtgggcgttgtgggtagtaccgaagaaggtgccgttgatggcattaatgaaattgcagaactgcgtaacaagctggtgaaagaaggtatctatttctacttccacatcgacgccgcctatggtggctatggtcgcgcaattctgctggatgaagataataagctgatcccgtataaggaccttcagagtaaattcgccgaatataacgtgttcaccgaagaagaaaacctggtgagtgaacatacctataacgcctatgccgcatttccggaagccgaaagtgttaccattgatccgcataaaatgggctatatcccgtatagtgcaggcggcattgccattcaggatattcgcatgcgtgatgttatcagctatttcgcaacctatgtgttcgaaaagggcgcagatattccggcactgctgggtgcttatattctggaaggcagtaaagcaggcgcaaccgcagccagtgtttgggcagcacataaaaccctgccgctgaatgttaccggttatggtaaactgctgggtgcaagcattgaaggcgcccgccgtttttataattttctgagcggcctggaattcaaggtgggcgataaaaccattgaagttcatccgctgaccgatccggattttaatatggttgattacgtgttccaggagaagggcaataataatctggtggaaatgaacgagctgaaccatgaattttacaaccaggcaagctacgttaccggtagcatctatggcaatgaatatctgaccagccataccgatttcgcaattccggattatggtaatagcccgtttaagtttgtgaacaacctgggcgtgaccgaagaaggctggaaagaagcaggtaaagtgaccgttctgcgcgccgctgtgatgacaccttatatgaataaggcagagaacttcgactacttcgccccgaaaattaagcaggccatgcaggaaaaactggaagccatctatgaagatcgtaag

SEQ ID NO: 14 - protein, 621 aa, Artificial sequence
  Engineered sequence
MSNTSFSAKDTDLSALFIGDKAENGQLYKDLLGKLVDEHLGWRQNYMPQDKPMISAEQQTSPEFRGTVNNMKDVLDELSSRLRSQSVPWHNAGRYWGHMNSETLMPAILAYNYAMLWNGNNVAYESSPATSQMEEEVGLEFATLMGYTNGWGHIVADGSLANLEGLWYARNIKSLPFAMKAVDPTIVAGKTDWELSNMSTKEIMDLVEANGDKIDEIKAKSARGGKDLDKLGKWLVPQTKHYSWLKAADIIGIGLDQVIPVPVDSNYRMDINELEKIIRELASTETPILGVVGVVGSTEEGAVDGINEIAELRNKLVKEGIYFYFHIDAAYGGYGRAILLDEDNKLIPYKDLQSKFAEYNVFTEEENLVSEHTYNAYAAFPEAESVTIDPHKMGYIPYSAGGIAIQDIRMRDVISYFATYVFEKGADIPALLGAYILEGSKAGATAASVWAAHKTLPLNVTGYGKLLGASIEGARRFYNFLSGLEFKVGDKTIEVHPLTDPDFNMVDYVFQEKGNNNLVEMNELNHEFYNQASYVTGSIYGNEYLTSHTDFAIPDYGNSPFKFVNNLGVTEEGWKEAGKVTVLRAAVMTPYMNKAENFDYFAPKIKQAMQEKLEAIYEDRK

SEQ ID NO: 15 - DNA, 1863 bp, Artificial sequence
  Engineered sequence
atgagcaacaccagtttcagcgcaaaagataccgatctgagtgcactgtttatcggtgacaaagcagaaaatggtcagctgtataaggacctgctgggcaaactggttgatgaacatctgggttggcgccagaattatatgccgcaggataaaccgatgatcagcgccgaacagcagaccagcccggaatttcgtggtaccgtgaataatatgaaggacgttctggatgagctgagcagtcgcctgcgtagtcagagcgttccgtggcataatgccggtcgttattggggccacatgaatagcgaaaccctgatgccggcaattctggcctataattatgcaatgctgtggaatggtaacaacgtggcctatgaaagcagcccggcaaccagccagatggaagaagaagttggtctggaatttgccaccctgatgggctataccaatggttggggccatattgttgcagatggtagcctggcaaatctggaaggcctgtggtatgcacgcaatattaagagcctgccgtttgccatgaaagccgttgatccgaccattgttgccggcaaaaccgattgggaactgagtaatatgagcaccaaagaaatcatggacctggttgaagccaatggtgacaaaattgatgagatcaaggccaaaagcgcccgcggcggtaaagatctggataaactgggtaaatggctggttccgcagaccaaacattatagttggctgaaagccgcagatattatcggcattggcctggatcaggttattccggttccggttgatagcaattatcgtatggatatcaacgagctggagaaaattatccgcgaactggcaagtaccgaaaccccgattctgggcgttgtgggcgttgtgggtagtaccgaagaaggtgccgttgatggcattaatgaaattgcagaactgcgtaacaagctggtgaaagaaggtatctatttctacttccacatcgacgccgcctatggtggctatggtcgcgcaattctgctggatgaagataataagctgatcccgtataaggaccttcagagtaaattcgccgaatataacgtgttcaccgaagaagaaaacctggtgagtgaacatacctataacgcctatgccgcactgccggaagccgaaagtgttaccattgatccgcataaaatgggctatatcccgtatagtgcaggcggcattgccattcaggatattcgcatgcgtgatgttatcagctatttcgcaacctatgtgttcgaaaagggcgcagatattccggcactgctgggtgcttatattctggaaggcagtaaagcaggcgcaaccgcagccagtgtttgggcagcacataaaaccctgccgctgaatgttaccggttatggtaaactggttggtgcaagcattgaaggcgcccgccgtttttataattttctgagcggcctggaattcaaggtgggcgataaaaccattgaagttcatccgctgaccgatccggattttaatatggttgattacgtgttccaggagaagggcaataataatctggtggaaatgaacgagctgaaccatgaattttacaaccaggcaagctacgttaccggtagcatctatggcaatgaatatctgaccagccataccgatttcgcaattccggattatggtaatagcccgtttaagtttgtgaacaacctgggcgtgaccgaagaaggctggaaagaagcaggtaaagtgaccgttctgcgcgccgctgtgatgacaccttatatgaataaggcagagaacttcgactacttcgccccgaaaattaagcaggccatgcaggaaaaactggaagccatctatgaagatcgtaag

SEQ ID NO: 16 - protein, 621 aa, Artificial sequence
  Engineered sequence
MSNTSFSAKDTDLSALFIGDKAENGQLYKDLLGKLVDEHLGWRQNYMPQDKPMISAEQQTSPEFRGTVNNMKDVLDELSSRLRSQSVPWHNAGRYWGHMNSETLMPAILAYNYAMLWNGNNVAYESSPATSQMEEEVGLEFATLMGYTNGWGHIVADGSLANLEGLWYARNIKSLPFAMKAVDPTIVAGKTDWELSNMSTKEIMDLVEANGDKIDEIKAKSARGGKDLDKLGKWLVPQTKHYSWLKAADIIGIGLDQVIPVPVDSNYRMDINELEKIIRELASTETPILGVVGVVGSTEEGAVDGINEIAELRNKLVKEGIYFYFHIDAAYGGYGRAILLDEDNKLIPYKDLQSKFAEYNVFTEEENLVSEHTYNAYAALPEAESVTIDPHKMGYIPYSAGGIAIQDIRMRDVISYFATYVFEKGADIPALLGAYILEGSKAGATAASVWAAHKTLPLNVTGYGKLVGASIEGARRFYNFLSGLEFKVGDKTIEVHPLTDPDFNMVDYVFQEKGNNNLVEMNELNHEFYNQASYVTGSIYGNEYLTSHTDFAIPDYGNSPFKFVNNLGVTEEGWKEAGKVTVLRAAVMTPYMNKAENFDYFAPKIKQAMQEKLEAIYEDRK

SEQ ID NO: 17 - DNA, 1863 bp, Artificial sequence
  Engineered sequence
atgagcaacaccagtttcagcgcaaaagataccgatctgagtgcactgtttatcggtgacaaagcagaaaatggtcagctgtataaggacctgctgggcaaactggttgatgaacatctgggttggcgccagaattatatgccgcaggataaaccgatgatcagcgccgaacagcagaccagcccggaatttcgtggtaccgtgaataatatgaaggacgttctggatgagctgagcagtcgcctgcgtagtcagagcgttccgtggcataatgccggtcgttattggggccacatgaatagcgaaaccctgatgccggcaattctggcctataattatgcaatgctgtggaatggtaacaacgtggcctatgaaagcagcccggcaaccagccagatggaagaagaagttggtctggaatttgccaccctgatgggctataccaatggttggggccatattgttgcagatggtagcctggcaaatctggaaggcctgtggtatgcacgcaatattaagagcctgccgtttgccatgaaagccgttgatccgaccattgttgccggcaaaaccgattgggaactgagtaatatgagcaccaaagaaatcatggacctggttgaagccaatggtgacaaaattgatgagatcaaggccaaaagcgcccgcggcggtaaagatctggataaactgggtaaatggctggttccgcagaccaaacattatagttggctgaaagccgcagatattatcggcattggcctggatcaggttattccggttccggttgatagcaattatcgtatggatatcaacgagctggagaaaattatccgcgaactggcaagtaccgaaaccccgattctgggcgttgtgggcgttgtgggtagtaccgaagaaggtgccgttgatggcattaatgaaattgcagaactgcgtaacaagctggtgaaagaaggtatctatttctacttccacatcgacgccgcctatggtggctatggtcgcgcaattctgctggatgaagataataagctgatcccgtataaggaccttcagagtaaattcgccgaatataacgtgttcaccgaagaagaaaacctggtgagtgaacatacctataacgcctatgccgcatttccggaagccgaaagtgttaccattgatccgcataaaatgggctatatcccgtatagtgcaggcggcattgccattcaggatattcgcatgcgtgatgttatcagctatttcgcaacctatgtgttcgaaaagggcgcagatattccggcactgctgggtgcttatattctggaaggcagtaaagcaggcgcaaccgcagccagtgtttgggcagcacataaaaccctgccgctgaatgttaccggttatggtaaactggttggtgcaagcattgaaggcgcccgccgtttttataattttctgagcggcctggaattcaaggtgggcgataaaaccattgaagttcatccgctgaccgatccggattttaatatggttgattacgtgttccaggagaagggcaataataatctggtggaaatgaacgagctgaaccatgaattttacgatcaggcaagctacgttaccggtagcatctatggcaatgaatatctgaccagccataccgatttcgcaattccggattatggtaatagcccgtttaagtttgtgaacaacctgggcgtgaccgaagaaggctggaaagaagcaggtaaagtgaccgttctgcgcgccgctgtgatgacaccttatatgaataaggcagagaacttcgactacttcgccccgaaaattaagcaggccatgcaggaaaaactggaagccatctatgaagatcgtaag

SEQ ID NO: 18 - protein, 621 aa, Artificial sequence
  Engineered sequence
MSNTSFSAKDTDLSALFIGDKAENGQLYKDLLGKLVDEHLGWRQNYMPQDKPMISAEQQTSPEFRGTVNNMKDVLDELSSRLRSQSVPWHNAGRYWGHMNSETLMPAILAYNYAMLWNGNNVAYESSPATSQMEEEVGLEFATLMGYTNGWGHIVADGSLANLEGLWYARNIKSLPFAMKAVDPTIVAGKTDWELSNMSTKEIMDLVEANGDKIDEIKAKSARGGKDLDKLGKWLVPQTKHYSWLKAADIIGIGLDQVIPVPVDSNYRMDINELEKIIRELASTETPILGVVGVVGSTEEGAVDGINEIAELRNKLVKEGIYFYFHIDAAYGGYGRAILLDEDNKLIPYKDLQSKFAEYNVFTEEENLVSEHTYNAYAAFPEAESVTIDPHKMGYIPYSAGGIAIQDIRMRDVISYFATYVFEKGADIPALLGAYILEGSKAGATAASVWAAHKTLPLNVTGYGKLVGASIEGARRFYNFLSGLEFKVGDKTIEVHPLTDPDFNMVDYVFQEKGNNNLVEMNELNHEFYDQASYVTGSIYGNEYLTSHTDFAIPDYGNSPFKFVNNLGVTEEGWKEAGKVTVLRAAVMTPYMNKAENFDYFAPKIKQAMQEKLEAIYEDRK

SEQ ID NO: 19 - DNA, 1863 bp, Artificial sequence
  Engineered sequence
atgagcaacaccagtttcagcgcaaaagataccgatctgagtgcactgtttatcggtgacaaagcagaaaatggtcagctgtataaggacctgctgggcaaactggttgatgaacatctgggttggcgccagaattatatgccgcaggatccgccgatgatcagcgccgaacagcagaccagcccggaatttcgtggtaccgtgaataatatgaaggacgttctggatgagctgagcagtcgcctgcgtagtcagagcgttccgtggcataatgccggtcgttattggggccacatgaatagcgaaaccctgatgccggcaattctggcctataattatgcaatgctgtggaatggtaacaacgtggcctatgaaagcagcccggcaaccagccagatggaagaagaagttggtctggaatttgccaccctgatgggctataccaatggttggggccatattgttgcagatggtagcctggcaaatctggaaggcctgtggtatgcacgcaatattaagagcctgccgtttgccatgaaagccgttgatccgaccattgttgccggcaaaaccgattgggaactgagtaatatgagcaccaaagaaatcatggacctggttgaagccaatggtgacaaaattgatgagatcaaggccaaaagcgcccgcggcggtaaagatctggataaactgggtaaatggctggttccgcagaccaaacattatagttggctgaaagccgcagatattatcggcattggcctggatcaggttattccggttccggttgatagcaattatcgtatggatatcaacgagctggagaaaattatccgcgaactggcaagtaccgaaaccccgattctgggcgttgtgggcgttgtgggtagtaccgaagaaggtgccgttgatggcattaatgaaattgcagaactgcgtaacaagctggtgaaagaaggtatctatttctacttccacatcgacgccgcctatggtggctatggtcgcgcaattctgctggatgaagataataagctgatcccgtataaggaccttcagagtaaattcgccgaatataacgtgttcaccgaagaagaaaacctggtgagtgaacatacctataacgcctatgccgcatttccggaagccgaaagtgttaccattgatccgcataaaatgggctatatcccgtatagtgcaggcggcattgccattcaggatattcgcatgcgtgatgttatcagctatttcgcaacctatgtgttcgaaaagggcgcagatattccggcactgctgggtgcttatattctggaaggcagtaaagcaggcgcaaccgcagccagtgtttgggcagcacataaaaccctgccgctgaatgttaccggttatggtaaactggttggtgcaagcattgaaggcgcccgccgtttttataattttctgagcggcctggaattcaaggtgggcgataaaaccattgaagttcatccgctgaccgatccggattttaatatggttgattacgtgttccaggagaagggcaataataatctggtggaaatgaacgagctgaaccatgaattttacaaccaggcaagctacgttaccggtagcatctatggcaatgaatatctgaccagccataccgatttcgcaattccggattatggtaatagcccgtttaagtttgtgaacaacctgggcgtgaccgaagaaggctggaaagaagcaggtaaagtgaccgttctgcgcgccgctgtgatgacaccttatatgaataaggcagagaacttcgactacttcgccccgaaaattaagcaggccatgcaggaaaaactggaagccatctatgaagatcgtaag

SEQ ID NO: 20 - protein, 621 aa, Artificial sequence
  Engineered sequence
MSNTSFSAKDTDLSALFIGDKAENGQLYKDLLGKLVDEHLGWRQNYMPQDPPMISAEQQTSPEFRGTVNNMKDVLDELSSRLRSQSVPWHNAGRYWGHMNSETLMPAILAYNYAMLWNGNNVAYESSPATSQMEEEVGLEFATLMGYTNGWGHIVADGSLANLEGLWYARNIKSLPFAMKAVDPTIVAGKTDWELSNMSTKEIMDLVEANGDKIDEIKAKSARGGKDLDKLGKWLVPQTKHYSWLKAADIIGIGLDQVIPVPVDSNYRMDINELEKIIRELASTETPILGVVGVVGSTEEGAVDGINEIAELRNKLVKEGIYFYFHIDAAYGGYGRAILLDEDNKLIPYKDLQSKFAEYNVFTEEENLVSEHTYNAYAAFPEAESVTIDPHKMGYIPYSAGGIAIQDIRMRDVISYFATYVFEKGADIPALLGAYILEGSKAGATAASVWAAHKTLPLNVTGYGKLVGASIEGARRFYNFLSGLEFKVGDKTIEVHPLTDPDFNMVDYVFQEKGNNNLVEMNELNHEFYNQASYVTGSIYGNEYLTSHTDFAIPDYGNSPFKFVNNLGVTEEGWKEAGKVTVLRAAVMTPYMNKAENFDYFAPKIKQAMQEKLEAIYEDRK

SEQ ID NO: 21 - DNA, 1863 bp, Artificial sequence
  Engineered sequence
atgagcaacaccagtttcagcgcaaaagataccgatctgagtgcactgtttatcggtgacaaagcagaaaatggtcagctgtataaggacctgctgggcaaactggttgatgaacatctgggttggcgccagaattatatgccgcaggatactccgatgatcagcgccgaacagcagaccagcccggaatttcgtggtaccgtgaataatatgaaggacgttctggatgagctgagcagtcgcctgcgtagtcagagcgttccgtggcataatgccggtcgttattggggccacatgaatagcgaaaccctgatgccggcaattctggcctataattatgcaatgctgtggaatggtaacaacgtggcctatgaaagcagcccggcaaccagccagatggaagaagaagttggtctggaatttgccaccctgatgggctataccaatggttggggccatattgttgcagatggtagcctggcaaatctggaaggcctgtggtatgcacgcaatattaagagcctgccgtttgccatgaaagccgttgatccgaccattgttgccggcaaaaccgattgggaactgagtaatatgagcaccaaagaaatcatggacctggttgaagccaatggtgacaaaattgatgagatcaaggccaaaagcgcccgcggcggtaaagatctggataaactgggtaaatggctggttccgcagaccaaacattatagttggctgaaagccgcagatattatcggcattggcctggatcaggttattccggttccggttgatagcaattatcgtatggatatcaacgagctggagaaaattatccgcgaactggcaagtaccgaaaccccgattctgggcgttgtgggcgttgtgggtagtaccgaagaaggtgccgttgatggcattaatgaaattgcagaactgcgtaacaagctggtgaaagaaggtatctatttctacttccacatcgacgccgcctatggtggctatggtcgcgcaattctgctggatgaagataataagctgatcccgtataaggaccttcagagtaaattcgccgaatataacgtgttcaccgaagaagaaaacctggtgagtgaacatacctataacgcctatgccgcatttccggaagccgaaagtgttaccattgatccgcataaaatgggctatatcccgtatagtgcaggcggcattgccattcaggatattcgcatgcgtgatgttatcagctatttcgcaacctatgtgttcgaaaagggcgcagatattccggcactgctgggtgcttatattctggaaggcagtaaagcaggcgcaaccgcagccagtgtttgggcagcacataaaaccctgccgctgaatgttaccggttatggtaaactggttggtgcaagcattgaaggcgcccgccgtttttataattttctgagcggcctggaattcaaggtgggcgataaaaccattgaagttcatccgctgaccgatccggattttaatatggttgattacgtgttccaggagaagggcaataataatctggtggaaatgaacgagctgaaccatgaattttacaaccaggcaagctacgttaccggtagcatctatggcaatgaatatctgaccagccataccgatttcgcaattccggattatggtaatagcccgtttaagtttgtgaacaacctgggcgtgaccgaagaaggctggaaagaagcaggtaaagtgaccgttctgcgcgccgctgtgatgacaccttatatgaataaggcagagaacttcgactacttcgccccgaaaattaagcaggccatgcaggaaaaactggaagccatctatgaagatcgtaag

SEQ ID NO: 22 - protein, 621 aa, Artificial sequence
  Engineered sequence
MSNTSFSAKDTDLSALFIGDKAENGQLYKDLLGKLVDEHLGWRQNYMPQDTPMISAEQQTSPEFRGTVNNMKDVLDELSSRLRSQSVPWHNAGRYWGHMNSETLMPAILAYNYAMLWNGNNVAYESSPATSQMEEEVGLEFATLMGYTNGWGHIVADGSLANLEGLWYARNIKSLPFAMKAVDPTIVAGKTDWELSNMSTKEIMDLVEANGDKIDEIKAKSARGGKDLDKLGKWLVPQTKHYSWLKAADIIGIGLDQVIPVPVDSNYRMDINELEKIIRELASTETPILGVVGVVGSTEEGAVDGINEIAELRNKLVKEGIYFYFHIDAAYGGYGRAILLDEDNKLIPYKDLQSKFAEYNVFTEEENLVSEHTYNAYAAFPEAESVTIDPHKMGYIPYSAGGIAIQDIRMRDVISYFATYVFEKGADIPALLGAYILEGSKAGATAASVWAAHKTLPLNVTGYGKLVGASIEGARRFYNFLSGLEFKVGDKTIEVHPLTDPDFNMVDYVFQEKGNNNLVEMNELNHEFYNQASYVTGSIYGNEYLTSHTDFAIPDYGNSPFKFVNNLGVTEEGWKEAGKVTVLRAAVMTPYMNKAENFDYFAPKIKQAMQEKLEAIYEDRK

SEQ ID NO: 23 - DNA, 1863 bp, Artificial sequence
  Engineered sequence
atgagcaacaccagtttcagcgcaaaagataccgatctgagtgcactgtttatcggtgacaaagcagaaaatggtcagctgtataaggacctgctgggcaaactggttgatgaacatctgggttggcgccagaattatatgccgcaggataaaactatgatcagcgccgaacagcagaccagcccggaatttcgtggtaccgtgaataatatgaaggacgttctggatgagctgagcagtcgcctgcgtagtcagagcgttccgtggcataatgccggtcgttattggggccacatgaatagcgaaaccctgatgccggcaattctggcctataattatgcaatgctgtggaatggtaacaacgtggcctatgaaagcagcccggcaaccagccagatggaagaagaagttggtctggaatttgccaccctgatgggctataccaatggttggggccatattgttgcagatggtagcctggcaaatctggaaggcctgtggtatgcacgcaatattaagagcctgccgtttgccatgaaagccgttgatccgaccattgttgccggcaaaaccgattgggaactgagtaatatgagcaccaaagaaatcatggacctggttgaagccaatggtgacaaaattgatgagatcaaggccaaaagcgcccgcggcggtaaagatctggataaactgggtaaatggctggttccgcagaccaaacattatagttggctgaaagccgcagatattatcggcattggcctggatcaggttattccggttccggttgatagcaattatcgtatggatatcaacgagctggagaaaattatccgcgaactggcaagtaccgaaaccccgattctgggcgttgtgggcgttgtgggtagtaccgaagaaggtgccgttgatggcattaatgaaattgcagaactgcgtaacaagctggtgaaagaaggtatctatttctacttccacatcgacgccgcctatggtggctatggtcgcgcaattctgctggatgaagataataagctgatcccgtataaggaccttcagagtaaattcgccgaatataacgtgttcaccgaagaagaaaacctggtgagtgaacatacctataacgcctatgccgcatttccggaagccgaaagtgttaccattgatccgcataaaatgggctatatcccgtatagtgcaggcggcattgccattcaggatattcgcatgcgtgatgttatcagctatttcgcaacctatgtgttcgaaaagggcgcagatattccggcactgctgggtgcttatattctggaaggcagtaaagcaggcgcaaccgcagccagtgtttgggcagcacataaaaccctgccgctgaatgttaccggttatggtaaactggttggtgcaagcattgaaggcgcccgccgtttttataattttctgagcggcctggaattcaaggtgggcgataaaaccattgaagttcatccgctgaccgatccggattttaatatggttgattacgtgttccaggagaagggcaataataatctggtggaaatgaacgagctgaaccatgaattttacaaccaggcaagctacgttaccggtagcatctatggcaatgaatatctgaccagccataccgatttcgcaattccggattatggtaatagcccgtttaagtttgtgaacaacctgggcgtgaccgaagaaggctggaaagaagcaggtaaagtgaccgttctgcgcgccgctgtgatgacaccttatatgaataaggcagagaacttcgactacttcgccccgaaaattaagcaggccatgcaggaaaaactggaagccatctatgaagatcgtaag

SEQ ID NO: 24 - protein, 621 aa, Artificial sequence
  Engineered sequence
MSNTSFSAKDTDLSALFIGDKAENGQLYKDLLGKLVDEHLGWRQNYMPQDKTMISAEQQTSPEFRGTVNNMKDVLDELSSRLRSQSVPWHNAGRYWGHMNSETLMPAILAYNYAMLWNGNNVAYESSPATSQMEEEVGLEFATLMGYTNGWGHIVADGSLANLEGLWYARNIKSLPFAMKAVDPTIVAGKTDWELSNMSTKEIMDLVEANGDKIDEIKAKSARGGKDLDKLGKWLVPQTKHYSWLKAADIIGIGLDQVIPVPVDSNYRMDINELEKIIRELASTETPILGVVGVVGSTEEGAVDGINEIAELRNKLVKEGIYFYFHIDAAYGGYGRAILLDEDNKLIPYKDLQSKFAEYNVFTEEENLVSEHTYNAYAAFPEAESVTIDPHKMGYIPYSAGGIAIQDIRMRDVISYFATYVFEKGADIPALLGAYILEGSKAGATAASVWAAHKTLPLNVTGYGKLVGASIEGARRFYNFLSGLEFKVGDKTIEVHPLTDPDFNMVDYVFQEKGNNNLVEMNELNHEFYNQASYVTGSIYGNEYLTSHTDFAIPDYGNSPFKFVNNLGVTEEGWKEAGKVTVLRAAVMTPYMNKAENFDYFAPKIKQAMQEKLEAIYEDRK

SEQ ID NO: 25 - DNA, 1863 bp, Artificial sequence
  Engineered sequence
atgagcaacaccagtttcagcgcaaaagataccgatctgagtgcactgtttatcggtgacaaagcagaaaatggtcagctgtataaggacctgctgggcaaactggttgatgaacatctgggttggcgccagaattatatgccgcaggataaagtgatgatcagcgccgaacagcagaccagcccggaatttcgtggtaccgtgaataatatgaaggacgttctggatgagctgagcagtcgcctgcgtagtcagagcgttccgtggcataatgccggtcgttattggggccacatgaatagcgaaaccctgatgccggcaattctggcctataattatgcaatgctgtggaatggtaacaacgtggcctatgaaagcagcccggcaaccagccagatggaagaagaagttggtctggaatttgccaccctgatgggctataccaatggttggggccatattgttgcagatggtagcctggcaaatctggaaggcctgtggtatgcacgcaatattaagagcctgccgtttgccatgaaagccgttgatccgaccattgttgccggcaaaaccgattgggaactgagtaatatgagcaccaaagaaatcatggacctggttgaagccaatggtgacaaaattgatgagatcaaggccaaaagcgcccgcggcggtaaagatctggataaactgggtaaatggctggttccgcagaccaaacattatagttggctgaaagccgcagatattatcggcattggcctggatcaggttattccggttccggttgatagcaattatcgtatggatatcaacgagctggagaaaattatccgcgaactggcaagtaccgaaaccccgattctgggcgttgtgggcgttgtgggtagtaccgaagaaggtgccgttgatggcattaatgaaattgcagaactgcgtaacaagctggtgaaagaaggtatctatttctacttccacatcgacgccgcctatggtggctatggtcgcgcaattctgctggatgaagataataagctgatcccgtataaggaccttcagagtaaattcgccgaatataacgtgttcaccgaagaagaaaacctggtgagtgaacatacctataacgcctatgccgcatttccggaagccgaaagtgttaccattgatccgcataaaatgggctatatcccgtatagtgcaggcggcattgccattcaggatattcgcatgcgtgatgttatcagctatttcgcaacctatgtgttcgaaaagggcgcagatattccggcactgctgggtgcttatattctggaaggcagtaaagcaggcgcaaccgcagccagtgtttgggcagcacataaaaccctgccgctgaatgttaccggttatggtaaactggttggtgcaagcattgaaggcgcccgccgtttttataattttctgagcggcctggaattcaaggtgggcgataaaaccattgaagttcatccgctgaccgatccggattttaatatggttgattacgtgttccaggagaagggcaataataatctggtggaaatgaacgagctgaaccatgaattttacaaccaggcaagctacgttaccggtagcatctatggcaatgaatatctgaccagccataccgatttcgcaattccggattatggtaatagcccgtttaagtttgtgaacaacctgggcgtgaccgaagaaggctggaaagaagcaggtaaagtgaccgttctgcgcgccgctgtgatgacaccttatatgaataaggcagagaacttcgactacttcgccccgaaaattaagcaggccatgcaggaaaaactggaagccatctatgaagatcgtaag

SEQ ID NO: 26 - protein, 621 aa, Artificial sequence
  Engineered sequence
MSNTSFSAKDTDLSALFIGDKAENGQLYKDLLGKLVDEHLGWRQNYMPQDKVMISAEQQTSPEFRGTVNNMKDVLDELSSRLRSQSVPWHNAGRYWGHMNSETLMPAILAYNYAMLWNGNNVAYESSPATSQMEEEVGLEFATLMGYTNGWGHIVADGSLANLEGLWYARNIKSLPFAMKAVDPTIVAGKTDWELSNMSTKEIMDLVEANGDKIDEIKAKSARGGKDLDKLGKWLVPQTKHYSWLKAADIIGIGLDQVIPVPVDSNYRMDINELEKIIRELASTETPILGVVGVVGSTEEGAVDGINEIAELRNKLVKEGIYFYFHIDAAYGGYGRAILLDEDNKLIPYKDLQSKFAEYNVFTEEENLVSEHTYNAYAAFPEAESVTIDPHKMGYIPYSAGGIAIQDIRMRDVISYFATYVFEKGADIPALLGAYILEGSKAGATAASVWAAHKTLPLNVTGYGKLVGASIEGARRFYNFLSGLEFKVGDKTIEVHPLTDPDFNMVDYVFQEKGNNNLVEMNELNHEFYNQASYVTGSIYGNEYLTSHTDFAIPDYGNSPFKFVNNLGVTEEGWKEAGKVTVLRAAVMTPYMNKAENFDYFAPKIKQAMQEKLEAIYEDRK

SEQ ID NO: 27 - DNA, 1863 bp, Artificial sequence
  Engineered sequence
atgagcaacaccagtttcagcgcaaaagataccgatctgagtgcactgtttatcggtgacaaagcagaaaatggtcagctgtataaggacctgctgggcaaactggttgatgaacatctgggttggcgccagaattatatgccgcaggataaaccgatgatcagcgccgaacagcagaccagcccggaatttcgtggtaccgtgaataatatgaaggacgttctggatgagctgagcagtcgcctgcgtagtcagagcgttccgtggcataatgccggtcgttattggggccacatgaatagcgaaaccctgatgccggcaattctggcctataattatgcaatgctgtggaatggtaacaacgtggcctatgaaagcagcccggcaaccagccagatggaagaagaagttggtctggaatttgccaccctgatgggctataccaatggttggggccatattgttgcagatggtagcctggcaaatctggaaggcctgtggtatgcacgcaatattaagagcctgccgtttgccatgaaagccgttgatccgaccattgttgccggcaaaaccgattgggaactgagtaatatgagcaccaaagaaatcatggacctggttgaagccaatggtgacaaaattgatgagatcaaggccaaaagcgcccgcggcggtaaagatctggataaactgggtaaatggctggttccgcagaccaaacattatagttggctgaaagccgcagatattatcggcattggcctggatcaggttattccggttccggttgatagcaattatcgtatggatatcaacgagctggagaaaattatccgcgaactggcaagtaccgaaaccccgattctgggcgttgtgggcgttgtgggtagtaccgaagaaggtgccgttgatggcattaatgaaattgcagaactgcgtaacaagctggtgaaagaaggtatctatttctacttccacatcgacgccgcctatggtggctatggtcgcgcaattctgctggatgaagataataagctgatcccgtataaggaccttcagagtaaattcgccgaatataacgtgttcaccgaagaagaaaacctggtgagtgaacatacctataacgcctatgccgcatttccggaagccgaaagtgttaccattgatccgcataaaatgggctatatcccgtatagtgcaggcggcattgccattcaggatattcgcatgcgtgatgttatcagctatttcgcaacctatgtgttcgaaaagggcgcagatattccggcactgctgggtgcttatattctggaaggcagtaaagcaggcgcaaccgcagccagtgtttgggcagcacataaaaccctgccgctgaatgttaccggttatggtaaactggttggtgcaagcattgaaggcgcccgccgtttttataattttctgagcggcctggaattcaaggtgggcgataaaaccattgaagttcatccgctgaccgatccggattttaatatggttgattacgtgttccaggagaagggcaataataatctggtggaaatgaacgagctgaaccatgaattttacaaccaggcaagctactggaccggtagcatctatggcaatgaatatctgaccagccataccgatttcgcaattccggattatggtaatagcccgtttaagtttgtgaacaacctgggcgtgaccgaagaaggctggaaagaagcaggtaaagtgaccgttctgcgcgccgctgtgatgacaccttatatgaataaggcagagaacttcgactacttcgccccgaaaattaagcaggccatgcaggaaaaactggaagccatctatgaagatcgtaag

SEQ ID NO: 28 - protein, 621 aa, Artificial sequence
  Engineered sequence
MSNTSFSAKDTDLSALFIGDKAENGQLYKDLLGKLVDEHLGWRQNYMPQDKPMISAEQQTSPEFRGTVNNMKDVLDELSSRLRSQSVPWHNAGRYWGHMNSETLMPAILAYNYAMLWNGNNVAYESSPATSQMEEEVGLEFATLMGYTNGWGHIVADGSLANLEGLWYARNIKSLPFAMKAVDPTIVAGKTDWELSNMSTKEIMDLVEANGDKIDEIKAKSARGGKDLDKLGKWLVPQTKHYSWLKAADIIGIGLDQVIPVPVDSNYRMDINELEKIIRELASTETPILGVVGVVGSTEEGAVDGINEIAELRNKLVKEGIYFYFHIDAAYGGYGRAILLDEDNKLIPYKDLQSKFAEYNVFTEEENLVSEHTYNAYAAFPEAESVTIDPHKMGYIPYSAGGIAIQDIRMRDVISYFATYVFEKGADIPALLGAYILEGSKAGATAASVWAAHKTLPLNVTGYGKLVGASIEGARRFYNFLSGLEFKVGDKTIEVHPLTDPDFNMVDYVFQEKGNNNLVEMNELNHEFYNQASYWTGSIYGNEYLTSHTDFAIPDYGNSPFKFVNNLGVTEEGWKEAGKVTVLRAAVMTPYMNKAENFDYFAPKIKQAMQEKLEAIYEDRK

SEQ ID NO: 29 - DNA, 1863 bp, Artificial sequence
  Engineered sequence
atgagcaacaccagtttcagcgcaaaagataccgatctgagtgcactgtttatcggtgacaaagcagaaaatggtcagctgtataaggacctgctgggcaaactggttgatgaacatctgggttggcgccagaattatatgccgcaggataaaccgatgatcagcgccgaacagcagaccagcccggaatttcgtggtaccgtgaataatatgaaggacgttctggatgagctgagcagtcgcctgcgtagtcagagcgttccgtggcataatgccggtcgttattggggccacatgaatagcgaaaccctgatgccggcaattctggcctataattatgcaatgctgtggaatggtaacaacgtggcctatgaaagcagcccggcaaccagccaggtggaagaagaagttggtctggaatttgccaccctgatgggctataccaatggttggggccatattgttgcagatggtagcctggcaaatctggaaggcctgtggtatgcacgcaatattaagagcctgccgtttgccatgaaagccgttgatccgaccattgttgccggcaaaaccgattgggaactgagtaatatgagcaccaaagaaatcatggacctggttgaagccaatggtgacaaaattgatgagatcaaggccaaaagcgcccgcggcggtaaagatctggataaactgggtaaatggctggttccgcagaccaaacattatagttggctgaaagccgcagatattatcggcattggcctggatcaggttattccggttccggttgatagcaattatcgtatggatatcaacgagctggagaaaattatccgcgaactggcaagtaccgaaaccccgattctgggcgttgtgggcgttgtgggtagtaccgaagaaggtgccgttgatggcattaatgaaattgcggaactgcgtaacaagctggtgaaagaaggtatctatttctacttccacatcgacgccgcctatggtggctatggtcgcgcaattctgctggatgaagataataagctgatcccgtataaggaccttcagagtaaattcgccgaatataacgtgttcaccgaagaagaaaacctggtgagtgaacatacctataacgcctatgccgcatttccggaagccgaaagtgttaccattgatccgcataaaatgggctatatcccgtatagtgcaggcggcattgccattcaggatattcgcatgcgtgatgttatcagctatttcgcaacctatgtgttcgaaaagggcgcagatattccggcactgctgggtgcttatattctggaaggcagtaaagcaggcgcaaccgcagccagtgtttgggcagcacataaaaccctgccgctgaatgttaccggttatggtagactggttggtgcaagcattgaaggcgcccgccgtttttataattttctgagcggcctggaattcaaggtgggcgataaaaccattgaagttcatccgctgaccgatccggattttaatatggttgattacgtgttccaggagaagggcaataataatctggtggaaatgaacgagctgaaccatgaattttacaaccaggcaagctacgttaccggtagcatctatggcaatgaatatctgaccagccataccgatttcgcaattccggattatggtaatagcccgtttaagtttgtgaacaacctgggcgtgaccgaagaaggctggaaagaagcaggtaaagtgaccgttctgcgcgccgctgtgatgacaccttatatgaataaggcagagaacttcgactacttcgccccgaaaattaagcaggccatgcaggaaaaactggaagccatctatgaagatcgtaag

SEQ ID NO: 30 - protein, 621 aa, Artificial sequence
  Engineered sequence
MSNTSFSAKDTDLSALFIGDKAENGQLYKDLLGKLVDEHLGWRQNYMPQDKPMISAEQQTSPEFRGTVNNMKDVLDELSSRLRSQSVPWHNAGRYWGHMNSETLMPAILAYNYAMLWNGNNVAYESSPATSQVEEEVGLEFATLMGYTNGWGHIVADGSLANLEGLWYARNIKSLPFAMKAVDPTIVAGKTDWELSNMSTKEIMDLVEANGDKIDEIKAKSARGGKDLDKLGKWLVPQTKHYSWLKAADIIGIGLDQVIPVPVDSNYRMDINELEKIIRELASTETPILGVVGVVGSTEEGAVDGINEIAELRNKLVKEGIYFYFHIDAAYGGYGRAILLDEDNKLIPYKDLQSKFAEYNVFTEEENLVSEHTYNAYAAFPEAESVTIDPHKMGYIPYSAGGIAIQDIRMRDVISYFATYVFEKGADIPALLGAYILEGSKAGATAASVWAAHKTLPLNVTGYGRLVGASIEGARRFYNFLSGLEFKVGDKTIEVHPLTDPDFNMVDYVFQEKGNNNLVEMNELNHEFYNQASYVTGSIYGNEYLTSHTDFAIPDYGNSPFKFVNNLGVTEEGWKEAGKVTVLRAAVMTPYMNKAENFDYFAPKIKQAMQEKLEAIYEDRK

SEQ ID NO: 31 - DNA, 1863 bp, Artificial sequence
  Engineered sequence
atgagcaacaccagtttcagcgcaaaagataccgatctgagtgcactgtttatcggtgacaaagcagaaaatggtcagctgtataaggacctgctgggcaaactggttgatgaacatctgggttggcgccagaattatatgccgcaggataaaccgatgatcagcgccgaacagcagaccagcccggaatttcgtggtaccgtgaataatatgaaggacgttctggatgagctgagcagtcgcctgcgtagtcagagcgttccgtggcataatgccggtcgttattggggccacatgaatagcgaaaccctgatgccggcaattctggcctataattatgcaatgctgtggaatggtaacaacgtggcctatgaaagcagcccggcaaccagccagatggaagaagaagttggtctggaatttgccaccctgatgggctataccaatggttggggccatattgttgcagatggtagcctggcaaatctggaaggcctgtggtatgcacgcaatattaagagcctgccgtttgccatgaaagccgttgatccgaccattgttgccggcaaaaccgattgggaactgagtaatatgagcaccaaagaaatcatggacctggttgaagccaatggtgacaaaattgatgagatcaaggccaaaagcgcccgcggcggtaaagatctggataaactgggtaaatggctggttccgcagaccaaacattatagttggctgaaagccgcagatattatcggcattggcctggatcaggttattccggttccggttgatagcaattatcgtatggatatcaacgagctggagaaaattatccgcgaactggcaagtaccgaaaccccgattctgggcgttgtgggcgttgtgggtagtaccgaagaaggtgccgttgatggcattaatgaaattgcagaactgcgtaacaagctggtgaaagaaggtatctatttctacttccacatcgacgccgcctatggtggctatggtcgcgcaattctgctggatgaagataataagctgatcccgtataaggaccttcagagtaaattcgccgaatataacgtgttcaccgaagaagaaaacctggtgagtgaacatacctataacgcctatgccgcatttccggaagccgaaagtgttaccattgatccgcataaaatgggctatatcccgtatagtgcaggcggcattgccattcaggatattcgcatgcgtgatgttatcagctatttcgcaacctatgtgttcgaaaagggcgcagatattccggcactgctgggtgcttatattctggaaggcagtaaagcaggcgcaaccgcagccagtgtttgggcagcacataaaaccctgccgctgaatgttaccggttatggtaaactggttggtgcaagcattgaaggcgcccgccgtttttataattttctgagcggcctggaattcaaggtgggcgataaaaccattgaagttcatccgctgaccgatccggattttaatatggttgattacgtgttccaggagaagggcaataataatctggtggaaatgaacgagctgaaccatgaattttacaaccaggcaagctacgttggtggtagcatctatggcaatgaatatctgaccagccataccgatttcgcaattccggattatggtaatagcccgtttaagtttgtgaacaacctgggcgtgaccgaagaaggctggaaagaagcaggtaaagtgaccgttctgcgcgccgctgtgatgacaccttatatgaataaggcagagaacttcgactacttcgccccgaaaattaagcaggccatgcaggaaaaactggaagccatctatgaagatcgtaag

SEQ ID NO: 32 - protein, 621 aa, Artificial sequence
  Engineered sequence
MSNTSFSAKDTDLSALFIGDKAENGQLYKDLLGKLVDEHLGWRQNYMPQDKPMISAEQQTSPEFRGTVNNMKDVLDELSSRLRSQSVPWHNAGRYWGHMNSETLMPAILAYNYAMLWNGNNVAYESSPATSQMEEEVGLEFATLMGYTNGWGHIVADGSLANLEGLWYARNIKSLPFAMKAVDPTIVAGKTDWELSNMSTKEIMDLVEANGDKIDEIKAKSARGGKDLDKLGKWLVPQTKHYSWLKAADIIGIGLDQVIPVPVDSNYRMDINELEKIIRELASTETPILGVVGVVGSTEEGAVDGINEIAELRNKLVKEGIYFYFHIDAAYGGYGRAILLDEDNKLIPYKDLQSKFAEYNVFTEEENLVSEHTYNAYAAFPEAESVTIDPHKMGYIPYSAGGIAIQDIRMRDVISYFATYVFEKGADIPALLGAYILEGSKAGATAASVWAAHKTLPLNVTGYGKLVGASIEGARRFYNFLSGLEFKVGDKTIEVHPLTDPDFNMVDYVFQEKGNNNLVEMNELNHEFYNQASYVGGSIYGNEYLTSHTDFAIPDYGNSPFKFVNNLGVTEEGWKEAGKVTVLRAAVMTPYMNKAENFDYFAPKIKQAMQEKLEAIYEDRK

SEQ ID NO: 33 - DNA, 1863 bp, Artificial sequence
  Engineered sequence
atgagcaacaccagtttcagcgcaaaagataccgatctgagtgcactgtttatcggtgacaaagcagaaaatggtcagctgtataaggacctgctgggcaaactggttgatgaacatctgggttggcgccagaattatatgccgcaggataaaccgatgatcagcgccgaacagcagaccagcccggaatttcgtggtaccgtgaataatatgaaggacgttctggatgagctgagcagtcgcctgcgtagtcagagcgttccgtggcataatgccggtcgttattggggccacatgaatagcgaaaccctgatgccggcaattctggcctataattatgcaatgctgtggaatggtaacaacgtggcctatgaaagcagcccggcaaccagccagatggaagaagaagttggtctggaatttgccaccctgatgggctataccaatggttggggccatattgttgcagatggtagcctggcaaatctggaaggcctgtggtatgcacgcaatattaagagcctgccgtttgccatgaaagccgttgatccgaccattgttgccggcaaaaccgattgggaactgagtaatatgagcaccaaagaaatcatggacctggttgaagccaatggtgacaaaattgatgagatcaaggccaaaagcgcccgcggcggtaaagatctggataaactgggtaaatggctggttccgcagaccaaacattatagttggctgaaagccgcagatattatcggcattggcctggatcaggttattccggttccggttgatagcaattatcgtatggatatcaacgagctggagaaaattatccgcgaactggcaagtaccgaaaccccgattctgggcgttgtgggcgttgtgggtagtaccgaagaaggtgccgttgatggcattaatgaaattgcagaactgcgtaacaagctggtgaaagaaggtatctatttctacttccacatcgacgccgcctatggtggctatggtcgcgcaattctgctggatgaagataataagctgatcccgtataaggaccttcagagtaaattcgccgaatataacgtgttcaccgaagaagaaaacctggtgagtgaacatacctataacgcctatgccgcatttccggaagccgaaagtgttaccattgatccgcataaaatgggctatatcccgtatagtgcaggcggcattgccattcaggatattcgcatgcgtgatgttatcagctatttcgcaacctatgtgttcgaaaagggcgcagatattccggcactgctgggtgcttatattctggaaggcagtaaagcaggcgcaaccgcagccagtgtttgggcagcacataaaaccctgccgctgaatgttaccggttatggtaaactggttggtgcaagcattgaaggcgcccgccgtttttataattttctgagcggcctggaattcaaggtgggcgataaaaccattgaagttcatccgctgaccgatccggattttaatatggttgattacgtgttccaggagaagggcaataataatctggtggaaatgaacgagctgaaccatgaattttacaaccaggcaagctacgttaccggtgtgatctatggcaatgaatatctgaccagccataccgatttcgcaattccggattatggtaatagcccgtttaagtttgtgaacaacctgggcgtgaccgaagaaggctggaaagaagcaggtaaagtgaccgttctgcgcgccgctgtgatgacaccttatatgaataaggcagagaacttcgactacttcgccccgaaaattaagcaggccatgcaggaaaaactggaagccatctatgaagatcgtaag

SEQ ID NO: 34 - protein, 621 aa, Artificial sequence
  Engineered sequence
MSNTSFSAKDTDLSALFIGDKAENGQLYKDLLGKLVDEHLGWRQNYMPQDKPMISAEQQTSPEFRGTVNNMKDVLDELSSRLRSQSVPWHNAGRYWGHMNSETLMPAILAYNYAMLWNGNNVAYESSPATSQMEEEVGLEFATLMGYTNGWGHIVADGSLANLEGLWYARNIKSLPFAMKAVDPTIVAGKTDWELSNMSTKEIMDLVEANGDKIDEIKAKSARGGKDLDKLGKWLVPQTKHYSWLKAADIIGIGLDQVIPVPVDSNYRMDINELEKIIRELASTETPILGVVGVVGSTEEGAVDGINEIAELRNKLVKEGIYFYFHIDAAYGGYGRAILLDEDNKLIPYKDLQSKFAEYNVFTEEENLVSEHTYNAYAAFPEAESVTIDPHKMGYIPYSAGGIAIQDIRMRDVISYFATYVFEKGADIPALLGAYILEGSKAGATAASVWAAHKTLPLNVTGYGKLVGASIEGARRFYNFLSGLEFKVGDKTIEVHPLTDPDFNMVDYVFQEKGNNNLVEMNELNHEFYNQASYVTGVIYGNEYLTSHTDFAIPDYGNSPFKFVNNLGVTEEGWKEAGKVTVLRAAVMTPYMNKAENFDYFAPKIKQAMQEKLEAIYEDRK

SEQ ID NO: 35 - DNA, 1863 bp, Artificial sequence
  Engineered sequence
atgagcaacaccagtttcagcgcaaaagataccgatctgagtgcactgtttatcggtgacaaagcagaaaatggtcagctgtataaggacctgctgggcaaactggttgatgaacatctgggttggcgccagaattatatgccgcaggataaaccgatgatcagcgccgaacagcagaccagcccggaatttcgtggtaccgtgaataatatgaaggacgttctggatgagctgagcagtcgcctgcgtagtcagagcgttccgtggcataatgccggtcgttattggggccacatgaatagcgaaaccctgatgccggcaattctggcctataattatgcaatgctgtggaatggtaacaacgtggcctatgaaagcagcccggcaaccagccagatggaagaagaagttggtctggaatttgccaccctgatgggctataccaatggttggggccatattgttgcagatggtagcctggcaaatctggaaggcctgtggtatgcacgcaatattaagagcctgccgtttgccatgaaagccgttgatccgaccattgttgccggcaaaaccgattgggaactgagtaatatgagcaccaaagaaatcatggacctggttgaagccaatggtgacaaaattgatgagatcaaggccaaaagcgcccgcggcggtaaagatctggataaactgggtaaatggctggttccgcagaccaaacattatagttggctgaaagccgcagatattatcggcattggcctggatcaggttattccggttccggttgatagcaattatcgtatggatccgaacgagctggagaaaattatccgcgaactggcaagtaccgaaaccccgattctgggcgttgtgggcgttgtgggtagtaccgaagaaggtgccgttgatggcattaatgaaattgcagaactgcgtaacaagctggtgaaagaaggtatctatttctacttccacatcgacgccgcctatggtggctatggtcgcgcaattctgctggatgaagataataagctgatcccgtataaggaccttcagagtaaattcgccgaatataacgtgttcaccgaagaagaaaacctggtgagtgaacatacctataacgcctatgccgcatttccggaagccgaaagtgttaccattgatccgcataaaatgggctatatcccgtatagtgcaggcggcattgccattcaggatattcgcatgcgtgatgttatcagctatttcgcaacctatgtgttcgaaaagggcgcagatattccggcactgctgggtgcttatattctggaaggcagtaaagcaggcgcaaccgcagccagtgtttgggcagcacataaaaccctgccgctgaatgttaccggttatggtaaactggttggtgcaagcattgaaggcgcccgccgtttttataattttctgagcggcctggaattcaaggtgggcgataaaaccattgaagttcatccgctgaccgatccggattttaatatggttgattacgtgttccaggagaagggcaataataatctggtggaaatgaacgagctgaaccatgaattttacaaccaggcaagctacgttaccggtagcatctatggcaatgaatatctgaccagccataccgatttcgcaattccggattatggtaatagcccgtttaagtttgtgaacaacctgggcgtgaccgaagaaggctggaaagaagcaggtaaagtgaccgttctgcgcgccgctgtgatgacaccttatatgaataaggcagagaacttcgactacttcgccccgaaaattaagcaggccatgcaggaaaaactggaagccatctatgaagatcgtaag

SEQ ID NO: 36 - protein, 621 aa, Artificial sequence
  Engineered sequence
MSNTSFSAKDTDLSALFIGDKAENGQLYKDLLGKLVDEHLGWRQNYMPQDKPMISAEQQTSPEFRGTVNNMKDVLDELSSRLRSQSVPWHNAGRYWGHMNSETLMPAILAYNYAMLWNGNNVAYESSPATSQMEEEVGLEFATLMGYTNGWGHIVADGSLANLEGLWYARNIKSLPFAMKAVDPTIVAGKTDWELSNMSTKEIMDLVEANGDKIDEIKAKSARGGKDLDKLGKWLVPQTKHYSWLKAADIIGIGLDQVIPVPVDSNYRMDPNELEKIIRELASTETPILGVVGVVGSTEEGAVDGINEIAELRNKLVKEGIYFYFHIDAAYGGYGRAILLDEDNKLIPYKDLQSKFAEYNVFTEEENLVSEHTYNAYAAFPEAESVTIDPHKMGYIPYSAGGIAIQDIRMRDVISYFATYVFEKGADIPALLGAYILEGSKAGATAASVWAAHKTLPLNVTGYGKLVGASIEGARRFYNFLSGLEFKVGDKTIEVHPLTDPDFNMVDYVFQEKGNNNLVEMNELNHEFYNQASYVTGSIYGNEYLTSHTDFAIPDYGNSPFKFVNNLGVTEEGWKEAGKVTVLRAAVMTPYMNKAENFDYFAPKIKQAMQEKLEAIYEDRK

SEQ ID NO: 37 - DNA, 1863 bp, Artificial sequence
  Engineered sequence
atgagcaacaccagtttcagcgcaaaagataccgatctgagtgcactgtttatcggtgacaaagcagaaaatggtcagctgtataaggacctgctgggcaaactggttgatgaacatctgggttggcgccagaattatatgccgcaggataaaccgatgatcagcgccgaacagcagaccagcccggaatttcgtggtaccgtgaataatatgaaggacgttctggatgagctgagcagtcgcctgcgtagtcagagcgttccgtggcataatgccggtcgttattggggccacatgaatagcgaaaccctgatgccggcaattctggcctataattatgcaatgctgtggaatggtaacaacgtgtcctatgaaagcagcccggcaaccagccagatggaagaagaagttggtctggaatttgccaccctgatgggctataccaatggttggggccatattgttgcagatggtagcctggcaaatctggaaggcctgtggtatgcacgcaatattaagagcctgccgtttgccatgaaagccgttgatccgaccattgttgccggcaaaaccgattgggaactgagtaatatgagcaccaaagaaatcatggacctggttgaagccaatggtgacaaaattgatgagatcaaggccaaaagcgcccgcggcggtaaagatctggataaactgggtaaatggctggttccgcagaccaaacattatagttggctgaaagccgcagatattatcggcattggcctggatcaggttattccggttccggttgatagcaattatcgtatggatagtaacgagctggagaaaattatccgcgaactggcaagtaccgaaaccccgattctgggcgttgtgggcgttgtgggtagtaccgaagaaggtgccgttgatggcattaatgaaattgcagaactgcgtaacaagctggtgaaagaaggtatctatttctacttccacatcgacgccgcctatggtggctatggtcgcgcaattctgctggatgaagataataagctgatcccgtataaggaccttcagagtaaattcgccgaatataacgtgttcaccgaagaagaaaacctggtgagtgaacatacctataacgcctatgccgcatttccggaagccgaaagtgttaccattgatccgcataaaatgggctatatcccgtatagtgcaggcggcattgccattcaggatattcgcatgcgtgatgttatcagctatttcgcaacctatgtgttcgaaaagggcgcagatattccggcactgctgggtgcttatattctggaaggcagtaaagcaggcgcaaccgcagccagtgtttgggcagcacataaaaccctgccgctgaatgttaccggttatggtaaactggttggtgcaagcattgaaggcgcccgccgtttttataattttctgagcggcctggaattcaaggtgggcgataaaaccattgaagttcatccgctgaccgatccggattttaatatggttgattacgtgttccaggagaagggcaataataatctggtggaaatgaacgagctgaaccatgaattttacaaccaggcaagctacgttaccggtagcatctatggcaatgaatatctgaccagccataccgatttcgcaattccggattatggtaatagcccgtttaagtttgtgaacaacctgggcgtgaccgaagaaggctggaaagaagcaggtaaagtgaccgttctgcgcgccgctgtgatgacaccttatatgaataaggcagagaacttcgactacttcgccccgaaaattaagcaggccatgcaggaaaaactggaagccatctatgaagatcgtaag

SEQ ID NO: 38 - protein, 621 aa, Artificial sequence
  Engineered sequence
MSNTSFSAKDTDLSALFIGDKAENGQLYKDLLGKLVDEHLGWRQNYMPQDKPMISAEQQTSPEFRGTVNNMKDVLDELSSRLRSQSVPWHNAGRYWGHMNSETLMPAILAYNYAMLWNGNNVSYESSPATSQMEEEVGLEFATLMGYTNGWGHIVADGSLANLEGLWYARNIKSLPFAMKAVDPTIVAGKTDWELSNMSTKEIMDLVEANGDKIDEIKAKSARGGKDLDKLGKWLVPQTKHYSWLKAADIIGIGLDQVIPVPVDSNYRMDSNELEKIIRELASTETPILGVVGVVGSTEEGAVDGINEIAELRNKLVKEGIYFYFHIDAAYGGYGRAILLDEDNKLIPYKDLQSKFAEYNVFTEEENLVSEHTYNAYAAFPEAESVTIDPHKMGYIPYSAGGIAIQDIRMRDVISYFATYVFEKGADIPALLGAYILEGSKAGATAASVWAAHKTLPLNVTGYGKLVGASIEGARRFYNFLSGLEFKVGDKTIEVHPLTDPDFNMVDYVFQEKGNNNLVEMNELNHEFYNQASYVTGSIYGNEYLTSHTDFAIPDYGNSPFKFVNNLGVTEEGWKEAGKVTVLRAAVMTPYMNKAENFDYFAPKIKQAMQEKLEAIYEDRK

SEQ ID NO: 39 - DNA, 1863 bp, Artificial sequence
  Engineered sequence
atgagcaacaccagtttcagcgcaaaagataccgatctgagtgcactgtttatcggtgacaaagcagaaaatggtcagctgtataaggacctgctgggcaaactggttgatgaacatctgggttggcgccagaattatatgccgcaggataaaccgatgatcagcgccgaacagcagaccagcccggaatttcgtggtaccgtgaataatatgaaggacgttctggatgagctgagcagtcgcctgcgtagtcagagcgttccgtggcataatgccggtcgttattggggccacatgaatagcgaaaccctgatgccggcaattctggcctataattatgcaatgctgtggaatggtaacaacgtggcctatgaaagcagcccggcaaccagccagatggaagaagaagttggtctggaatttgccaccctgatgggctataccaatggttggggccatattgttgcagatggtagcctggcaaatctggaaggcctgtggtatgcacgcaatattaagagcctgccgtttgccatgaaagccgttgatccgaccattgttgccggcaaaaccgattgggaactgagtaatatgagcaccaaagaaatcatggacctggttgaagccaatggtgacaaaattgatgagatcaaggccaaaagcgcccgcggcggtaaagatctggataaactgggtaaatggctggttccgcagaccaaacattatagttggctgaaagccgcagatattatcggcattggcctggatcaggttattccggttccggttgatagcaattatcgtatggatatcaacgagctggagaaaattatccgcgaactggcaagtaccgaaaccccgattctgggcgttgtgggcgctgtgggtagtaccgaagaaggtgccgttgatggcattaatgaaattgcagaactgcgtaacaagctggtgaaagaaggtatctatttctacttccacatcgacgccgcctatggtggctatggtcgcgcaattctgctggatgaagataataagctgatcccgtataaggaccttcagagtaaattcgccgaatataacgtgttcaccgaagaagaaaacctggtgagtgaacatacctataactcctatgccgcatttccggaagccgaaagtgttaccattgatccgcataaaatgggctatatcccgtatagtgcaggcggcattgccattcaggatattcgcatgcgtgatgttatcagctatttcgcaacctatgtgttcgaaaagggcgcagatattccggcactgctgggtgcttatattctggaaggcagtaaagcaggcgcaaccgcagccagtgtttgggcagcacataaaaccctgccgctgaatgttaccggttatggtaaactggttggtgcaagcattgaaggcgcccgccgtttttataattttctgagcggcctggaattcaaggtgggcgataaaaccattgaagttcatccgctgaccgatccggattttaatatggttgattacgtgttccaggagaagggcaataataatctggtggaaatgaacgagctgaaccatgaattttacaaccaggcaagctacgttaccggtagcatctatggcaatgaatatctgaccagccataccgatttcgcaattccggattatggtaatagcccgtttaagtttgtgaacaacctgggcgtgaccgaagaaggctggaaagaagcaggtaaagtgaccgttctgcgcgccgctgtgatgacaccttatatgaataaggcagagaacttcgactacttcgccccgaaaattaagcaggccatgcaggaaaaactggaagccatctatgaagatcgtaag

SEQ ID NO: 40 - protein, 621 aa, Artificial sequence
  Engineered sequence
MSNTSFSAKDTDLSALFIGDKAENGQLYKDLLGKLVDEHLGWRQNYMPQDKPMISAEQQTSPEFRGTVNNMKDVLDELSSRLRSQSVPWHNAGRYWGHMNSETLMPAILAYNYAMLWNGNNVAYESSPATSQMEEEVGLEFATLMGYTNGWGHIVADGSLANLEGLWYARNIKSLPFAMKAVDPTIVAGKTDWELSNMSTKEIMDLVEANGDKIDEIKAKSARGGKDLDKLGKWLVPQTKHYSWLKAADIIGIGLDQVIPVPVDSNYRMDINELEKIIRELASTETPILGVVGAVGSTEEGAVDGINEIAELRNKLVKEGIYFYFHIDAAYGGYGRAILLDEDNKLIPYKDLQSKFAEYNVFTEEENLVSEHTYNSYAAFPEAESVTIDPHKMGYIPYSAGGIAIQDIRMRDVISYFATYVFEKGADIPALLGAYILEGSKAGATAASVWAAHKTLPLNVTGYGKLVGASIEGARRFYNFLSGLEFKVGDKTIEVHPLTDPDFNMVDYVFQEKGNNNLVEMNELNHEFYNQASYVTGSIYGNEYLTSHTDFAIPDYGNSPFKFVNNLGVTEEGWKEAGKVTVLRAAVMTPYMNKAENFDYFAPKIKQAMQEKLEAIYEDRK

SEQ ID NO: 41 - DNA, 1863 bp, Artificial sequence
  Engineered sequence
atgagcaacaccagtttcagcgcaaaagataccgatctgagtgcactgtttatcggtgacaaagcagaaaatggtcagctgtataaggacctgctgggcaaactggttgatgaacatctgggttggcgccagaattatatgccgcaggataaaccgatgatcagcgccgaacagcagaccagcccggaatttcgtggtaccgtgaataatatgaaggacgttctggatgagctgagcagtcgcctgcgtagtcagagcgttccgtggcataatgccggtcgttattggggccacatgaatagcgaaaccctgatgccggcaattctggcctataattatgcaatgctgtggaatggtaacaacgtggcctatgaaagcagcccggcaaccagccagatggaagaagaagttggtctggaatttgccaccctgatgggctataccaatggttggggccatattgttgcagatggtagcctggcaaatctggaaggcctgtggtatgcacgcaatattaagagcctgccgtttgccatgaaagccgttgatccgaccattgttgccggcaaaaccgattgggaactgagtaatatgagcaccaaagaaatcatggacctggttgaagccaatggtgacaaaattgatgagatcaaggccaaaagcgcccgcggcggtaaagatctggataaactgggtaaatggctggttccgcagaccaaacattatagttggctgaaagccgcagatattatcggcattggcctggatcaggttattccggttccggttgatagcaattatcgtatggatatcaacgagctggagaaaattatccgcgaactggcaagtaccgaaaccccgattctgggcgttgtgggcgttgtgggtagtaccgaagaaggtgccgttgatggcattaatgaaattgcagaactgcgtaacaagctggtgaaagaaggtatctatttctacttccacatcgacgccgcctatggtggctatggtcgcgcaattctgctggatgaagataataagctgatcccgtataaggaccttcagagtaaattcgccgaatataacgtgttcaccgaagaagaaaacctggtgagtgaacatacctataacgcctatgccgcatttccggaagccgaaagtgttaccactgatccgcataaaatgggctatatcccgtatagtgcaggcggcattgccattcaggatattcgcatgcgtgatgttatcagctatttcgcaacctatgtgttcgaaaagggcgcagatattccggcactgctgggtgcttatattctggaaggcagtaaagcaggcgcaaccgcagccagtgtttgggcagcacataaaaccctgccgctgaatgttaccggttatggtaaactggttggtgcaagcattgaaggcgcccgccgtttttataattttctgagcggcctggaattcaaggtgggcgataaaaccattgaagttcatccgctgaccgatccggattttaatatggttgattacgtgttccaggagaagggcaataataatctggtggaaatgaacgagctgaaccatgaattttacaaccaggcaagctacgttaccggtagcatctatggcaatgaatatctgaccagccataccgatttcgcaattccggattatggtaatagcccgtttaagtttgtgaacaacctgggcgtgaccgaagaaggctggaaagaagcaggtaaagtgaccgttctgcgcgccgctgtgatgacaccttatatgaataaggcagagaacttcgactacttcgccccgaaaattaagcaggccatgcaggaaaaactggaagccatctatgaagatcgtaag

SEQ ID NO: 42 - protein, 621 aa, Artificial sequence
  Engineered sequence
MSNTSFSAKDTDLSALFIGDKAENGQLYKDLLGKLVDEHLGWRQNYMPQDKPMISAEQQTSPEFRGTVNNMKDVLDELSSRLRSQSVPWHNAGRYWGHMNSETLMPAILAYNYAMLWNGNNVAYESSPATSQMEEEVGLEFATLMGYTNGWGHIVADGSLANLEGLWYARNIKSLPFAMKAVDPTIVAGKTDWELSNMSTKEIMDLVEANGDKIDEIKAKSARGGKDLDKLGKWLVPQTKHYSWLKAADIIGIGLDQVIPVPVDSNYRMDINELEKIIRELASTETPILGVVGVVGSTEEGAVDGINEIAELRNKLVKEGIYFYFHIDAAYGGYGRAILLDEDNKLIPYKDLQSKFAEYNVFTEEENLVSEHTYNAYAAFPEAESVTTDPHKMGYIPYSAGGIAIQDIRMRDVISYFATYVFEKGADIPALLGAYILEGSKAGATAASVWAAHKTLPLNVTGYGKLVGASIEGARRFYNFLSGLEFKVGDKTIEVHPLTDPDFNMVDYVFQEKGNNNLVEMNELNHEFYNQASYVTGSIYGNEYLTSHTDFAIPDYGNSPFKFVNNLGVTEEGWKEAGKVTVLRAAVMTPYMNKAENFDYFAPKIKQAMQEKLEAIYEDRK

SEQ ID NO: 43 - DNA, 1863 bp, Artificial sequence
  Engineered sequence
atgagcaacaccagtttcagcgcaaaagataccgatctgagtgcactgtttatcggtgacaaagcagaaaatggtcagctgtataaggacctgctgggcaaactggttgatgaacatctgggttggcgccagaattatatgccgcaggatccgccgatgatcagcgccgaacagcagaccagcccggaatttcgtggtaccgtgaataatatgaaggacgttctggatgagctgagcagtcgcctgcgtagtcagagcgttccgtggcataatgccggtcgttattggggccacatgaatagcgaaaccctgatgccggcaattctggcctataattatgcaatgctgtggaatggtaacaacgtggcctatgaaagcagcccggcaaccagccagatggaagaagaagttggtctggaatttgccaccctgatgggctataccaatggttggggccatattgttgcagatggtagcctggcaaatctggaaggcctgtggtatgcacgcaatattaagagcctgccgtttgccatgaaagccgttgatccgaccattgttgccggcaaaaccgattgggaactgagtaatatgagcaccaaagaaatcatggacctggttgaagccaatggtgacaaaattgatgagatcaaggccaaaagcgcccgcggcggtaaagatctggataaactgggtaaatggctggttccgcagaccaaacattatagttggctgaaagccgcagatattatcggcattggcctggatcaggttattccggttccggttgatagcaattatcgtatggatatcaacgagctggagaaaattatccgcgaactggcaagtaccgaaaccccgattctgggcgttgtgggcgttgtgggtagtaccgaagaaggtgccgttgatggcattaatgaaattgcagaactgcgtaacaagctggtgaaagaaggtatctatttctacttccacatcgacgccgcctatggtggctatggtcgcgcaattctgctggatgaagataataagctgatcccgtataaggaccttcagagtaaattcgccgaatataacgtgttcaccgaagaagaaaacctggtgagtgaacatacctataacgcctatgccgcatttccggaagccgaaagtgttaccattgatccgcataaaatgggctatatcccgtatagtgcaggcggcattgccattcaggatattcgcatgcgtgatgttatcagctatttcgcaacctatgtgttcgaaaagggcgcagatattccggcactgctgggtgcttatattctggaaggcagtaaagcaggcgcaaccgcagccagtgtttgggcagcacataaaaccctgccgctgaatgttaccggttatggtgttctggttggtgcaagcattgaaggcgcccgccgtttttataattttctgagcggcctggaattcaaggtgggcgataaaaccattgaagttcatccgctgaccgatccggattttaatatggttgattacgtgttccaggagaagggcaataataatctggtggaaatgaacgagctgaaccatgaattttacaaccaggcaagctacgttaccggtagcatctatggcaatgaatatctgaccagccataccgatttcgcaattccggattatggtaatagcccgtttaagtttgtgaacaacctgggcgtgaccgaagaaggctggaaagaagcaggtaaagtgaccgttctgcgcgccgctgtgatgacaccttatatgaataaggcagagaacttcgactacttcgccccgaaaattaagcaggccatgcaggaaaaactggaagccatctatgaagatcgtaag

SEQ ID NO: 44 - protein, 621 aa, Artificial sequence
  Engineered sequence
MSNTSFSAKDTDLSALFIGDKAENGQLYKDLLGKLVDEHLGWRQNYMPQDPPMISAEQQTSPEFRGTVNNMKDVLDELSSRLRSQSVPWHNAGRYWGHMNSETLMPAILAYNYAMLWNGNNVAYESSPATSQMEEEVGLEFATLMGYTNGWGHIVADGSLANLEGLWYARNIKSLPFAMKAVDPTIVAGKTDWELSNMSTKEIMDLVEANGDKIDEIKAKSARGGKDLDKLGKWLVPQTKHYSWLKAADIIGIGLDQVIPVPVDSNYRMDINELEKIIRELASTETPILGVVGVVGSTEEGAVDGINEIAELRNKLVKEGIYFYFHIDAAYGGYGRAILLDEDNKLIPYKDLQSKFAEYNVFTEEENLVSEHTYNAYAAFPEAESVTIDPHKMGYIPYSAGGIAIQDIRMRDVISYFATYVFEKGADIPALLGAYILEGSKAGATAASVWAAHKTLPLNVTGYGVLVGASIEGARRFYNFLSGLEFKVGDKTIEVHPLTDPDFNMVDYVFQEKGNNNLVEMNELNHEFYNQASYVTGSIYGNEYLTSHTDFAIPDYGNSPFKFVNNLGVTEEGWKEAGKVTVLRAAVMTPYMNKAENFDYFAPKIKQAMQEKLEAIYEDRK

SEQ ID NO: 45 - DNA, 1863 bp, Artificial sequence
  Engineered sequence
atgagcaacaccagtttcagcgcaaaagataccgatctgagtgcactgtttatcggtgacaaagcagaaaatggtcagctgtataaggacctgctgggcaaactggttgatgaacatctgggttggcgccagaattatatgccgcaggatccgccgatgatcagcgccgaacagcagaccagcccggaatttcgtggtaccgtgaataatatgaaggacgttctggatgagctgagcagtcgcctgcgtagtcagagcgttccgtggcataatgccggtcgttattggggccacatgaatagcgaaaccctgatgccggcaattctggcctataattatgcaatgctgtggaatggtaacaacgtggcctatgaaagcagcccggcaaccagccagatggaagaagaagttggtctggaatttgccaccctgatgggctataccaatggttggggccatattgttgcagatggtagcctggcaaatctggaaggcctgtggtatgcacgcaatattaagagcctgccgtttgccatgaaagccgttgatccgaccattgttgccggcaaaaccgattgggaactgagtaatatgagcaccaaagaaatcatggacctggttgaagccaatggtgacaaaattgatgagatcaaggccaaaagcgcccgcggcggtaaagatctggataaactgggtaaatggctggttccgcagaccaaacattatagttggctgaaagccgcagatattatcggcattggcctggatcaggttattccggttccggttgatagcaattatcgtatggatatcaacgagctggagaaaattatccgcgaactggcaagtaccgaaaccccgattctgggcgttgtgggcgttgtgggtagtaccgaagaaggtgccgttgatggcattaatgaaattgcagaactgcgtaacaagctggtgaaagaaggtatctatttctacttccacatcgacgccgcctatggtggctatggtcgcgcaattctgctggatgaagataataagctgatcccgtataaggaccttcagagtaaattcgccgaatataacgtgttcaccgaagaagaaaacctggtgagtgaacatacctataacgcctatgccgcatttccggaagccgaaagtgttaccattgatccgcataaaatgggctatatcccgtatagtgcaggcggcattgccattcaggatattcgcatgcgtgatgttatcagctatttcgcaacctatgtgttcgaaaagggcgcagatattccggcactgctgggtgcttatattctggaaggcagtaaagcaggcgcaaccgcagccagtgtttgggcagcacataaaaccctgccgctgaatgttaccggttatggtaaactgctgggtgcaagcattgaaggcgcccgccgtttttataattttctgagcggcctggaattcaaggtgggcgataaaaccattgaagttcatccgctgaccgatccggattttaatatggttgattacgtgttccaggagaagggcaataataatctggtggaaatgaacgagctgaaccatgaattttacaaccaggcaagctacgttaccggtagcatctatggcaatgaatatctgaccagccataccgatttcgcaattccggattatggtaatagcccgtttaagtttgtgaacaacctgggcgtgaccgaagaaggctggaaagaagcaggtaaagtgaccgttctgcgcgccgctgtgatgacaccttatatgaataaggcagagaacttcgactacttcgccccgaaaattaagcaggccatgcaggaaaaactggaagccatctatgaagatcgtaag

SEQ ID NO: 46 - protein, 621 aa, Artificial sequence
  Engineered sequence
MSNTSFSAKDTDLSALFIGDKAENGQLYKDLLGKLVDEHLGWRQNYMPQDPPMISAEQQTSPEFRGTVNNMKDVLDELSSRLRSQSVPWHNAGRYWGHMNSETLMPAILAYNYAMLWNGNNVAYESSPATSQMEEEVGLEFATLMGYTNGWGHIVADGSLANLEGLWYARNIKSLPFAMKAVDPTIVAGKTDWELSNMSTKEIMDLVEANGDKIDEIKAKSARGGKDLDKLGKWLVPQTKHYSWLKAADIIGIGLDQVIPVPVDSNYRMDINELEKIIRELASTETPILGVVGVVGSTEEGAVDGINEIAELRNKLVKEGIYFYFHIDAAYGGYGRAILLDEDNKLIPYKDLQSKFAEYNVFTEEENLVSEHTYNAYAAFPEAESVTIDPHKMGYIPYSAGGIAIQDIRMRDVISYFATYVFEKGADIPALLGAYILEGSKAGATAASVWAAHKTLPLNVTGYGKLLGASIEGARRFYNFLSGLEFKVGDKTIEVHPLTDPDFNMVDYVFQEKGNNNLVEMNELNHEFYNQASYVTGSIYGNEYLTSHTDFAIPDYGNSPFKFVNNLGVTEEGWKEAGKVTVLRAAVMTPYMNKAENFDYFAPKIKQAMQEKLEAIYEDRK

SEQ ID NO: 47 - DNA, 1863 bp, Artificial sequence
  Engineered sequence
atgagcaacaccagtttcagcgcaaaagataccgatctgagtgcactgtttatcggtgacaaagcagaaaatggtcagctgtataaggacctgctgggcaaactggttgatgaacatctgggttggcgccagaattatatgccgcaggatccgccgatgatcagcgccgaacagcagaccagcccggaatttcgtggtaccgtgaataatatgaaggacgttctggatgagctgagcagtcgcctgcgtagtcagagcgttccgtggcataatgccggtcgttattggggccacatgaatagcgaaaccctgatgccggcaattctggcctataattatgcaatgctgtggaatggtaacaacgtggcctatgaaagcagcccggcaaccagccagatggaagaagaagttggtctggaatttgccaccctgatgggctataccaatggttggggccatattgttgcagatggtagcctggcaaatctggaaggcctgtggtatgcacgcaatattaagagcctgccgtttgccatgaaagccgttgatccgaccattgttgccggcaaaaccgattgggaactgagtaatatgagcaccaaagaaatcatggacctggttgaagccctgggtgacaaaattgatgagatcaaggccaaaagcgcccgcggcggtaaagatctggataaactgggtaaatggctggttccgcagaccaaacattatagttggctgaaagccgcagatattatcggcattggcctggatcaggttattccggttccggttgatagcaattatcgtatggatatcaacgagctggagaaaattatccgcgaactggcaagtaccgaaaccccgattctgggcgttgtgggcgttgtgggtagtaccgaagaaggtgccgttgatggcattaatgaaattgcagaactgcgtaacaagctggtgaaagaaggtatctatttctacttccacatcgacgccgcctatggtggctatggtcgcgcaattctgctggatgaagataataagctgatcccgtataaggaccttcagagtaaattcgccgaatataacgtgttcaccgaagaagaaaacctggtgagtgaacatacctataacgcctatgccgcatttccggaagccgaaagtgttaccattgatccgcataaaatgggctatatcccgtatagtgcaggcggcattgccattcaggatattcgcatgcgtgatgttatcagctatttcgcaacctatgtgttcgaaaagggcgcagatattccggcactgctgggtgcttatattctggaaggcagtaaagcaggcgcaaccgcagccagtgtttgggcagcacataaaaccctgccgctgaatgttaccggttatggtaaactggttggtgcaagcattgaaggcgcccgccgtttttataattttctgagcggcctggaattcaaggtgggcgataaaaccattgaagttcatccgctgaccgatccggattttaatatggttgattacgtgttccaggagaagggcaataataatctggtggaaatgaacgagctgaaccatgaattttacgaccaggcaagctacgttaccggtagcatctatggcaatgaatatctgaccagccataccgatttcgcaattccggattatggtaatagcccgtttaagtttgtgaacaacctgggcgtgaccgaagaaggctggaaagaagcaggtaaagtgaccgttctgcgcgccgctgtgatgacaccttatatgaataaggcagagaacttcgactacttcgccccgaaaattaagcaggccatgcaggaaaaactggaagccatctatgaagatcgtaag

SEQ ID NO: 48 - protein, 621 aa, Artificial sequence
  Engineered sequence
MSNTSFSAKDTDLSALFIGDKAENGQLYKDLLGKLVDEHLGWRQNYMPQDPPMISAEQQTSPEFRGTVNNMKDVLDELSSRLRSQSVPWHNAGRYWGHMNSETLMPAILAYNYAMLWNGNNVAYESSPATSQMEEEVGLEFATLMGYTNGWGHIVADGSLANLEGLWYARNIKSLPFAMKAVDPTIVAGKTDWELSNMSTKEIMDLVEALGDKIDEIKAKSARGGKDLDKLGKWLVPQTKHYSWLKAADIIGIGLDQVIPVPVDSNYRMDINELEKIIRELASTETPILGVVGVVGSTEEGAVDGINEIAELRNKLVKEGIYFYFHIDAAYGGYGRAILLDEDNKLIPYKDLQSKFAEYNVFTEEENLVSEHTYNAYAAFPEAESVTIDPHKMGYIPYSAGGIAIQDIRMRDVISYFATYVFEKGADIPALLGAYILEGSKAGATAASVWAAHKTLPLNVTGYGKLVGASIEGARRFYNFLSGLEFKVGDKTIEVHPLTDPDFNMVDYVFQEKGNNNLVEMNELNHEFYDQASYVTGSIYGNEYLTSHTDFAIPDYGNSPFKFVNNLGVTEEGWKEAGKVTVLRAAVMTPYMNKAENFDYFAPKIKQAMQEKLEAIYEDRK

SEQ ID NO: 49 - DNA, 1863 bp, Artificial sequence
  Engineered sequence
atgagcaacaccagtttcagcgcaaaagataccgatctgagtgcactgtttatcggtgacaaagcagaaaatggtcagctgtataaggacctgctgggcaaactggttgatgaacatctgggttggcgccagaattatatgccgcaggatccgccgatgatcagcgccgaacagcagaccagcccggaatttcgtggtaccgtgaataatatgaaggacgttctggatgagctgagcagtcgcctgcgtagtcagagcgttccgtggcataatgccggtcgttattggggccacatgaatagcgaaaccctgatgccggcaattctggcctataattatgcaatgctgtggaatggtaacaacgtggcctatgaaagcagcccggcaaccagccagatggaagaagaagttggtctggaatttgccaccctgatgggctataccaatggttggggccatattgttgcagatggtagcctggcaaatctggaaggcctgtggtatgcacgcaatattaagagcctgccgtttgccatgaaagccgttgatccgaccattgttgccggcaaaaccgattgggaactgagtaatatgagcaccaaagaaatcatggacctggttgaagccaatggtgacaaaattgatgagatcaaggccaaaagcgcccgcggcggtaaagatctggataaactgggtaaatggctggttccgcagaccaaacattatagttggctgaaagccgcagatattatcggcattggcctggatcaggttattccggttccggttgatagcaattatcgtatggatatcaacgagctggagaaaattatccgcgaactggcaagtaccgaaaccccgattctgggcgttgtgggcgcggtgggtagtaccgaagaaggtgccgttgatggcattaatgaaattgcagaactgcgtaacaagctggtgaaagaaggtatctatttctacttccacatcgacgccgcctatggtggctatggtcgcgcaattctgctggatgaagataataagctgatcccgtataaggaccttcagagtaaattcgccgaatataacgtgttcaccgaagaagaaaacctggtgagtgaacatacctataacgcctatgccgcatttccggaagccgaaagtgttaccattgatccgcataaaatgggctatatcccgtatagtgcaggcggcattgccattcaggatattcgcatgcgtgatgttatcagctatttcgcaacctatgtgttcgaaaagggcgcagatattccggcactgctgggtgcttatattctggaaggcagtaaagcaggcgcaaccgcagccagtgtttgggcagcacataaaaccctgccgctgaatgttaccggttatggtaaactggttggtgcaagcattgaaggcgcccgccgtttttataattttctgagcggcctggaattcaaggtgggcgataaaaccattgaagttcatccgctgaccgatccggattttaatatggttgattacgtgttccaggagaagggcaataataatctggtggaaatgaacgagctgaaccatgaattttacaaccaggcaagctactggaccggtagcatctatggcaatgaatatctgaccagccataccgatttcgcaattccggattatggtaatagcccgtttaagtttgtgaacaacctgggcgtgaccgaagaaggctggaaagaagcaggtaaagtgaccgttctgcgcgccgctgtgatgacaccttatatgaataaggcagagaacttcgactacttcgccccgaaaattaagcaggccatgcaggaaaaactggaagccatctatgaagatcgtaag

SEQ ID NO: 50 - protein, 621 aa, Artificial sequence
  Engineered sequence
MSNTSFSAKDTDLSALFIGDKAENGQLYKDLLGKLVDEHLGWRQNYMPQDPPMISAEQQTSPEFRGTVNNMKDVLDELSSRLRSQSVPWHNAGRYWGHMNSETLMPAILAYNYAMLWNGNNVAYESSPATSQMEEEVGLEFATLMGYTNGWGHIVADGSLANLEGLWYARNIKSLPFAMKAVDPTIVAGKTDWELSNMSTKEIMDLVEANGDKIDEIKAKSARGGKDLDKLGKWLVPQTKHYSWLKAADIIGIGLDQVIPVPVDSNYRMDINELEKIIRELASTETPILGVVGAVGSTEEGAVDGINEIAELRNKLVKEGIYFYFHIDAAYGGYGRAILLDEDNKLIPYKDLQSKFAEYNVFTEEENLVSEHTYNAYAAFPEAESVTIDPHKMGYIPYSAGGIAIQDIRMRDVISYFATYVFEKGADIPALLGAYILEGSKAGATAASVWAAHKTLPLNVTGYGKLVGASIEGARRFYNFLSGLEFKVGDKTIEVHPLTDPDFNMVDYVFQEKGNNNLVEMNELNHEFYNQASYWTGSIYGNEYLTSHTDFAIPDYGNSPFKFVNNLGVTEEGWKEAGKVTVLRAAVMTPYMNKAENFDYFAPKIKQAMQEKLEAIYEDRK

SEQ ID NO: 51 - DNA, 1863 bp, Artificial sequence
  Engineered sequence
atgagcaacaccagtttcagcgcaaaagataccgatctgagtgcactgtttatcggtgacaaagcagaaaatggtcagctgtataaggacctgctgggcaaactggttgatgaacatctgggttggcgccagaattatatgccgcaggatccgccgatgatcagcgccgaacagcagaccagcccggaatttcgtggtaccgtgaataatatgaaggacgttctggatgagctgagcagtcgcctgcgtagtcagagcgttccgtggcataatgccggtcgttattggggccacatgaatagcgaaaccctgatgccggcaattctggcctataattatgcaatgctgtggaatggtaacaacgtggcctatgaaagcagcccggcaaccagccagatggaagaagaagttggtctggaatttgccaccctgatgggctataccaatggttggggccatattgttgcagatggtagcctggcaaatctggaaggcctgtggtatgcacgcaatattaagagcctgccgtttgccatgaaagccgttgatccgaccattgttgccggcaaaaccgattgggaactgagtaatatgagcaccaaagaaatcatggacctggttgaagccaatggtgacaaaattgatgagatcaaggccaaaagcgcccgcggcggtaaagatctggataaactgggtaaatggctggttccgcagaccaaacattatagttggctgaaagccgcagatattatcggcattggcctggatcaggttattccggttccggttgatagcaattatcgtatggatatcaacgagctggagaaaattatccgcgaactggcaagtaccgaaaccccgattctgggcgttgtgggcgttgtgggtagtaccgaagaaggtgccgttgatggcattaatgaaattgcagaactgcgtaacaagctggtgaaagaaggtatctatttctacttccacatcgacgccgcctatggtggctatggtcgcgcaattctgctggatgaagataataagctgatcccgtataaggaccttcagagtaaattcgccgaatataacgtgttcaccgaagaagaaaacctggtgagtgaacatacctataacgcctatgccgcatttccggaagccgaaagtgttaccattgatccgcataaaatgggctatatcccgtatagtgcaggcggcattgccattcaggatattcgcatgcgtgatgttatcagctatttcgcaacctatgtgttcgaaaagggcgcagatattccggcactgctgggtgcttatattctggaaggcagtaaagcaggcgcaaccgcagccagtgtttgggcagcacataaaaccctgccgctgaatgttaccggttatggtaaactggttggtgcaagcattgaaggcgcccgccgtttttataattttctgagcggcctggaattcaaggtgggcgataaaaccattgaagttcatccgctgaccgatccggattttaatatggttgattacgtgttccaggagaagggcaataataatctggtggaaatgaacgagctgaaccatgaattttacgaccaggcaagctacgttaccggtagcatctatggcaatgaatatctgaccagccataccgatttcgcaattccggattatggtaatagcccgtttaagtttgtgaacaacctgggcgtgaccgaagaaggctggaaagaagcaggtaaagtgaccgttctgcgcgccgctgtgatgacaccttatatgaataaggcagagaacttcgactacttcgccccgaaaattaagcaggccatgcaggaaaaactggaagccatctatgaagatcgtaag

SEQ ID NO: 52 - protein, 621 aa, Artificial sequence
  Engineered sequence
MSNTSFSAKDTDLSALFIGDKAENGQLYKDLLGKLVDEHLGWRQNYMPQDPPMISAEQQTSPEFRGTVNNMKDVLDELSSRLRSQSVPWHNAGRYWGHMNSETLMPAILAYNYAMLWNGNNVAYESSPATSQMEEEVGLEFATLMGYTNGWGHIVADGSLANLEGLWYARNIKSLPFAMKAVDPTIVAGKTDWELSNMSTKEIMDLVEANGDKIDEIKAKSARGGKDLDKLGKWLVPQTKHYSWLKAADIIGIGLDQVIPVPVDSNYRMDINELEKIIRELASTETPILGVVGVVGSTEEGAVDGINEIAELRNKLVKEGIYFYFHIDAAYGGYGRAILLDEDNKLIPYKDLQSKFAEYNVFTEEENLVSEHTYNAYAAFPEAESVTIDPHKMGYIPYSAGGIAIQDIRMRDVISYFATYVFEKGADIPALLGAYILEGSKAGATAASVWAAHKTLPLNVTGYGKLVGASIEGARRFYNFLSGLEFKVGDKTIEVHPLTDPDFNMVDYVFQEKGNNNLVEMNELNHEFYDQASYVTGSIYGNEYLTSHTDFAIPDYGNSPFKFVNNLGVTEEGWKEAGKVTVLRAAVMTPYMNKAENFDYFAPKIKQAMQEKLEAIYEDRK

SEQ ID NO: 53 - DNA, 1863 bp, Artificial sequence
  Engineered sequence
atgagcaacaccagtttcagcgcaaaagataccgatctgagtgcactgtttatcggtgacaaagcagaaaatggtcagctgtataaggacctgctgggcaaactggttgatgaacatctgggttggcgccagaattatatgccgcaggatccgccgatgatcagcgccgaacagcagaccagcccggaatttcgtggtaccgtgaataatatgaaggacgttctggatgagctgagcagtcgcctgcgtagtcaaagcgttccgtggcataatgccggtcgttattggggccacatgaatagcgaaaccctgatgccggcaattctggcctataattatgcaatgctgtggaatggtaacaacgtggcctatgaaagcagcccggcaaccagccagatggaagaagaagttggtctggaatttgccaccctgatgggctataccaatggttggggccatattgttgcagatggtagcctggcaaatctggaaggcctgtggtatgcacgcaatattaagagcctgccgtttgccatgaaagccgttgatccgaccattgttgccggcaaaaccgattgggaactgagtaatatgagcaccaaagaaatcatggacctggttgaagccaatggtgacaaaattgatgagatcaaggccaaaagcgcccgcggcggtaaagatctggataaactgggtaaatggctggttccgcagaccaaacattatagttggctgaaagccgcagatattatcggcattggcctggatcaggttattccggttccggttgatagcaattatcgtatggatatcaacgagctggagaaaattatccgcgaactggcaagtaccgaaaccccgattctgggcgttgtgggcgcggtgggtagtaccgaagaaggtgccgttgatggcattaatgaaattgcagaactgcgtaacaagctggtgaaagaaggtatctatttctacttccacatcgacgccgcctatggtggctatggtcgcgcaattctgctggatgaagataataagctgatcccgtataaggaccttcagagtaaattcgccgaatataacgtgttcaccgaagaagaaaacctggtgagtgaacatacctataacgcctatgccgcatttccggaagccgaaagtgttaccattgatccgcataaaatgggctatatcccgtatagtgcaggcggcattgccattcaggatattcgcatgcgtgatgttatcagctatttcgcaacctatgtgttcgaaaagggcgcagatattccggcactgctgggtgcttatattctggaaggcagtaaagcaggcgcaaccgcagccagtgtttgggcagcacataaaaccctgccgctgaatgttaccggttatggtaaactggttggtgcaagcattgaaggcgcccgccgtttttataattttctgagcggcctggaattcaaggtgggcgataaaaccattgaagttcatccgctgaccgatccggattttaatatggttgattacgtgttccaggagaagggcaataataatctggtggaaatgaacgagctgaaccatgaattttacaaccaggcaagctacgttaccggtagcatctatggcaatgaatatctgaccagccataccgatttcgcaattccggattatggtaatagcccgtttaagtttgtgaacaacctgggcgtgaccgaagaaggctggaaagaagcaggtaaagtgaccgttctgcgcgccgctgtgatgacaccttatatgaataaggcagagaacttcgactacttcgccccgaaaattaagcaggccatgcaggaaaaactggaagccatctatgaagatcgtaag

SEQ ID NO: 54 - protein, 621 aa, Artificial sequence
  Engineered sequence
MSNTSFSAKDTDLSALFIGDKAENGQLYKDLLGKLVDEHLGWRQNYMPQDPPMISAEQQTSPEFRGTVNNMKDVLDELSSRLRSQSVPWHNAGRYWGHMNSETLMPAILAYNYAMLWNGNNVAYESSPATSQMEEEVGLEFATLMGYTNGWGHIVADGSLANLEGLWYARNIKSLPFAMKAVDPTIVAGKTDWELSNMSTKEIMDLVEANGDKIDEIKAKSARGGKDLDKLGKWLVPQTKHYSWLKAADIIGIGLDQVIPVPVDSNYRMDINELEKIIRELASTETPILGVVGAVGSTEEGAVDGINEIAELRNKLVKEGIYFYFHIDAAYGGYGRAILLDEDNKLIPYKDLQSKFAEYNVFTEEENLVSEHTYNAYAAFPEAESVTIDPHKMGYIPYSAGGIAIQDIRMRDVISYFATYVFEKGADIPALLGAYILEGSKAGATAASVWAAHKTLPLNVTGYGKLVGASIEGARRFYNFLSGLEFKVGDKTIEVHPLTDPDFNMVDYVFQEKGNNNLVEMNELNHEFYNQASYVTGSIYGNEYLTSHTDFAIPDYGNSPFKFVNNLGVTEEGWKEAGKVTVLRAAVMTPYMNKAENFDYFAPKIKQAMQEKLEAIYEDRK

SEQ ID NO: 55 - DNA, 1863 bp, Artificial sequence
  Engineered sequence
atgagcaacaccagtttcagcgcaaaagataccgatctgagtgcactgtttatcggtgacaaagcagaaaatggtcagctgtataaggacctgctgggcaaactggttgatgaacatctgggttggcgccagaattatatgccgcaggatccgccgatgatcagcgccgaacagcagaccagcccggaatttcgtggtaccgtgaataatatgaaggacgttctggatgagctgagcagtcgcctgcgtagtcagagcgttccgtggcataatgccggtcgttattggggccacatgaatagcgaaaccctgatgccggcaattctggcctataattatgcaatgctgtggaatggtaacaacgtggcctatgaaagcagcccggcaaccagccagatggaagaagaagttggtctggaatttgccaccctgatgggctataccaatggttggggccatattgttgcagatggtagcctggcaaatctggaaggcctgtggtatgcacgcaatattaagagcctgccgtttgccatgaaagccgttgatccgaccattgttgccggcaaaaccgattgggaactgagtaatatgagcaccaaagaaatcatggacctggttgaagccctgggtgacaaaattgatgagatcaaggccaaaagcgcccgcggcggtaaagatctggataaactgggtaaatggctggttccgcagaccaaacattatagttggctgaaagccgcagatattatcggcattggcctggatcaggttattccggttccggttgatagcaattatcgtatggatatcaacgagctggagaaaattatccgcgaactggcaagtaccgaaaccccgattctgggcgttgtgggcgcggtgggtagtaccgaagaaggtgccgttgatggcattaatgaaattgcagaactgcgtaacaagctggtgaaagaaggtatctatttctacttccacatcgacgccgcctatggtggctatggtcgcgcaattctgctggatgaagataataagctgatcccgtataaggaccttcagagtaaattcgccgaatataacgtgttcaccgaagaagaaaacctggtgagtgaacatacctataacgcctatgccgcatttccggaagccgaaagtgttaccattgatccgcataaaatgggctatatcccgtatagtgcaggcggcattgccattcaggatattcgcatgcgtgatgttatcagctatttcgcaacctatgtgttcgaaaagggcgcagatattccggcactgctgggtgcttatattctggaaggcagtaaagcaggcgcaaccgcagccagtgtttgggcagcacataaaaccctgccgctgaatgttaccggttatggtaaactggttggtgcaagcattgaaggcgcccgccgtttttataattttctgagcggcctggaattcaaggtgggcgataaaaccattgaagttcatccgctgaccgatccggattttaatatggttgattacgtgttccaggagaagggcaataataatctggtggaaatgaacgagctgaaccatgaattttacaaccaggcaagctactggaccggtagcatctatggcaatgaatatctgaccagccataccgatttcgcaattccggattatggtaatagcccgtttaagtttgtgaacaacctgggcgtgaccgaagaaggctggaaagaagcaggtaaagtgaccgttctgcgcgccgctgtgatgacaccttatatgaataaggcagagaacttcgactacttcgccccgaaaattaagcaggccatgcaggaaaaactggaagccatctatgaagatcgtaag

SEQ ID NO: 56 - protein, 621 aa, Artificial sequence
  Engineered sequence
MSNTSFSAKDTDLSALFIGDKAENGQLYKDLLGKLVDEHLGWRQNYMPQDPPMISAEQQTSPEFRGTVNNMKDVLDELSSRLRSQSVPWHNAGRYWGHMNSETLMPAILAYNYAMLWNGNNVAYESSPATSQMEEEVGLEFATLMGYTNGWGHIVADGSLANLEGLWYARNIKSLPFAMKAVDPTIVAGKTDWELSNMSTKEIMDLVEALGDKIDEIKAKSARGGKDLDKLGKWLVPQTKHYSWLKAADIIGIGLDQVIPVPVDSNYRMDINELEKIIRELASTETPILGVVGAVGSTEEGAVDGINEIAELRNKLVKEGIYFYFHIDAAYGGYGRAILLDEDNKLIPYKDLQSKFAEYNVFTEEENLVSEHTYNAYAAFPEAESVTIDPHKMGYIPYSAGGIAIQDIRMRDVISYFATYVFEKGADIPALLGAYILEGSKAGATAASVWAAHKTLPLNVTGYGKLVGASIEGARRFYNFLSGLEFKVGDKTIEVHPLTDPDFNMVDYVFQEKGNNNLVEMNELNHEFYNQASYWTGSIYGNEYLTSHTDFAIPDYGNSPFKFVNNLGVTEEGWKEAGKVTVLRAAVMTPYMNKAENFDYFAPKIKQAMQEKLEAIYEDRK

SEQ ID NO: 57 - DNA, 1863 bp, Artificial sequence
  Engineered sequence
atgagcaacaccagtttcagcgcaaaagataccgatctgagtgcactgtttatcggtgacaaagcagaaaatggtcagctgtataaggacctgctgggcaaactggttgatgaacatctgggttggcgccagaattatatgccgcaggatccgccgatgatcagcgccgaacagcagaccagcccggaatttcgtggtaccgtgaataatatgaaggacgttctggatgagctgagcagtcgcctgcgtagtcagagcgttccgtggcataatgccggtcgttattggggccacatgaatagcgaaaccctgatgccggcaattctggcctataattatgcaatgctgtggaatggtaacaacgtggcctatgaaagcagcccggcaaccagccagatggaagaagaagttggtctggaatttgccaccctgatgggctataccaatggttggggccatattgttgcagatggtagcctggcaaatctggaaggcctgtggtatgcacgcaatattaagagcctgccgtttgccatgaaagccgttgatccgaccattgttgccggcaaaaccgattgggaactgagtaatatgagcaccaaagaaatcatggacctggttgaagccaatggtgacaaaattgatgagatcaaggccaaaagcgcccgcggcggtaaagatctggataaactgggtaaatggctggttccgcagaccaaacattatagttggctgaaagccgcagatattatcggcattggcctggatcaggttattccggttccggttgatagcaattatcgtatggatatcaacgagctggagaaaattatccgcgaactggcaagtaccgaaaccccgattctgggcgttgtgggcgttgtgggtagtaccgaagaaggtgccgttgatggcattaatgaaattgcagaactgcgtaacaagctggtgaaagaaggtatctatttctacttccacatcgacgccgcctatggtggctatggtcgcgcaattctgctggatgaagataataagctgatcccgtataaggaccttcagagtaaattcgccgaatataacgtgttcaccgaagaagaaaacctggtgagtgaacatacctataacgcctatgccgcatttccggaagccgaaagtgttaccaccgatccgcataaaatgggctatatcccgtatagtgcaggcggcattgccattcaggatattcgcatgcgtgatgttatcagctatttcgcaacctatgtgttcgaaaagggcgcagatattccggcactgctgggtgcttatattctggaaggcagtaaagcaggcgcaaccgcagccagtgtttgggcagcacataaaaccctgccgctgaatgttaccggttatggtaaactggttggtgcaagcattgaaggcgcccgccgtttttataattttctgagcggcctggaattcaaggtgggcgataaaaccattgaagttcatccgctgaccgatccggattttaatatggttgattacgtgttccaggagaagggcaataataatctggtggaaatgaacgagctgaaccatgaattttacaaccaggcaagctacgttaccggtagcatctatggcaatgaatatctgaccagccataccgatttcgcaattccggattatggtaatagcccgtttaagtttgtgaacaacctgggcgtgaccgaagaaggctggaaagaagcaggtaaagtgaccgttctgcgcgccgctgtgatgacaccttatatgaataaggcagagaacttcgactacttcgccccgaaaattaagcaggccatgcaggaaaaactggaagccatctatgaagatcgtaag

SEQ ID NO: 58 - protein, 621 aa, Artificial sequence
  Engineered sequence
MSNTSFSAKDTDLSALFIGDKAENGQLYKDLLGKLVDEHLGWRQNYMPQDPPMISAEQQTSPEFRGTVNNMKDVLDELSSRLRSQSVPWHNAGRYWGHMNSETLMPAILAYNYAMLWNGNNVAYESSPATSQMEEEVGLEFATLMGYTNGWGHIVADGSLANLEGLWYARNIKSLPFAMKAVDPTIVAGKTDWELSNMSTKEIMDLVEANGDKIDEIKAKSARGGKDLDKLGKWLVPQTKHYSWLKAADIIGIGLDQVIPVPVDSNYRMDINELEKIIRELASTETPILGVVGVVGSTEEGAVDGINEIAELRNKLVKEGIYFYFHIDAAYGGYGRAILLDEDNKLIPYKDLQSKFAEYNVFTEEENLVSEHTYNAYAAFPEAESVTTDPHKMGYIPYSAGGIAIQDIRMRDVISYFATYVFEKGADIPALLGAYILEGSKAGATAASVWAAHKTLPLNVTGYGKLVGASIEGARRFYNFLSGLEFKVGDKTIEVHPLTDPDFNMVDYVFQEKGNNNLVEMNELNHEFYNQASYVTGSIYGNEYLTSHTDFAIPDYGNSPFKFVNNLGVTEEGWKEAGKVTVLRAAVMTPYMNKAENFDYFAPKIKQAMQEKLEAIYEDRK

SEQ ID NO: 59 - DNA, 1863 bp, Artificial sequence
  Engineered sequence
atgagcaacaccagtttcagcgcaaaagataccgatctgagtgcactgtttatcggtgacaaagcagaaaatggtcagctgtataaggaactgctgggcaaactggttgatgaacatctgggttggcgccagaattatatgccgcaggatccgtcgatgatcagcgccgaacagcagaccagcccggaatttcgtggtaccgtgaataatatgcgtgacgttctggatgagctgagcagtcgcctgcgtagtcagagcgttccgtggcataatgccggtcgttattggggccacatgaatagcgaaaccctgatgccggcaattctggcctataattatgcaatgctgtggaatggtaacaacgtggcctatgaaagcagcccggcaaccagccagatggaagaagaagttggtctggaatttgccaccctgatgggctataccaatggttggggccatattgttgcagatggtagcctggcaaatctggaaggcctgtggtatgcacgcaatattaagagcctgccgtttgccatgaaagccgttgatccgaccattgttgccggcaaaaccgattgggaactgagtaatatgagcaccaaagaaatcatggacctggttgaagccaatggtgacaaaattgatgagatcaaggccaaaagcgcccgcggcggtaaagatctggataaactgggtaaatggctggttccgcagaccaaacattatagttggctgaaagccgcagatattatcggcattggcctggatcaggttattccggttccggttgatagcaattatcgtatggatatcaacgagctggagaaaattatccgcgaactggcaagtaccgaaaccccgattctgggcgttgtgggcgttgtgggtagtaccgaagaaggtgccgttgatggcattaatgaaattgcagaactgcgtaacaagctggtgaaagaaggtatctatttctacttccacatcgacgccgcctatggtggctatggtcgcgcaattctgctggatgaagataataagctgatcccgtataaggaccttcagagtaaattcgccgaatataacgtgttcaccgaagaagaaaacctggtgagtgaacatacctataacgcctatgccgcatttccggaagccgaaagtgttaccattgatccgcataaaatgggctatatcccgtatagtgcaggcggcattgccattcaggatattcgcatgcgtgatgttatcagctatttcgcaacctatgtgttcgaaaagggcgcagatattccggcactgctgggtgcttatattctggaaggcagtaaagcaggcgcaaccgcagccagtgtttgggcagcacataaaaccctgccgctgaatgttaccggttatggtaaactggttggtgcaagcattgaaggcgcccgccgtttttataattttctgagcggcctggaattcaaggtgggcgataaaaccattgaagttcatccgctgaccgatccggattttaatatggttgattacgtgttccaggagaagggcaataataatctggtggaaatgaacgagctgaaccatgaattttacaaccaggcaagctacgttaccggtagcatctatggcaatgaatatctgaccagccataccgatttcgcaattccggattatggtaatagcccgtttaagtttgtgaacaacctgggcgtgaccgaagaaggctggaaagaagcaggtaaagtgaccgttctgcgcgccgctgtgatgacaccttatatgaataaggcagagaacttcgactacttcgccccgaaaattaagcaggccatgcaggaaaaactggaagccatctatgaagatcgtaag

SEQ ID NO: 60 - protein, 621 aa, Artificial sequence
  Engineered sequence
MSNTSFSAKDTDLSALFIGDKAENGQLYKELLGKLVDEHLGWRQNYMPQDPSMISAEQQTSPEFRGTVNNMRDVLDELSSRLRSQSVPWHNAGRYWGHMNSETLMPAILAYNYAMLWNGNNVAYESSPATSQMEEEVGLEFATLMGYTNGWGHIVADGSLANLEGLWYARNIKSLPFAMKAVDPTIVAGKTDWELSNMSTKEIMDLVEANGDKIDEIKAKSARGGKDLDKLGKWLVPQTKHYSWLKAADIIGIGLDQVIPVPVDSNYRMDINELEKIIRELASTETPILGVVGVVGSTEEGAVDGINEIAELRNKLVKEGIYFYFHIDAAYGGYGRAILLDEDNKLIPYKDLQSKFAEYNVFTEEENLVSEHTYNAYAAFPEAESVTIDPHKMGYIPYSAGGIAIQDIRMRDVISYFATYVFEKGADIPALLGAYILEGSKAGATAASVWAAHKTLPLNVTGYGKLVGASIEGARRFYNFLSGLEFKVGDKTIEVHPLTDPDFNMVDYVFQEKGNNNLVEMNELNHEFYNQASYVTGSIYGNEYLTSHTDFAIPDYGNSPFKFVNNLGVTEEGWKEAGKVTVLRAAVMTPYMNKAENFDYFAPKIKQAMQEKLEAIYEDRK

SEQ ID NO: 61 - DNA, 1863 bp, Artificial sequence
  Engineered sequence
atgagcaacaccagtttcagcgcaaaagataccgatctgagtgcactgtttatcggtgacaaagcagaaaatggtcagctgtataaggaactgctgggcaaactggttgatgaacatctgggttggcgccagaattatatgccgcaggatccgccgatgatcagcgccgaacagcagaccagcccggaatttcgtggtaccgtgaataatatgcgtgacgttctggatgagctgagcagtcgcctgcgtagtcagagcgttccgtggcataatgccggtcgttattggggccacatgaatagcgaaaccctgatgccggcaattctggcctataattatgcaatgctgtggaatggtaacaacgtggcctatgaaagcagcccggcaaccagccagatggaagaagaagttggtctggaatttgccaccctgatgggctataccaatggttggggccatattgttgcagatggtagcctggcaaatctggaaggcctgtggtatgcacgcaatattaagagcctgccgtttgccatgaaagccgttgatccgaccattgttgccggcaaaaccgattgggaactgagtaatatgagcaccaaagaaatcatggacctggttgaagccaatggtgacaaaattgatgagatcaaggccaaaagcgcccgcggcggtaaagatctggataaactgggtaaatggctggttccgcagaccaaacattatagttggctgaaagccgcagatattatcggcattggcctggatcaggttattccggttccggttgatagcaattatcgtatggatatcaacgagctggagaaaattatccgcgaactggcaagtaccgaaaccccgattctgggcgttgtgggcgttgtgggtagtaccgaagaaggtgccgttgatggcattaatgaaattgcagaactgcgtaacaagctggtgaaagaaggtatctatttctacttccacatcgacgccgcctatggtggctatggtcgcgcaattctgctggatgaagataataagctgatcccgtataaggaccttcagagtaaattcgccgaatataacgtgttcaccgaagaagaaaacctggtgagtgaacatacctataacgcctatgccgcatttccggaagccgaaagtgttaccattgatccgcataaaatgggctatatcccgtatagtgcaggcggcattgccattcaggatattcgcatgcgtgatgttatcagctatttcgcaacctatgtgttcgaaaagggcgcagatattccggcactgctgggtgcttatattctggaaggcagtaaagcaggcgcaaccgcagccagtgtttgggcagcacataaaaccctgccgctgaatgttaccggttatggtaaactggttggtgcaagcattgaaggcgcccgccgtttttataattttctgagcggcctggaattcaaggtgggcgataaaaccattgaagttcatccgctgaccgatccggattttaatatggttgattacgtgttccaggagaagggcaataataatctggtggaaatgaacgagctgaaccatgaattttacaaccaggcaagctacgttaccggtagcatctatggcaatgaatatctgaccagccataccgatttcgcaattccggattatggtaatagcccgtttaagtttgtgaacaacctgggcgtgaccgaagaaggctggaaagaagcaggtaaagtgaccgttctgcgcgccgctgtgatgacaccttatatgaataaggcagagaacttcgactacttcgccccgaaaattaagcaggccatgcaggaaaaactggaagccatctatgaagatcgtaag

SEQ ID NO: 62 - protein, 621 aa, Artificial sequence
  Engineered sequence
MSNTSFSAKDTDLSALFIGDKAENGQLYKELLGKLVDEHLGWRQNYMPQDPPMISAEQQTSPEFRGTVNNMRDVLDELSSRLRSQSVPWHNAGRYWGHMNSETLMPAILAYNYAMLWNGNNVAYESSPATSQMEEEVGLEFATLMGYTNGWGHIVADGSLANLEGLWYARNIKSLPFAMKAVDPTIVAGKTDWELSNMSTKEIMDLVEANGDKIDEIKAKSARGGKDLDKLGKWLVPQTKHYSWLKAADIIGIGLDQVIPVPVDSNYRMDINELEKIIRELASTETPILGVVGVVGSTEEGAVDGINEIAELRNKLVKEGIYFYFHIDAAYGGYGRAILLDEDNKLIPYKDLQSKFAEYNVFTEEENLVSEHTYNAYAAFPEAESVTIDPHKMGYIPYSAGGIAIQDIRMRDVISYFATYVFEKGADIPALLGAYILEGSKAGATAASVWAAHKTLPLNVTGYGKLVGASIEGARRFYNFLSGLEFKVGDKTIEVHPLTDPDFNMVDYVFQEKGNNNLVEMNELNHEFYNQASYVTGSIYGNEYLTSHTDFAIPDYGNSPFKFVNNLGVTEEGWKEAGKVTVLRAAVMTPYMNKAENFDYFAPKIKQAMQEKLEAIYEDRK

SEQ ID NO: 63 - DNA, 1863 bp, Artificial sequence
  Engineered sequence
atgagcaacaccagtttcagcgcaaaagataccgatctgagtgcactgtttatcggtgacaaagcagaaaatggtcagctgtataaggaactgctgggcaaactggttgatgaacatctgggttggcgccagaattatatgccgcaggatccgtcgatgatcagcgccgaacagcagaccagcccggaatttcgtggtaccgtgaataatatgaaggacgttctggatgagctgagcagtcgcctgcgtagtcagagcgttccgtggcataatgccggtcgttattggggccacatgaatagcgaaaccctgatgccggcaattctggcctataattatgcaatgctgtggaatggtaacaacgtggcctatgaaagcagcccggcaaccagccagatggaagaagaagttggtctggaatttgccaccctgatgggctataccaatggttggggccatattgttgcagatggtagcctggcaaatctggaaggcctgtggtatgcacgcaatattaagagcctgccgtttgccatgaaagccgttgatccgaccattgttgccggcaaaaccgattgggaactgagtaatatgagcaccaaagaaatcatggacctggttgaagccaatggtgacaaaattgatgagatcaaggccaaaagcgcccgcggcggtaaagatctggataaactgggtaaatggctggttccgcagaccaaacattatagttggctgaaagccgcagatattatcggcattggcctggatcaggttattccggttccggttgatagcaattatcgtatggatatcaacgagctggagaaaattatccgcgaactggcaagtaccgaaaccccgattctgggcgttgtgggcgttgtgggtagtaccgaagaaggtgccgttgatggcattaatgaaattgcagaactgcgtaacaagctggtgaaagaaggtatctatttctacttccacatcgacgccgcctatggtggctatggtcgcgcaattctgctggatgaagataataagctgatcccgtataaggaccttcagagtaaattcgccgaatataacgtgttcaccgaagaagaaaacctggtgagtgaacatacctataacgcctatgccgcatttccggaagccgaaagtgttaccattgatccgcataaaatgggctatatcccgtatagtgcaggcggcattgccattcaggatattcgcatgcgtgatgttatcagctatttcgcaacctatgtgttcgaaaagggcgcagatattccggcactgctgggtgcttatattctggaaggcagtaaagcaggcgcaaccgcagccagtgtttgggcagcacataaaaccctgccgctgaatgttaccggttatggtaaactggttggtgcaagcattgaaggcgcccgccgtttttataattttctgagcggcctggaattcaaggtgggcgataaaaccattgaagttcatccgctgaccgatccggattttaatatggttgattacgtgttccaggagaagggcaataataatctggtggaaatgaacgagctgaaccatgaattttacaaccaggcaagctacgttaccggtagcatctatggcaatgaatatctgaccagccataccgatttcgcaattccggattatggtaatagcccgtttaagtttgtgaacaacctgggcgtgaccgaagaaggctggaaagaagcaggtaaagtgaccgttctgcgcgccgctgtgatgacaccttatatgaataaggcagagaacttcgactacttcgccccgaaaattaagcaggccatgcaggaaaaactggaagccatctatgaagatcgtaag

SEQ ID NO: 64 - protein, 621 aa, Artificial sequence
  Engineered sequence
MSNTSFSAKDTDLSALFIGDKAENGQLYKELLGKLVDEHLGWRQNYMPQDPSMISAEQQTSPEFRGTVNNMKDVLDELSSRLRSQSVPWHNAGRYWGHMNSETLMPAILAYNYAMLWNGNNVAYESSPATSQMEEEVGLEFATLMGYTNGWGHIVADGSLANLEGLWYARNIKSLPFAMKAVDPTIVAGKTDWELSNMSTKEIMDLVEANGDKIDEIKAKSARGGKDLDKLGKWLVPQTKHYSWLKAADIIGIGLDQVIPVPVDSNYRMDINELEKIIRELASTETPILGVVGVVGSTEEGAVDGINEIAELRNKLVKEGIYFYFHIDAAYGGYGRAILLDEDNKLIPYKDLQSKFAEYNVFTEEENLVSEHTYNAYAAFPEAESVTIDPHKMGYIPYSAGGIAIQDIRMRDVISYFATYVFEKGADIPALLGAYILEGSKAGATAASVWAAHKTLPLNVTGYGKLVGASIEGARRFYNFLSGLEFKVGDKTIEVHPLTDPDFNMVDYVFQEKGNNNLVEMNELNHEFYNQASYVTGSIYGNEYLTSHTDFAIPDYGNSPFKFVNNLGVTEEGWKEAGKVTVLRAAVMTPYMNKAENFDYFAPKIKQAMQEKLEAIYEDRK

SEQ ID NO: 65 - DNA, 1863 bp, Artificial sequence
  Engineered sequence
atgagcaacaccagtttcagcgcaaaagataccgatctgagtgcactgtttatcggtgacaaagcagaaaatggtcagctgtataaggacctgctgggcaaactggttgatgaacatctgggttggcgccgtaactatatgccgcaggatccgccgatgatcagctcggaacagcagaccagcccggaatttcgtggtaccgtgaataatatgaaggacgttctggatgagctgagcagtcgcctgcgtagtcagagcgttccgtggcataatgccggtcgttattggggccacatgaatagcgaaaccctgatgccggcaattctggcctataattatgcaatgctgtggaatggtaacaacgtggcctatgaaagcagcccggcaaccagccagatggaagaagaagttggtctggaatttgccaccctgatgggctataccaatggttggggccatattgttgcagatggtagcctggcaaatctggaaggcctgtggtatgcacgcaatattaagagcctgccgtttgccatgaaagccgttgatccgaccattgttgccggcaaaaccgattgggaactgagtaatatgagcaccaaagaaatcatggacctggttgaagccaatggtgacaaaattgatgagatcaaggccaaaagcgcccgcggcggtaaagatctggataaactgggtaaatggctggttccgcagaccaaacattatagttggctgaaagccgcagatattatcggcattggcctggatcaggttattccggttccggttgatagcaattatcgtatggatatcaacgagctggagaaaattatccgcgaactggcaagtaccgaaaccccgattctgggcgttgtgggcgttgtgggtagtaccgaagaaggtgccgttgatggcattaatgaaattgcagaactgcgtaacaagctggtgaaagaaggtatctatttctacttccacatcgacgccgcctatggtggctatggtcgcgcaattctgctggatgaagataataagctgatcccgtataaggaccttcagagtaaattcgccgaatataacgtgttcaccgaagaagaaaacctggtgagtgaacatacctataacgcctatgccgcatttccggaagccgaaagtgttaccattgatccgcataaaatgggctatatcccgtatagtgcaggcggcattgccattcaggatattcgcatgcgtgatgttatcagctatttcgcaacctatgtgttcgaaaagggcgcagatattccggcactgctgggtgcttatattctggaaggcagtaaagcaggcgcaaccgcagccagtgtttgggcagcacataaaaccctgccgctgaatgttaccggttatggtaaactggttggtgcaagcattgaaggcgcccgccgtttttataattttctgagcggcctggaattcaaggtgggcgataaaaccattgaagttcatccgctgaccgatccggattttaatatggttgattacgtgttccaggagaagggcaataataatctggtggaaatgaacgagctgaaccatgaattttacaaccaggcaagctacgttaccggtagcatctatggcaatgaatatctgaccagccataccgatttcgcaattccggattatggtaatagcccgtttaagtttgtgaacaacctgggcgtgaccgaagaaggctggaaagaagcaggtaaagtgaccgttctgcgcgccgctgtgatgacaccttatatgaataaggcagagaacttcgactacttcgccccgaaaattaagcaggccatgcaggaaaaactggaagccatctatgaagatcgtaag

SEQ ID NO: 66 - protein, 621 aa, Artificial sequence
  Engineered sequence
MSNTSFSAKDTDLSALFIGDKAENGQLYKDLLGKLVDEHLGWRRNYMPQDPPMISSEQQTSPEFRGTVNNMKDVLDELSSRLRSQSVPWHNAGRYWGHMNSETLMPAILAYNYAMLWNGNNVAYESSPATSQMEEEVGLEFATLMGYTNGWGHIVADGSLANLEGLWYARNIKSLPFAMKAVDPTIVAGKTDWELSNMSTKEIMDLVEANGDKIDEIKAKSARGGKDLDKLGKWLVPQTKHYSWLKAADIIGIGLDQVIPVPVDSNYRMDINELEKIIRELASTETPILGVVGVVGSTEEGAVDGINEIAELRNKLVKEGIYFYFHIDAAYGGYGRAILLDEDNKLIPYKDLQSKFAEYNVFTEEENLVSEHTYNAYAAFPEAESVTIDPHKMGYIPYSAGGIAIQDIRMRDVISYFATYVFEKGADIPALLGAYILEGSKAGATAASVWAAHKTLPLNVTGYGKLVGASIEGARRFYNFLSGLEFKVGDKTIEVHPLTDPDFNMVDYVFQEKGNNNLVEMNELNHEFYNQASYVTGSIYGNEYLTSHTDFAIPDYGNSPFKFVNNLGVTEEGWKEAGKVTVLRAAVMTPYMNKAENFDYFAPKIKQAMQEKLEAIYEDRK

SEQ ID NO: 67 - DNA, 1863 bp, Artificial sequence
  Engineered sequence
atgagcaacaccagtttcagcgcaaaagataccgatctgagtgcactgtttatcggtgacaaagcagaaaatggtcagctgtataaggacctgctgggcaaactggttgatgaacatctgggttggcgccgtaactatatgccgcaggatccgccgatgatcagcacggaacgtcagaccagcccggaatttcgtggtaccgtgaataatatgaaggacgttctggatgagctgagcagtcgcctgcgtagtcagagcgttccgtggcataatgccggtcgttattggggccacatgaatagcgaaaccctgatgccggcaattctggcctataattatgcaatgctgtggaatggtaacaacgtggcctatgaaagcagcccggcaaccagccagatggaagaagaagttggtctggaatttgccaccctgatgggctataccaatggttggggccatattgttgcagatggtagcctggcaaatctggaaggcctgtggtatgcacgcaatattaagagcctgccgtttgccatgaaagccgttgatccgaccattgttgccggcaaaaccgattgggaactgagtaatatgagcaccaaagaaatcatggacctggttgaagccaatggtgacaaaattgatgagatcaaggccaaaagcgcccgcggcggtaaagatctggataaactgggtaaatggctggttccgcagaccaaacattatagttggctgaaagccgcagatattatcggcattggcctggatcaggttattccggttccggttgatagcaattatcgtatggatatcaacgagctggagaaaattatccgcgaactggcaagtaccgaaaccccgattctgggcgttgtgggcgttgtgggtagtaccgaagaaggtgccgttgatggcattaatgaaattgcagaactgcgtaacaagctggtgaaagaaggtatctatttctacttccacatcgacgccgcctatggtggctatggtcgcgcaattctgctggatgaagataataagctgatcccgtataaggaccttcagagtaaattcgccgaatataacgtgttcaccgaagaagaaaacctggtgagtgaacatacctataacgcctatgccgcatttccggaagccgaaagtgttaccattgatccgcataaaatgggctatatcccgtatagtgcaggcggcattgccattcaggatattcgcatgcgtgatgttatcagctatttcgcaacctatgtgttcgaaaagggcgcagatattccggcactgctgggtgcttatattctggaaggcagtaaagcaggcgcaaccgcagccagtgtttgggcagcacatcgtaccctgccgctgaatgttaccggttatggtaaactggttggtgcaagcattgaaggcgcccgccgtttttataattttctgagcggcctggaattcaaggtgggcgataaaaccattgaagttcatccgctgaccgatccggattttaatatggttgattacgtgttccaggagaagggcaataataatctggtggaaatgaacgagctgaaccatgaattttacaaccaggcaagctacgttaccggtagcatctatggcaatgaatatctgaccagccataccgatttcgcaattccggattatggtaatagcccgtttaagtttgtgaacaacctgggcgtgaccgaagaaggctggaaagaagcaggtaaagtgaccgttctgcgcgccgctgtgatgacaccttatatgaataaggcagagaacttcgactacttcgccccgaaaattaagcaggccatgcaggaaaaactggaagccatctatgaagatcgtaag

SEQ ID NO: 68 - protein, 621 aa, Artificial sequence
  Engineered sequence
MSNTSFSAKDTDLSALFIGDKAENGQLYKDLLGKLVDEHLGWRRNYMPQDPPMISTERQTSPEFRGTVNNMKDVLDELSSRLRSQSVPWHNAGRYWGHMNSETLMPAILAYNYAMLWNGNNVAYESSPATSQMEEEVGLEFATLMGYTNGWGHIVADGSLANLEGLWYARNIKSLPFAMKAVDPTIVAGKTDWELSNMSTKEIMDLVEANGDKIDEIKAKSARGGKDLDKLGKWLVPQTKHYSWLKAADIIGIGLDQVIPVPVDSNYRMDINELEKIIRELASTETPILGVVGVVGSTEEGAVDGINEIAELRNKLVKEGIYFYFHIDAAYGGYGRAILLDEDNKLIPYKDLQSKFAEYNVFTEEENLVSEHTYNAYAAFPEAESVTIDPHKMGYIPYSAGGIAIQDIRMRDVISYFATYVFEKGADIPALLGAYILEGSKAGATAASVWAAHRTLPLNVTGYGKLVGASIEGARRFYNFLSGLEFKVGDKTIEVHPLTDPDFNMVDYVFQEKGNNNLVEMNELNHEFYNQASYVTGSIYGNEYLTSHTDFAIPDYGNSPFKFVNNLGVTEEGWKEAGKVTVLRAAVMTPYMNKAENFDYFAPKIKQAMQEKLEAIYEDRK

SEQ ID NO: 69 - DNA, 1863 bp, Artificial sequence
  Engineered sequence
atgagcaacaccagtttcagcgcaaaagataccgatctgagtgcactgtttatcggtgacaaagcagaaaatggtcagctgtataaggacctgctgggcaaactggttgatgaacatctgggttggcgccgtaactatatgccgcaggatccgccgatgatcagcgcggaacagcagaccagcccggaatttcgtggtaccgtgaataatatgaaggacgttctggatgagctgagcagtcgcctgcgtagtcagagcgttccgtggcataatgccggtcgttattggggccacatgaatagcgaaaccctgatgccggcaattctggcctataattatgcaatgctgtggaatggtaacaacgtggcctatgaaagcagcccggcaaccagccagatggaagaagaagttggtctggaatttgccaccctgatgggctataccaatggttggggccatattgttgcagatggtagcctggcaaatctggaaggcctgtggtatgcacgcaatattaagagcctgccgtttgccatgaaagccgttgatccgaccattgttgccggcaaaaccgattgggaactgagtaatatgagcaccaaagaaatcatggacctggttgaagccaatggtgacaaaattgatgagatcaaggccaaaagcgcccgcggcggtaaagatctggataaactgggtaaatggctggttccgcagaccaaacattatagttggctgaaagccgcagatattatcggcattggcctggatcaggttattccggttccggttgatagcaattatcgtatggatatcaacgagctggagaaaattatccgcgaactggcaagtaccgaaaccccgattctgggcgttgtgggcgttgtgggtagtaccgaagaaggtgccgttgatggcattaatgaaattgcagaactgcgtaacaagctggtgaaagaaggtatctatttctacttccacatcgacgccgcctatggtggctatggtcgcgcaattctgctggatgaagataataagctgatcccgtataaggaccttcagagtaaattcgccgaatataacgtgttcaccgaagaagaaaacctggtgagtgaacatacctataacgcctatgccgcatttccggaagccgaaagtgttaccattgatccgcataaaatgggctatatcccgtatagtgcaggcggcattgccattcaggatattcgcatgcgtgatgttatcagctatttcgcaacctatgtgttcgaaaagggcgcagatattccggcactgctgggtgcttatattctggaaggcagtaaagcaggcgcaaccgcagccagtgtttgggcagcacatcgtaccctgccgctgaatgttaccggttatggtaaactggttggtgcaagcattgaaggcgcccgccgtttttataattttctgagcggcctggaattcaaggtgggcgataaaaccattgaagttcatccgctgaccgatccggattttaatatggttgattacgtgttccaggagaagggcaataataatctggtggaaatgaacgagctgaaccatgaattttacaaccaggcaagctacgttaccggtagcatctatggcaatgaatatctgaccagccataccgatttcgcaattccggattatggtaatagcccgtttaagtttgtgaacaacctgggcgtgaccgaagaaggctggaaagaagcaggtaaagtgaccgttctgcgcgccgctgtgatgacaccttatatgaataaggcagagaacttcgactacttcgccccgaaaattaagcaggccatgcaggaaaaactggaagccatctatgaagatcgtaag

SEQ ID NO: 70 - protein, 621 aa, Artificial sequence
  Engineered sequence
MSNTSFSAKDTDLSALFIGDKAENGQLYKDLLGKLVDEHLGWRRNYMPQDPPMISAEQQTSPEFRGTVNNMKDVLDELSSRLRSQSVPWHNAGRYWGHMNSETLMPAILAYNYAMLWNGNNVAYESSPATSQMEEEVGLEFATLMGYTNGWGHIVADGSLANLEGLWYARNIKSLPFAMKAVDPTIVAGKTDWELSNMSTKEIMDLVEANGDKIDEIKAKSARGGKDLDKLGKWLVPQTKHYSWLKAADIIGIGLDQVIPVPVDSNYRMDINELEKIIRELASTETPILGVVGVVGSTEEGAVDGINEIAELRNKLVKEGIYFYFHIDAAYGGYGRAILLDEDNKLIPYKDLQSKFAEYNVFTEEENLVSEHTYNAYAAFPEAESVTIDPHKMGYIPYSAGGIAIQDIRMRDVISYFATYVFEKGADIPALLGAYILEGSKAGATAASVWAAHRTLPLNVTGYGKLVGASIEGARRFYNFLSGLEFKVGDKTIEVHPLTDPDFNMVDYVFQEKGNNNLVEMNELNHEFYNQASYVTGSIYGNEYLTSHTDFAIPDYGNSPFKFVNNLGVTEEGWKEAGKVTVLRAAVMTPYMNKAENFDYFAPKIKQAMQEKLEAIYEDRK

SEQ ID NO: 71 - DNA, 1863 bp, Artificial sequence
  Engineered sequence
atgagcaacaccagtttcagcgcaaaagataccgatctgagtgcactgtttatcggtgacaaagcagaaaatggtcagctgtataaggacctgctgggcaaactggttgatgaacatctgggttggcgccagaactatatgccgcaggatccgccgatgatcagctcggaacagcagaccagcccggactttcgtggtaccgtgaataatatgaaggacgttctggatgagctgagcagtcgcctgcgtagtcagagcgttccgtggcataatgccggtcgttattggggccacatgaatagcgaaaccctgatgccggcaattctggcctataattatgcaatgctgtggaatggtaacaacgtggcctatgaaagcagcccggcaaccagccagatggaagaagaagttggtctggaatttgccaccctgatgggctataccaatggttggggccatattgttgcagatggtagcctggcaaatctggaaggcctgtggtatgcacgcaatattaagagcctgccgtttgccatgaaagccgttgatccgaccattgttgccggcaaaaccgattgggaactgagtaatatgagcaccaaagaaatcatggacctggttgaagccaatggtgacaaaattgatgagatcaaggccaaaagcgcccgcggcggtaaagatctggataaactgggtaaatggctggttccgcagaccaaacattatagttggctgaaagccgcagatattatcggcattggcctggatcaggttattccggttccggttgatagcaattatcgtatggatatcaacgagctggagaaaattatccgcgaactggcaagtaccgaaaccccgattctgggcgttgtgggcgttgtgggtagtaccgaagaaggtgccgttgatggcattaatgaaattgcagaactgcgtaacaagctggtgaaagaaggtatctatttctacttccacatcgacgccgcctatggtggctatggtcgcgcaattctgctggatgaagataataagctgatcccgtataaggaccttcagagtaaattcgccgaatataacgtgttcaccgaagaagaaaacctggtgagtgaacatacctataacgcctatgccgcatttccggaagccgaaagtgttaccattgatccgcataaaatgggctatatcccgtatagtgcaggcggcattgccattcaggatattcgcatgcgtgatgttatcagctatttcgcaacctatgtgttcgaaaagggcgcagatattccggcactgctgggtgcttatattctggaaggcagtaaagcaggcgcaaccgcagccagtgtttgggcagcacatcgtaccctgccgctgaatgttaccggttatggtaaactggttggtgcaagcattgaaggcgcccgccgtttttataattttctgagcggcctggaattcaaggtgggcgataaaaccattgaagttcatccgctgaccgatccggattttaatatggttgattacgtgttccaggagaagggcaataataatctggtggaaatgaacgagctgaaccatgaattttacaaccaggcaagctacgttaccggtagcatctatggcaatgaatatctgaccagccataccgatttcgcaattccggattatggtaatagcccgtttaagtttgtgaacaacctgggcgtgaccgaagaaggctggaaagaagcaggtaaagtgaccgttctgcgcgccgctgtgatgacaccttatatgaataaggcagagaacttcgactacttcgccccgaaaattaagcaggccatgcaggaaaaactggaagccatctatgaagatcgtaag

SEQ ID NO: 72 - protein, 621 aa, Artificial sequence
  Engineered sequence
MSNTSFSAKDTDLSALFIGDKAENGQLYKDLLGKLVDEHLGWRQNYMPQDPPMISSEQQTSPDFRGTVNNMKDVLDELSSRLRSQSVPWHNAGRYWGHMNSETLMPAILAYNYAMLWNGNNVAYESSPATSQMEEEVGLEFATLMGYTNGWGHIVADGSLANLEGLWYARNIKSLPFAMKAVDPTIVAGKTDWELSNMSTKEIMDLVEANGDKIDEIKAKSARGGKDLDKLGKWLVPQTKHYSWLKAADIIGIGLDQVIPVPVDSNYRMDINELEKIIRELASTETPILGVVGVVGSTEEGAVDGINEIAELRNKLVKEGIYFYFHIDAAYGGYGRAILLDEDNKLIPYKDLQSKFAEYNVFTEEENLVSEHTYNAYAAFPEAESVTIDPHKMGYIPYSAGGIAIQDIRMRDVISYFATYVFEKGADIPALLGAYILEGSKAGATAASVWAAHRTLPLNVTGYGKLVGASIEGARRFYNFLSGLEFKVGDKTIEVHPLTDPDFNMVDYVFQEKGNNNLVEMNELNHEFYNQASYVTGSIYGNEYLTSHTDFAIPDYGNSPFKFVNNLGVTEEGWKEAGKVTVLRAAVMTPYMNKAENFDYFAPKIKQAMQEKLEAIYEDRK

SEQ ID NO: 73 - DNA, 1863 bp, Artificial sequence
  Engineered sequence
atgagcaacaccagtttcagcgcaaaagataccgatctgagtgcactgtttatcggtgacaaagcagaaaatggtcagctgtataaggacctgctgggcaaactggttgatgaacatctgggttggcgcaagaactatatgccgcaggatccgccgatgatcagcccggaacgtcagaccagcccggaatttcgtggtaccgtgaataatatgaaggacgttctggatgagctgagcagtcgcctgcgtagtcagagcgttccgtggcataatgccggtcgttattggggccacatgaatagcgaaaccctgatgccggcaattctggcctataattatgcaatgctgtggaatggtaacaacgtggcctatgaaagcagcccggcaaccagccagatggaagaagaagttggtctggaatttgccaccctgatgggctataccaatggttggggccatattgttgcagatggtagcctggcaaatctggaaggcctgtggtatgcacgcaatattaagagcctgccgtttgccatgaaagccgttgatccgaccattgttgccggcaaaaccgattgggaactgagtaatatgagcaccaaagaaatcatggacctggttgaagccaatggtgacaaaattgatgagatcaaggccaaaagcgcccgcggcggtaaagatctggataaactgggtaaatggctggttccgcagaccaaacattatagttggctgaaagccgcagatattatcggcattggcctggatcaggttattccggttccggttgatagcaattatcgtatggatatcaacgagctggagaaaattatccgcgaactggcaagtaccgaaaccccgattctgggcgttgtgggcgttgtgggtagtaccgaagaaggtgccgttgatggcattaatgaaattgcagaactgcgtaacaagctggtgaaagaaggtatctatttctacttccacatcgacgccgcctatggtggctatggtcgcgcaattctgctggatgaagataataagctgatcccgtataaggaccttcagagtaaattcgccgaatataacgtgttcaccgaagaagaaaacctggtgagtgaacatacctataacgcctatgccgcatttccggaagccgaaagtgttaccattgatccgcataaaatgggctatatcccgtatagtgcaggcggcattgccattcaggatattcgcatgcgtgatgttatcagctatttcgcaacctatgtgttcgaaaagggcgcagatattccggcactgctgggtgcttatattctggaaggcagtaaagcaggcgcaaccgcagccagtgtttgggcagcacataaaaccctgccgctgaatgttaccggttatggtaaactggttggtgcaagcattgaaggcgcccgccgtttttataattttctgagcggcctggaattcaaggtgggcgataaaaccattgaagttcatccgctgaccgatccggattttaatatggttgattacgtgttccaggagaagggcaataataatctggtggaaatgaacgagctgaaccatgaattttacaaccaggcaagctacgttaccggtagcatctatggcaatgaatatctgaccagccataccgatttcgcaattccggattatggtaatagcccgtttaagtttgtgaacaacctgggcgtgaccgaagaaggctggaaagaagcaggtaaagtgaccgttctgcgcgccgctgtgatgacaccttatatgaataaggcagagaacttcgactacttcgccccgaaaattaagcaggccatgcaggaaaaactggaagccatctatgaagatcgtaag

SEQ ID NO: 74 - protein, 621 aa, Artificial sequence
  Engineered sequence
MSNTSFSAKDTDLSALFIGDKAENGQLYKDLLGKLVDEHLGWRKNYMPQDPPMISPERQTSPEFRGTVNNMKDVLDELSSRLRSQSVPWHNAGRYWGHMNSETLMPAILAYNYAMLWNGNNVAYESSPATSQMEEEVGLEFATLMGYTNGWGHIVADGSLANLEGLWYARNIKSLPFAMKAVDPTIVAGKTDWELSNMSTKEIMDLVEANGDKIDEIKAKSARGGKDLDKLGKWLVPQTKHYSWLKAADIIGIGLDQVIPVPVDSNYRMDINELEKIIRELASTETPILGVVGVVGSTEEGAVDGINEIAELRNKLVKEGIYFYFHIDAAYGGYGRAILLDEDNKLIPYKDLQSKFAEYNVFTEEENLVSEHTYNAYAAFPEAESVTIDPHKMGYIPYSAGGIAIQDIRMRDVISYFATYVFEKGADIPALLGAYILEGSKAGATAASVWAAHKTLPLNVTGYGKLVGASIEGARRFYNFLSGLEFKVGDKTIEVHPLTDPDFNMVDYVFQEKGNNNLVEMNELNHEFYNQASYVTGSIYGNEYLTSHTDFAIPDYGNSPFKFVNNLGVTEEGWKEAGKVTVLRAAVMTPYMNKAENFDYFAPKIKQAMQEKLEAIYEDRK

SEQ ID NO: 75 - DNA, 1863 bp, Artificial sequence
  Engineered sequence
atgagcaacaccagtttcagcgcaaaagataccgatctgagtgcactgtttatcggtgacaaagcagaaaatggtcagctgtataaggacctgctgggcaaactggttgatgaacatctgggttggcgccagaactatatgccgcaggatccgccgatgatcagcccggaacgtcagaccagcccggactttcgtggtaccgtgaataatatgaaggacgttctggatgagctgagcagtcgcctgcgtagtcagagcgttccgtggcataatgccggtcgttattggggccacatgaatagcgaaaccctgatgccggcaattctggcctataattatgcaatgctgtggaatggtaacaacgtggcctatgaaagcagcccggcaaccagccagatggaagaagaagttggtctggaatttgccaccctgatgggctataccaatggttggggccatattgttgcagatggtagcctggcaaatctggaaggcctgtggtatgcacgcaatattaagagcctgccgtttgccatgaaagccgttgatccgaccattgttgccggcaaaaccgattgggaactgagtaatatgagcaccaaagaaatcatggacctggttgaagccaatggtgacaaaattgatgagatcaaggccaaaagcgcccgcggcggtaaagatctggataaactgggtaaatggctggttccgcagaccaaacattatagttggctgaaagccgcagatattatcggcattggcctggatcaggttattccggttccggttgatagcaattatcgtatggatatcaacgagctggagaaaattatccgcgaactggcaagtaccgaaaccccgattctgggcgttgtgggcgttgtgggtagtaccgaagaaggtgccgttgatggcattaatgaaattgcagaactgcgtaacaagctggtgaaagaaggtatctatttctacttccacatcgacgccgcctatggtggctatggtcgcgcaattctgctggatgaagataataagctgatcccgtataaggaccttcagagtaaattcgccgaatataacgtgttcaccgaagaagaaaacctggtgagtgaacatacctataacgcctatgccgcatttccggaagccgaaagtgttaccattgatccgcataaaatgggctatatcccgtatagtgcaggcggcattgccattcaggatattcgcatgcgtgatgttatcagctatttcgcaacctatgtgttcgaaaagggcgcagatattccggcactgctgggtgcttatattctggaaggcagtaaagcaggcgcaaccgcagccagtgtttgggcagcacataaaaccctgccgctgaatgttaccggttatggtaaactggttggtgcaagcattgaaggcgcccgccgtttttataattttctgagcggcctggaattcaaggtgggcgataaaaccattgaagttcatccgctgaccgatccggattttaatatggttgattacgtgttccaggagaagggcaataataatctggtggaaatgaacgagctgaaccatgaattttacaaccaggcaagctacgttaccggtagcatctatggcaatgaatatctgaccagccataccgatttcgcaattccggattatggtaatagcccgtttaagtttgtgaacaacctgggcgtgaccgaagaaggctggaaagaagcaggtaaagtgaccgttctgcgcgccgctgtgatgacaccttatatgaataaggcagagaacttcgactacttcgccccgaaaattaagcaggccatgcaggaaaaactggaagccatctatgaagatcgtaag

SEQ ID NO: 76 - protein, 621 aa, Artificial sequence
  Engineered sequence
MSNTSFSAKDTDLSALFIGDKAENGQLYKDLLGKLVDEHLGWRQNYMPQDPPMISPERQTSPDFRGTVNNMKDVLDELSSRLRSQSVPWHNAGRYWGHMNSETLMPAILAYNYAMLWNGNNVAYESSPATSQMEEEVGLEFATLMGYTNGWGHIVADGSLANLEGLWYARNIKSLPFAMKAVDPTIVAGKTDWELSNMSTKEIMDLVEANGDKIDEIKAKSARGGKDLDKLGKWLVPQTKHYSWLKAADIIGIGLDQVIPVPVDSNYRMDINELEKIIRELASTETPILGVVGVVGSTEEGAVDGINEIAELRNKLVKEGIYFYFHIDAAYGGYGRAILLDEDNKLIPYKDLQSKFAEYNVFTEEENLVSEHTYNAYAAFPEAESVTIDPHKMGYIPYSAGGIAIQDIRMRDVISYFATYVFEKGADIPALLGAYILEGSKAGATAASVWAAHKTLPLNVTGYGKLVGASIEGARRFYNFLSGLEFKVGDKTIEVHPLTDPDFNMVDYVFQEKGNNNLVEMNELNHEFYNQASYVTGSIYGNEYLTSHTDFAIPDYGNSPFKFVNNLGVTEEGWKEAGKVTVLRAAVMTPYMNKAENFDYFAPKIKQAMQEKLEAIYEDRK

SEQ ID NO: 77 - DNA, 1863 bp, Artificial sequence
  Engineered sequence
atgagcaacaccagtttcagcgcaaaagataccgatctgagtgcactgtttatcggtgacaaagcagaaaatggtcagctgtataaggacctgctgggcaaactggttgatgaacatctgggttggcgccagaactatatgccgcaggatccgccgatgatcagcgcggaacgtcagaccagcccggaatttcgtggtaccgtgaataatatgaaggacgttctggatgagctgagcagtcgcctgcgtagtcagagcgttccgtggcataatgccggtcgttattggggccacatgaatagcgaaaccctgatgccggcaattctggcctataattatgcaatgctgtggaatggtaacaacgtggcctatgaaagcagcccggcaaccagccagatggaagaagaagttggtctggaatttgccaccctgatgggctataccaatggttggggccatattgttgcagatggtagcctggcaaatctggaaggcctgtggtatgcacgcaatattaagagcctgccgtttgccatgaaagccgttgatccgaccattgttgccggcaaaaccgattgggaactgagtaatatgagcaccaaagaaatcatggacctggttgaagccaatggtgacaaaattgatgagatcaaggccaaaagcgcccgcggcggtaaagatctggataaactgggtaaatggctggttccgcagaccaaacattatagttggctgaaagccgcagatattatcggcattggcctggatcaggttattccggttccggttgatagcaattatcgtatggatatcaacgagctggagaaaattatccgcgaactggcaagtaccgaaaccccgattctgggcgttgtgggcgttgtgggtagtaccgaagaaggtgccgttgatggcattaatgaaattgcagaactgcgtaacaagctggtgaaagaaggtatctatttctacttccacatcgacgccgcctatggtggctatggtcgcgcaattctgctggatgaagataataagctgatcccgtataaggaccttcagagtaaattcgccgaatataacgtgttcaccgaagaagaaaacctggtgagtgaacatacctataacgcctatgccgcatttccggaagccgaaagtgttaccattgatccgcataaaatgggctatatcccgtatagtgcaggcggcattgccattcaggatattcgcatgcgtgatgttatcagctatttcgcaacctatgtgttcgaaaagggcgcagatattccggcactgctgggtgcttatattctggaaggcagtaaagcaggcgcaaccgcagccagtgtttgggcagcacatcgtaccctgccgctgaatgttaccggttatggtaaactggttggtgcaagcattgaaggcgcccgccgtttttataattttctgagcggcctggaattcaaggtgggcgataaaaccattgaagttcatccgctgaccgatccggattttaatatggttgattacgtgttccaggagaagggcaataataatctggtggaaatgaacgagctgaaccatgaattttacaaccaggcaagctacgttaccggtagcatctatggcaatgaatatctgaccagccataccgatttcgcaattccggattatggtaatagcccgtttaagtttgtgaacaacctgggcgtgaccgaagaaggctggaaagaagcaggtaaagtgaccgttctgcgcgccgctgtgatgacaccttatatgaataaggcagagaacttcgactacttcgccccgaaaattaagcaggccatgcaggaaaaactggaagccatctatgaagatcgtaag

SEQ ID NO: 78 - protein, 621 aa, Artificial sequence
  Engineered sequence
MSNTSFSAKDTDLSALFIGDKAENGQLYKDLLGKLVDEHLGWRQNYMPQDPPMISAERQTSPEFRGTVNNMKDVLDELSSRLRSQSVPWHNAGRYWGHMNSETLMPAILAYNYAMLWNGNNVAYESSPATSQMEEEVGLEFATLMGYTNGWGHIVADGSLANLEGLWYARNIKSLPFAMKAVDPTIVAGKTDWELSNMSTKEIMDLVEANGDKIDEIKAKSARGGKDLDKLGKWLVPQTKHYSWLKAADIIGIGLDQVIPVPVDSNYRMDINELEKIIRELASTETPILGVVGVVGSTEEGAVDGINEIAELRNKLVKEGIYFYFHIDAAYGGYGRAILLDEDNKLIPYKDLQSKFAEYNVFTEEENLVSEHTYNAYAAFPEAESVTIDPHKMGYIPYSAGGIAIQDIRMRDVISYFATYVFEKGADIPALLGAYILEGSKAGATAASVWAAHRTLPLNVTGYGKLVGASIEGARRFYNFLSGLEFKVGDKTIEVHPLTDPDFNMVDYVFQEKGNNNLVEMNELNHEFYNQASYVTGSIYGNEYLTSHTDFAIPDYGNSPFKFVNNLGVTEEGWKEAGKVTVLRAAVMTPYMNKAENFDYFAPKIKQAMQEKLEAIYEDRK

SEQ ID NO: 79 - DNA, 1863 bp, Artificial sequence
  Engineered sequence
atgagcaacaccagtttcagcgcaaaagataccgatctgagtgcactgtttatcggtgacaaagcagaaaatggtcagctgtataaggacctgctgggcaaactggttgatgaacatctgggttggcgccagaactatatgccgcaggatccgccgatgatcagcccggaacgtcagaccagcccggactttcgtggtaccgtgaataatatgaaggacgttctggatgagctgagcagtcgcctgcgtagtcagagcgttccgtggcataatgccggtcgttattggggccacatgaatagcgaaaccctgatgccggcaattctggcctataattatgcaatgctgtggaatggtaacaacgtggcctatgaaagcagcccggcaaccagccagatggaagaagaagttggtctggaatttgccaccctgatgggctataccaatggttggggccatattgttgcagatggtagcctggcaaatctggaaggcctgtggtatgcacgcaatattaagagcctgccgtttgccatgaaagccgttgatccgaccattgttgccggcaaaaccgattgggaactgagtaatatgagcaccaaagaaatcatggacctggttgaagccaatggtgacaaaattgatgagatcaaggccaaaagcgcccgcggcggtaaagatctggataaactgggtaaatggctggttccgcagaccaaacattatagttggctgaaagccgcagatattatcggcattggcctggatcaggttattccggttccggttgatagcaattatcgtatggatatcaacgagctggagaaaattatccgcgaactggcaagtaccgaaaccccgattctgggcgttgtgggcgttgtgggtagtaccgaagaaggtgccgttgatggcattaatgaaattgcagaactgcgtaacaagctggtgaaagaaggtatctatttctacttccacatcgacgccgcctatggtggctatggtcgcgcaattctgctggatgaagataataagctgatcccgtataaggaccttcagagtaaattcgccgaatataacgtgttcaccgaagaagaaaacctggtgagtgaacatacctataacgcctatgccgcatttccggaagccgaaagtgttaccattgatccgcataaaatgggctatatcccgtatagtgcaggcggcattgccattcaggatattcgcatgcgtgatgttatcagctatttcgcaacctatgtgttcgaaaagggcgcagatattccggcactgctgggtgcttatattctggaaggcagtaaagcaggcgcaaccgcagccagtgtttgggcagcacatcgtaccctgccgctgaatgttaccggttatggtaaactggttggtgcaagcattgaaggcgcccgccgtttttataattttctgagcggcctggaattcaaggtgggcgataaaaccattgaagttcatccgctgaccgatccggattttaatatggttgattacgtgttccaggagaagggcaataataatctggtggaaatgaacgagctgaaccatgaattttacaaccaggcaagctacgttaccggtagcatctatggcaatgaatatctgaccagccataccgatttcgcaattccggattatggtaatagcccgtttaagtttgtgaacaacctgggcgtgaccgaagaaggctggaaagaagcaggtaaagtgaccgttctgcgcgccgctgtgatgacaccttatatgaataaggcagagaacttcgactacttcgccccgaaaattaagcaggccatgcaggaaaaactggaagccatctatgaagatcgtaag

SEQ ID NO: 80 - protein, 621 aa, Artificial sequence
  Engineered sequence
MSNTSFSAKDTDLSALFIGDKAENGQLYKDLLGKLVDEHLGWRQNYMPQDPPMISPERQTSPDFRGTVNNMKDVLDELSSRLRSQSVPWHNAGRYWGHMNSETLMPAILAYNYAMLWNGNNVAYESSPATSQMEEEVGLEFATLMGYTNGWGHIVADGSLANLEGLWYARNIKSLPFAMKAVDPTIVAGKTDWELSNMSTKEIMDLVEANGDKIDEIKAKSARGGKDLDKLGKWLVPQTKHYSWLKAADIIGIGLDQVIPVPVDSNYRMDINELEKIIRELASTETPILGVVGVVGSTEEGAVDGINEIAELRNKLVKEGIYFYFHIDAAYGGYGRAILLDEDNKLIPYKDLQSKFAEYNVFTEEENLVSEHTYNAYAAFPEAESVTIDPHKMGYIPYSAGGIAIQDIRMRDVISYFATYVFEKGADIPALLGAYILEGSKAGATAASVWAAHRTLPLNVTGYGKLVGASIEGARRFYNFLSGLEFKVGDKTIEVHPLTDPDFNMVDYVFQEKGNNNLVEMNELNHEFYNQASYVTGSIYGNEYLTSHTDFAIPDYGNSPFKFVNNLGVTEEGWKEAGKVTVLRAAVMTPYMNKAENFDYFAPKIKQAMQEKLEAIYEDRK

SEQ ID NO: 81 - DNA, 1863 bp, Artificial sequence
  Engineered sequence
atgagcaacaccagtttcagcgcaaaagatacctatctgagtgcactgtttatcggtgacaaagcagaaaatggtcagctgtataaggacctgctgggcaaactggttgatgaacatctgggttggcgccagaattatatgccgcaggatccgccgatgatcagcgccgaacagcagaccagcccggaatttcgtggtaccgtgaataatatgaaggacgttctggatgagctgagcagtcgcctgcgtagtcagagcgttccgtggcataatgccggtcgttattggggccacatgaatagcgaaaccctgatgccggcaattctggcctataattatgcaatgctgtggaatggtaacaacgtggcctatgaaagcagcccggcaaccagccagatggaagaagaagttggtctggaatttgccaccctgatgggctataccaatggttggggccatattgttgcagatggtagcctggcaaatctggaaggcctgtggtatgcacgcaatattaagagcctgccgtttgccatgaaagccgttgatccgaccattgttgccggcaaaaccgattgggaactgagtaatatgagcaccaaagaaatcatggacctggttgaagccaatggtgacaaaattgatgagatcaaggccaaaagcgcccgcggcggtaaagatctggataaactgggtaaatggctggttccgcagaccaaacattatagttggctgaaagccgcagatattatcggcattggcctggatcaggttattccggttccggttgatagcaattatcgtatggatatcaacgagctggagaaaattatccgcgaactggcaagtaccgaaaccccgattctgggcgttgtgggcgttgtgggtagtaccgaagaaggtgccgttgatggcattaatgaaattgcagaactgcgtaacaagctggtgaaagaaggtatctatttctacttccacatcgacgccgcctatggtggctatggtcgcgcaattctgctggatgaagataataagctgatcccgtataaggaccttcagagtaaattcgccgaatataacgtgttcaccgaagaagaaaacctggtgagtgaacatacctataacgcctatgccgcatttccggaagccgaaagtgttaccattgatccgcataaaatgggctatatcccgtatagtgcaggcggcattgccattcaggatattcgcatgcgtgatgttatcagctatttcgcaacctatgtgttcgaaaagggcgcagatattccggcactgctgggtgcttatattctggaaggcagtaaagcaggcgcaaccgcagccagtgtttgggcagcacataaaaccctgccgctgaatgttaccggttatggtaaactggttggtgcaagcattgaaggcgcccgccgtttttataattttctgagcggcctggaattcaaggtgggcgataaaaccattgaagttcatccgctgaccgatccggattttaatatggttgattacgtgttccaggagaagggcaataataatctggtggaaatgaacgagctgaaccatgaattttacaaccaggcaagctacgttaccggtagcatctatggcaatgaatatctgaccagccataccgatttcgcaattccggattatggtaatagcccgtttaagtttgtgaacaacctgggcgtgaccgaagaaggctggaaagaagcaggtaaagtgaccgttctgcgcgccgctgtgatgacaccttatatgaataaggcagagaacttcgactacttcgccccgaaaattaagcaggccatgcaggaaaaactggaagccatctatgaagatcgtaag

SEQ ID NO: 82 - protein, 621 aa, Artificial sequence
  Engineered sequence
MSNTSFSAKDTYLSALFIGDKAENGQLYKDLLGKLVDEHLGWRQNYMPQDPPMISAEQQTSPEFRGTVNNMKDVLDELSSRLRSQSVPWHNAGRYWGHMNSETLMPAILAYNYAMLWNGNNVAYESSPATSQMEEEVGLEFATLMGYTNGWGHIVADGSLANLEGLWYARNIKSLPFAMKAVDPTIVAGKTDWELSNMSTKEIMDLVEANGDKIDEIKAKSARGGKDLDKLGKWLVPQTKHYSWLKAADIIGIGLDQVIPVPVDSNYRMDINELEKIIRELASTETPILGVVGVVGSTEEGAVDGINEIAELRNKLVKEGIYFYFHIDAAYGGYGRAILLDEDNKLIPYKDLQSKFAEYNVFTEEENLVSEHTYNAYAAFPEAESVTIDPHKMGYIPYSAGGIAIQDIRMRDVISYFATYVFEKGADIPALLGAYILEGSKAGATAASVWAAHKTLPLNVTGYGKLVGASIEGARRFYNFLSGLEFKVGDKTIEVHPLTDPDFNMVDYVFQEKGNNNLVEMNELNHEFYNQASYVTGSIYGNEYLTSHTDFAIPDYGNSPFKFVNNLGVTEEGWKEAGKVTVLRAAVMTPYMNKAENFDYFAPKIKQAMQEKLEAIYEDRK

SEQ ID NO: 83 - DNA, 1863 bp, Artificial sequence
  Engineered sequence
atgagcaacaccagtttcagcgcaaaagataccactctgagtgcactgtttatcggtgacaaagcagaaaatggtcagctgtataaggacctgctgggcaaactggttgatgaacatctgggttggcgccagaattatatgccgcaggatccgccgatgatcagcgccgaacagcagaccagcccggaatttcgtggtaccgtgaataatatgaaggacgttctggatgagctgagcagtcgcctgcgtagtcagagcgttccgtggcataatgccggtcgttattggggccacatgaatagcgaaaccctgatgccggcaattctggcctataattatgcaatgctgtggaatggtaacaacgtggcctatgaaagcagcccggcaaccagccagatggaagaagaagttggtctggaatttgccaccctgatgggctataccaatggttggggccatattgttgcagatggtagcctggcaaatctggaaggcctgtggtatgcacgcaatattaagagcctgccgtttgccatgaaagccgttgatccgaccattgttgccggcaaaaccgattgggaactgagtaatatgagcaccaaagaaatcatggacctggttgaagccaatggtgacaaaattgatgagatcaaggccaaaagcgcccgcggcggtaaagatctggataaactgggtaaatggctggttccgcagaccaaacattatagttggctgaaagccgcagatattatcggcattggcctggatcaggttattccggttccggttgatagcaattatcgtatggatatcaacgagctggagaaaattatccgcgaactggcaagtaccgaaaccccgattctgggcgttgtgggcgttgtgggtagtaccgaagaaggtgccgttgatggcattaatgaaattgcagaactgcgtaacaagctggtgaaagaaggtatctatttctacttccacatcgacgccgcctatggtggctatggtcgcgcaattctgctggatgaagataataagctgatcccgtataaggaccttcagagtaaattcgccgaatataacgtgttcaccgaagaagaaaacctggtgagtgaacatacctataacgcctatgccgcatttccggaagccgaaagtgttaccattgatccgcataaaatgggctatatcccgtatagtgcaggcggcattgccattcaggatattcgcatgcgtgatgttatcagctatttcgcaacctatgtgttcgaaaagggcgcagatattccggcactgctgggtgcttatattctggaaggcagtaaagcaggcgcaaccgcagccagtgtttgggcagcacataaaaccctgccgctgaatgttaccggttatggtaaactggttggtgcaagcattgaaggcgcccgccgtttttataattttctgagcggcctggaattcaaggtgggcgataaaaccattgaagttcatccgctgaccgatccggattttaatatggttgattacgtgttccaggagaagggcaataataatctggtggaaatgaacgagctgaaccatgaattttacaaccaggcaagctacgttaccggtagcatctatggcaatgaatatctgaccagccataccgatttcgcaattccggattatggtaatagcccgtttaagtttgtgaacaacctgggcgtgaccgaagaaggctggaaagaagcaggtaaagtgaccgttctgcgcgccgctgtgatgacaccttatatgaataaggcagagaacttcgactacttcgccccgaaaattaagcaggccatgcaggaaaaactggaagccatctatgaagatcgtaag

SEQ ID NO: 84 - protein, 621 aa, Artificial sequence
  Engineered sequence
MSNTSFSAKDTTLSALFIGDKAENGQLYKDLLGKLVDEHLGWRQNYMPQDPPMISAEQQTSPEFRGTVNNMKDVLDELSSRLRSQSVPWHNAGRYWGHMNSETLMPAILAYNYAMLWNGNNVAYESSPATSQMEEEVGLEFATLMGYTNGWGHIVADGSLANLEGLWYARNIKSLPFAMKAVDPTIVAGKTDWELSNMSTKEIMDLVEANGDKIDEIKAKSARGGKDLDKLGKWLVPQTKHYSWLKAADIIGIGLDQVIPVPVDSNYRMDINELEKIIRELASTETPILGVVGVVGSTEEGAVDGINEIAELRNKLVKEGIYFYFHIDAAYGGYGRAILLDEDNKLIPYKDLQSKFAEYNVFTEEENLVSEHTYNAYAAFPEAESVTIDPHKMGYIPYSAGGIAIQDIRMRDVISYFATYVFEKGADIPALLGAYILEGSKAGATAASVWAAHKTLPLNVTGYGKLVGASIEGARRFYNFLSGLEFKVGDKTIEVHPLTDPDFNMVDYVFQEKGNNNLVEMNELNHEFYNQASYVTGSIYGNEYLTSHTDFAIPDYGNSPFKFVNNLGVTEEGWKEAGKVTVLRAAVMTPYMNKAENFDYFAPKIKQAMQEKLEAIYEDRK

SEQ ID NO: 85 - DNA, 1863 bp, Artificial sequence
  Engineered sequence
atgagcaacaccagtttcagcgcaaaagataccgatctgagtgcactgtttatcggtgacaaagcagaaaatggtacgctgtataaggacctgctgggcaaactggttgatgaacatctgggttggcgccagaattatatgccgcaggatccgccgatgatcagcgccgaacagcagaccagcccggaatttcgtggtaccgtgaataatatgaaggacgttctggatgagctgagcagtcgcctgcgtagtcagagcgttccgtggcataatgccggtcgttattggggccacatgaatagcgaaaccctgatgccggcaattctggcctataattatgcaatgctgtggaatggtaacaacgtggcctatgaaagcagcccggcaaccagccagatggaagaagaagttggtctggaatttgccaccctgatgggctataccaatggttggggccatattgttgcagatggtagcctggcaaatctggaaggcctgtggtatgcacgcaatattaagagcctgccgtttgccatgaaagccgttgatccgaccattgttgccggcaaaaccgattgggaactgagtaatatgagcaccaaagaaatcatggacctggttgaagccaatggtgacaaaattgatgagatcaaggccaaaagcgcccgcggcggtaaagatctggataaactgggtaaatggctggttccgcagaccaaacattatagttggctgaaagccgcagatattatcggcattggcctggatcaggttattccggttccggttgatagcaattatcgtatggatatcaacgagctggagaaaattatccgcgaactggcaagtaccgaaaccccgattctgggcgttgtgggcgttgtgggtagtaccgaagaaggtgccgttgatggcattaatgaaattgcagaactgcgtaacaagctggtgaaagaaggtatctatttctacttccacatcgacgccgcctatggtggctatggtcgcgcaattctgctggatgaagataataagctgatcccgtataaggaccttcagagtaaattcgccgaatataacgtgttcaccgaagaagaaaacctggtgagtgaacatacctataacgcctatgccgcatttccggaagccgaaagtgttaccattgatccgcataaaatgggctatatcccgtatagtgcaggcggcattgccattcaggatattcgcatgcgtgatgttatcagctatttcgcaacctatgtgttcgaaaagggcgcagatattccggcactgctgggtgcttatattctggaaggcagtaaagcaggcgcaaccgcagccagtgtttgggcagcacataaaaccctgccgctgaatgttaccggttatggtaaactggttggtgcaagcattgaaggcgcccgccgtttttataattttctgagcggcctggaattcaaggtgggcgataaaaccattgaagttcatccgctgaccgatccggattttaatatggttgattacgtgttccaggagaagggcaataataatctggtggaaatgaacgagctgaaccatgaattttacaaccaggcaagctacgttaccggtagcatctatggcaatgaatatctgaccagccataccgatttcgcaattccggattatggtaatagcccgtttaagtttgtgaacaacctgggcgtgaccgaagaaggctggaaagaagcaggtaaagtgaccgttctgcgcgccgctgtgatgacaccttatatgaataaggcagagaacttcgactacttcgccccgaaaattaagcaggccatgcaggaaaaactggaagccatctatgaagatcgtaag

SEQ ID NO: 86 - protein, 621 aa, Artificial sequence
  Engineered sequence
MSNTSFSAKDTDLSALFIGDKAENGTLYKDLLGKLVDEHLGWRQNYMPQDPPMISAEQQTSPEFRGTVNNMKDVLDELSSRLRSQSVPWHNAGRYWGHMNSETLMPAILAYNYAMLWNGNNVAYESSPATSQMEEEVGLEFATLMGYTNGWGHIVADGSLANLEGLWYARNIKSLPFAMKAVDPTIVAGKTDWELSNMSTKEIMDLVEANGDKIDEIKAKSARGGKDLDKLGKWLVPQTKHYSWLKAADIIGIGLDQVIPVPVDSNYRMDINELEKIIRELASTETPILGVVGVVGSTEEGAVDGINEIAELRNKLVKEGIYFYFHIDAAYGGYGRAILLDEDNKLIPYKDLQSKFAEYNVFTEEENLVSEHTYNAYAAFPEAESVTIDPHKMGYIPYSAGGIAIQDIRMRDVISYFATYVFEKGADIPALLGAYILEGSKAGATAASVWAAHKTLPLNVTGYGKLVGASIEGARRFYNFLSGLEFKVGDKTIEVHPLTDPDFNMVDYVFQEKGNNNLVEMNELNHEFYNQASYVTGSIYGNEYLTSHTDFAIPDYGNSPFKFVNNLGVTEEGWKEAGKVTVLRAAVMTPYMNKAENFDYFAPKIKQAMQEKLEAIYEDRK

SEQ ID NO: 87 - DNA, 1863 bp, Artificial sequence
  Engineered sequence
atgagcaacaccagtttcagcgcaaaagataccgatctgagtgcactgtttatcggtgacaaagcagaaaatggttttctgtataaggacctgctgggcaaactggttgatgaacatctgggttggcgccagaattatatgccgcaggatccgccgatgatcagcgccgaacagcagaccagcccggaatttcgtggtaccgtgaataatatgaaggacgttctggatgagctgagcagtcgcctgcgtagtcagagcgttccgtggcataatgccggtcgttattggggccacatgaatagcgaaaccctgatgccggcaattctggcctataattatgcaatgctgtggaatggtaacaacgtggcctatgaaagcagcccggcaaccagccagatggaagaagaagttggtctggaatttgccaccctgatgggctataccaatggttggggccatattgttgcagatggtagcctggcaaatctggaaggcctgtggtatgcacgcaatattaagagcctgccgtttgccatgaaagccgttgatccgaccattgttgccggcaaaaccgattgggaactgagtaatatgagcaccaaagaaatcatggacctggttgaagccaatggtgacaaaattgatgagatcaaggccaaaagcgcccgcggcggtaaagatctggataaactgggtaaatggctggttccgcagaccaaacattatagttggctgaaagccgcagatattatcggcattggcctggatcaggttattccggttccggttgatagcaattatcgtatggatatcaacgagctggagaaaattatccgcgaactggcaagtaccgaaaccccgattctgggcgttgtgggcgttgtgggtagtaccgaagaaggtgccgttgatggcattaatgaaattgcagaactgcgtaacaagctggtgaaagaaggtatctatttctacttccacatcgacgccgcctatggtggctatggtcgcgcaattctgctggatgaagataataagctgatcccgtataaggaccttcagagtaaattcgccgaatataacgtgttcaccgaagaagaaaacctggtgagtgaacatacctataacgcctatgccgcatttccggaagccgaaagtgttaccattgatccgcataaaatgggctatatcccgtatagtgcaggcggcattgccattcaggatattcgcatgcgtgatgttatcagctatttcgcaacctatgtgttcgaaaagggcgcagatattccggcactgctgggtgcttatattctggaaggcagtaaagcaggcgcaaccgcagccagtgtttgggcagcacataaaaccctgccgctgaatgttaccggttatggtaaactggttggtgcaagcattgaaggcgcccgccgtttttataattttctgagcggcctggaattcaaggtgggcgataaaaccattgaagttcatccgctgaccgatccggattttaatatggttgattacgtgttccaggagaagggcaataataatctggtggaaatgaacgagctgaaccatgaattttacaaccaggcaagctacgttaccggtagcatctatggcaatgaatatctgaccagccataccgatttcgcaattccggattatggtaatagcccgtttaagtttgtgaacaacctgggcgtgaccgaagaaggctggaaagaagcaggtaaagtgaccgttctgcgcgccgctgtgatgacaccttatatgaataaggcagagaacttcgactacttcgccccgaaaattaagcaggccatgcaggaaaaactggaagccatctatgaagatcgtaag

SEQ ID NO: 88 - protein, 621 aa, Artificial sequence
  Engineered sequence
MSNTSFSAKDTDLSALFIGDKAENGFLYKDLLGKLVDEHLGWRQNYMPQDPPMISAEQQTSPEFRGTVNNMKDVLDELSSRLRSQSVPWHNAGRYWGHMNSETLMPAILAYNYAMLWNGNNVAYESSPATSQMEEEVGLEFATLMGYTNGWGHIVADGSLANLEGLWYARNIKSLPFAMKAVDPTIVAGKTDWELSNMSTKEIMDLVEANGDKIDEIKAKSARGGKDLDKLGKWLVPQTKHYSWLKAADIIGIGLDQVIPVPVDSNYRMDINELEKIIRELASTETPILGVVGVVGSTEEGAVDGINEIAELRNKLVKEGIYFYFHIDAAYGGYGRAILLDEDNKLIPYKDLQSKFAEYNVFTEEENLVSEHTYNAYAAFPEAESVTIDPHKMGYIPYSAGGIAIQDIRMRDVISYFATYVFEKGADIPALLGAYILEGSKAGATAASVWAAHKTLPLNVTGYGKLVGASIEGARRFYNFLSGLEFKVGDKTIEVHPLTDPDFNMVDYVFQEKGNNNLVEMNELNHEFYNQASYVTGSIYGNEYLTSHTDFAIPDYGNSPFKFVNNLGVTEEGWKEAGKVTVLRAAVMTPYMNKAENFDYFAPKIKQAMQEKLEAIYEDRK

SEQ ID NO: 89 - DNA, 1863 bp, Artificial sequence
  Engineered sequence
atgagcaacaccagtttcagcgcaaaagataccgatctgagtgcactgtttatcggtgacaaagcagaaaatggtcagctgtataaggacctgctgggcaaactggttgatgaacatctgggttggcgcattaattatatgccgcaggatccgccgatgatcagcgccgaacagcagaccagcccggaatttcgtggtaccgtgaataatatgaaggacgttctggatgagctgagcagtcgcctgcgtagtcagagcgttccgtggcataatgccggtcgttattggggccacatgaatagcgaaaccctgatgccggcaattctggcctataattatgcaatgctgtggaatggtaacaacgtggcctatgaaagcagcccggcaaccagccagatggaagaagaagttggtctggaatttgccaccctgatgggctataccaatggttggggccatattgttgcagatggtagcctggcaaatctggaaggcctgtggtatgcacgcaatattaagagcctgccgtttgccatgaaagccgttgatccgaccattgttgccggcaaaaccgattgggaactgagtaatatgagcaccaaagaaatcatggacctggttgaagccaatggtgacaaaattgatgagatcaaggccaaaagcgcccgcggcggtaaagatctggataaactgggtaaatggctggttccgcagaccaaacattatagttggctgaaagccgcagatattatcggcattggcctggatcaggttattccggttccggttgatagcaattatcgtatggatatcaacgagctggagaaaattatccgcgaactggcaagtaccgaaaccccgattctgggcgttgtgggcgttgtgggtagtaccgaagaaggtgccgttgatggcattaatgaaattgcagaactgcgtaacaagctggtgaaagaaggtatctatttctacttccacatcgacgccgcctatggtggctatggtcgcgcaattctgctggatgaagataataagctgatcccgtataaggaccttcagagtaaattcgccgaatataacgtgttcaccgaagaagaaaacctggtgagtgaacatacctataacgcctatgccgcatttccggaagccgaaagtgttaccattgatccgcataaaatgggctatatcccgtatagtgcaggcggcattgccattcaggatattcgcatgcgtgatgttatcagctatttcgcaacctatgtgttcgaaaagggcgcagatattccggcactgctgggtgcttatattctggaaggcagtaaagcaggcgcaaccgcagccagtgtttgggcagcacataaaaccctgccgctgaatgttaccggttatggtaaactggttggtgcaagcattgaaggcgcccgccgtttttataattttctgagcggcctggaattcaaggtgggcgataaaaccattgaagttcatccgctgaccgatccggattttaatatggttgattacgtgttccaggagaagggcaataataatctggtggaaatgaacgagctgaaccatgaattttacaaccaggcaagctacgttaccggtagcatctatggcaatgaatatctgaccagccataccgatttcgcaattccggattatggtaatagcccgtttaagtttgtgaacaacctgggcgtgaccgaagaaggctggaaagaagcaggtaaagtgaccgttctgcgcgccgctgtgatgacaccttatatgaataaggcagagaacttcgactacttcgccccgaaaattaagcaggccatgcaggaaaaactggaagccatctatgaagatcgtaag

SEQ ID NO: 90 - protein, 621 aa, Artificial sequence
  Engineered sequence
MSNTSFSAKDTDLSALFIGDKAENGQLYKDLLGKLVDEHLGWRINYMPQDPPMISAEQQTSPEFRGTVNNMKDVLDELSSRLRSQSVPWHNAGRYWGHMNSETLMPAILAYNYAMLWNGNNVAYESSPATSQMEEEVGLEFATLMGYTNGWGHIVADGSLANLEGLWYARNIKSLPFAMKAVDPTIVAGKTDWELSNMSTKEIMDLVEANGDKIDEIKAKSARGGKDLDKLGKWLVPQTKHYSWLKAADIIGIGLDQVIPVPVDSNYRMDINELEKIIRELASTETPILGVVGVVGSTEEGAVDGINEIAELRNKLVKEGIYFYFHIDAAYGGYGRAILLDEDNKLIPYKDLQSKFAEYNVFTEEENLVSEHTYNAYAAFPEAESVTIDPHKMGYIPYSAGGIAIQDIRMRDVISYFATYVFEKGADIPALLGAYILEGSKAGATAASVWAAHKTLPLNVTGYGKLVGASIEGARRFYNFLSGLEFKVGDKTIEVHPLTDPDFNMVDYVFQEKGNNNLVEMNELNHEFYNQASYVTGSIYGNEYLTSHTDFAIPDYGNSPFKFVNNLGVTEEGWKEAGKVTVLRAAVMTPYMNKAENFDYFAPKIKQAMQEKLEAIYEDRK

SEQ ID NO: 91 - DNA, 1863 bp, Artificial sequence
  Engineered sequence
atgagcaacaccagtttcagcgcaaaagataccgatctgagtgcactgtttatcggtgacaaagcagaaaatggtcagctgtataaggacctgctgggcaaactggttgatgaacatctgggttggcgcctgaattatatgccgcaggatccgccgatgatcagcgccgaacagcagaccagcccggaatttcgtggtaccgtgaataatatgaaggacgttctggatgagctgagcagtcgcctgcgtagtcagagcgttccgtggcataatgccggtcgttattggggccacatgaatagcgaaaccctgatgccggcaattctggcctataattatgcaatgctgtggaatggtaacaacgtggcctatgaaagcagcccggcaaccagccagatggaagaagaagttggtctggaatttgccaccctgatgggctataccaatggttggggccatattgttgcagatggtagcctggcaaatctggaaggcctgtggtatgcacgcaatattaagagcctgccgtttgccatgaaagccgttgatccgaccattgttgccggcaaaaccgattgggaactgagtaatatgagcaccaaagaaatcatggacctggttgaagccaatggtgacaaaattgatgagatcaaggccaaaagcgcccgcggcggtaaagatctggataaactgggtaaatggctggttccgcagaccaaacattatagttggctgaaagccgcagatattatcggcattggcctggatcaggttattccggttccggttgatagcaattatcgtatggatatcaacgagctggagaaaattatccgcgaactggcaagtaccgaaaccccgattctgggcgttgtgggcgttgtgggtagtaccgaagaaggtgccgttgatggcattaatgaaattgcagaactgcgtaacaagctggtgaaagaaggtatctatttctacttccacatcgacgccgcctatggtggctatggtcgcgcaattctgctggatgaagataataagctgatcccgtataaggaccttcagagtaaattcgccgaatataacgtgttcaccgaagaagaaaacctggtgagtgaacatacctataacgcctatgccgcatttccggaagccgaaagtgttaccattgatccgcataaaatgggctatatcccgtatagtgcaggcggcattgccattcaggatattcgcatgcgtgatgttatcagctatttcgcaacctatgtgttcgaaaagggcgcagatattccggcactgctgggtgcttatattctggaaggcagtaaagcaggcgcaaccgcagccagtgtttgggcagcacataaaaccctgccgctgaatgttaccggttatggtaaactggttggtgcaagcattgaaggcgcccgccgtttttataattttctgagcggcctggaattcaaggtgggcgataaaaccattgaagttcatccgctgaccgatccggattttaatatggttgattacgtgttccaggagaagggcaataataatctggtggaaatgaacgagctgaaccatgaattttacaaccaggcaagctacgttaccggtagcatctatggcaatgaatatctgaccagccataccgatttcgcaattccggattatggtaatagcccgtttaagtttgtgaacaacctgggcgtgaccgaagaaggctggaaagaagcaggtaaagtgaccgttctgcgcgccgctgtgatgacaccttatatgaataaggcagagaacttcgactacttcgccccgaaaattaagcaggccatgcaggaaaaactggaagccatctatgaagatcgtaag

SEQ ID NO: 92 - protein, 621 aa, Artificial sequence
  Engineered sequence
MSNTSFSAKDTDLSALFIGDKAENGQLYKDLLGKLVDEHLGWRLNYMPQDPPMISAEQQTSPEFRGTVNNMKDVLDELSSRLRSQSVPWHNAGRYWGHMNSETLMPAILAYNYAMLWNGNNVAYESSPATSQMEEEVGLEFATLMGYTNGWGHIVADGSLANLEGLWYARNIKSLPFAMKAVDPTIVAGKTDWELSNMSTKEIMDLVEANGDKIDEIKAKSARGGKDLDKLGKWLVPQTKHYSWLKAADIIGIGLDQVIPVPVDSNYRMDINELEKIIRELASTETPILGVVGVVGSTEEGAVDGINEIAELRNKLVKEGIYFYFHIDAAYGGYGRAILLDEDNKLIPYKDLQSKFAEYNVFTEEENLVSEHTYNAYAAFPEAESVTIDPHKMGYIPYSAGGIAIQDIRMRDVISYFATYVFEKGADIPALLGAYILEGSKAGATAASVWAAHKTLPLNVTGYGKLVGASIEGARRFYNFLSGLEFKVGDKTIEVHPLTDPDFNMVDYVFQEKGNNNLVEMNELNHEFYNQASYVTGSIYGNEYLTSHTDFAIPDYGNSPFKFVNNLGVTEEGWKEAGKVTVLRAAVMTPYMNKAENFDYFAPKIKQAMQEKLEAIYEDRK

SEQ ID NO: 93 - DNA, 1863 bp, Artificial sequence
  Engineered sequence
atgagcaacaccagtttcagcgcaaaagataccgatctgagtgcactgtttatcggtgacaaagcagaaaatggtcagctgtataaggacctgctgggcaaactggttgatgaacatctgggttggcgccagaattatatgccgcaggatccgccgatgatcagcgccgaaaggcagaccagcccggaatttcgtggtaccgtgaataatatgaaggacgttctggatgagctgagcagtcgcctgcgtagtcagagcgttccgtggcataatgccggtcgttattggggccacatgaatagcgaaaccctgatgccggcaattctggcctataattatgcaatgctgtggaatggtaacaacgtggcctatgaaagcagcccggcaaccagccagatggaagaagaagttggtctggaatttgccaccctgatgggctataccaatggttggggccatattgttgcagatggtagcctggcaaatctggaaggcctgtggtatgcacgcaatattaagagcctgccgtttgccatgaaagccgttgatccgaccattgttgccggcaaaaccgattgggaactgagtaatatgagcaccaaagaaatcatggacctggttgaagccaatggtgacaaaattgatgagatcaaggccaaaagcgcccgcggcggtaaagatctggataaactgggtaaatggctggttccgcagaccaaacattatagttggctgaaagccgcagatattatcggcattggcctggatcaggttattccggttccggttgatagcaattatcgtatggatatcaacgagctggagaaaattatccgcgaactggcaagtaccgaaaccccgattctgggcgttgtgggcgttgtgggtagtaccgaagaaggtgccgttgatggcattaatgaaattgcagaactgcgtaacaagctggtgaaagaaggtatctatttctacttccacatcgacgccgcctatggtggctatggtcgcgcaattctgctggatgaagataataagctgatcccgtataaggaccttcagagtaaattcgccgaatataacgtgttcaccgaagaagaaaacctggtgagtgaacatacctataacgcctatgccgcatttccggaagccgaaagtgttaccattgatccgcataaaatgggctatatcccgtatagtgcaggcggcattgccattcaggatattcgcatgcgtgatgttatcagctatttcgcaacctatgtgttcgaaaagggcgcagatattccggcactgctgggtgcttatattctggaaggcagtaaagcaggcgcaaccgcagccagtgtttgggcagcacataaaaccctgccgctgaatgttaccggttatggtaaactggttggtgcaagcattgaaggcgcccgccgtttttataattttctgagcggcctggaattcaaggtgggcgataaaaccattgaagttcatccgctgaccgatccggattttaatatggttgattacgtgttccaggagaagggcaataataatctggtggaaatgaacgagctgaaccatgaattttacaaccaggcaagctacgttaccggtagcatctatggcaatgaatatctgaccagccataccgatttcgcaattccggattatggtaatagcccgtttaagtttgtgaacaacctgggcgtgaccgaagaaggctggaaagaagcaggtaaagtgaccgttctgcgcgccgctgtgatgacaccttatatgaataaggcagagaacttcgactacttcgccccgaaaattaagcaggccatgcaggaaaaactggaagccatctatgaagatcgtaag

SEQ ID NO: 94 - protein, 621 aa, Artificial sequence
  Engineered sequence
MSNTSFSAKDTDLSALFIGDKAENGQLYKDLLGKLVDEHLGWRQNYMPQDPPMISAERQTSPEFRGTVNNMKDVLDELSSRLRSQSVPWHNAGRYWGHMNSETLMPAILAYNYAMLWNGNNVAYESSPATSQMEEEVGLEFATLMGYTNGWGHIVADGSLANLEGLWYARNIKSLPFAMKAVDPTIVAGKTDWELSNMSTKEIMDLVEANGDKIDEIKAKSARGGKDLDKLGKWLVPQTKHYSWLKAADIIGIGLDQVIPVPVDSNYRMDINELEKIIRELASTETPILGVVGVVGSTEEGAVDGINEIAELRNKLVKEGIYFYFHIDAAYGGYGRAILLDEDNKLIPYKDLQSKFAEYNVFTEEENLVSEHTYNAYAAFPEAESVTIDPHKMGYIPYSAGGIAIQDIRMRDVISYFATYVFEKGADIPALLGAYILEGSKAGATAASVWAAHKTLPLNVTGYGKLVGASIEGARRFYNFLSGLEFKVGDKTIEVHPLTDPDFNMVDYVFQEKGNNNLVEMNELNHEFYNQASYVTGSIYGNEYLTSHTDFAIPDYGNSPFKFVNNLGVTEEGWKEAGKVTVLRAAVMTPYMNKAENFDYFAPKIKQAMQEKLEAIYEDRK

SEQ ID NO: 95 - DNA, 1863 bp, Artificial sequence
  Engineered sequence
atgagcaacaccagtttcagcgcaaaagataccgatctgagtgcactgtttatcggtgacaaagcagaaaatggtcagctgtataaggacctgctgggcaaactggttgatgaacatctgggttggcgccagaattatatgccgcaggatccgccgatgatcagcgccgaagttcagaccagcccggaatttcgtggtaccgtgaataatatgaaggacgttctggatgagctgagcagtcgcctgcgtagtcagagcgttccgtggcataatgccggtcgttattggggccacatgaatagcgaaaccctgatgccggcaattctggcctataattatgcaatgctgtggaatggtaacaacgtggcctatgaaagcagcccggcaaccagccagatggaagaagaagttggtctggaatttgccaccctgatgggctataccaatggttggggccatattgttgcagatggtagcctggcaaatctggaaggcctgtggtatgcacgcaatattaagagcctgccgtttgccatgaaagccgttgatccgaccattgttgccggcaaaaccgattgggaactgagtaatatgagcaccaaagaaatcatggacctggttgaagccaatggtgacaaaattgatgagatcaaggccaaaagcgcccgcggcggtaaagatctggataaactgggtaaatggctggttccgcagaccaaacattatagttggctgaaagccgcagatattatcggcattggcctggatcaggttattccggttccggttgatagcaattatcgtatggatatcaacgagctggagaaaattatccgcgaactggcaagtaccgaaaccccgattctgggcgttgtgggcgttgtgggtagtaccgaagaaggtgccgttgatggcattaatgaaattgcagaactgcgtaacaagctggtgaaagaaggtatctatttctacttccacatcgacgccgcctatggtggctatggtcgcgcaattctgctggatgaagataataagctgatcccgtataaggaccttcagagtaaattcgccgaatataacgtgttcaccgaagaagaaaacctggtgagtgaacatacctataacgcctatgccgcatttccggaagccgaaagtgttaccattgatccgcataaaatgggctatatcccgtatagtgcaggcggcattgccattcaggatattcgcatgcgtgatgttatcagctatttcgcaacctatgtgttcgaaaagggcgcagatattccggcactgctgggtgcttatattctggaaggcagtaaagcaggcgcaaccgcagccagtgtttgggcagcacataaaaccctgccgctgaatgttaccggttatggtaaactggttggtgcaagcattgaaggcgcccgccgtttttataattttctgagcggcctggaattcaaggtgggcgataaaaccattgaagttcatccgctgaccgatccggattttaatatggttgattacgtgttccaggagaagggcaataataatctggtggaaatgaacgagctgaaccatgaattttacaaccaggcaagctacgttaccggtagcatctatggcaatgaatatctgaccagccataccgatttcgcaattccggattatggtaatagcccgtttaagtttgtgaacaacctgggcgtgaccgaagaaggctggaaagaagcaggtaaagtgaccgttctgcgcgccgctgtgatgacaccttatatgaataaggcagagaacttcgactacttcgccccgaaaattaagcaggccatgcaggaaaaactggaagccatctatgaagatcgtaag

SEQ ID NO: 96 - protein, 621 aa, Artificial sequence
  Engineered sequence
MSNTSFSAKDTDLSALFIGDKAENGQLYKDLLGKLVDEHLGWRQNYMPQDPPMISAEVQTSPEFRGTVNNMKDVLDELSSRLRSQSVPWHNAGRYWGHMNSETLMPAILAYNYAMLWNGNNVAYESSPATSQMEEEVGLEFATLMGYTNGWGHIVADGSLANLEGLWYARNIKSLPFAMKAVDPTIVAGKTDWELSNMSTKEIMDLVEANGDKIDEIKAKSARGGKDLDKLGKWLVPQTKHYSWLKAADIIGIGLDQVIPVPVDSNYRMDINELEKIIRELASTETPILGVVGVVGSTEEGAVDGINEIAELRNKLVKEGIYFYFHIDAAYGGYGRAILLDEDNKLIPYKDLQSKFAEYNVFTEEENLVSEHTYNAYAAFPEAESVTIDPHKMGYIPYSAGGIAIQDIRMRDVISYFATYVFEKGADIPALLGAYILEGSKAGATAASVWAAHKTLPLNVTGYGKLVGASIEGARRFYNFLSGLEFKVGDKTIEVHPLTDPDFNMVDYVFQEKGNNNLVEMNELNHEFYNQASYVTGSIYGNEYLTSHTDFAIPDYGNSPFKFVNNLGVTEEGWKEAGKVTVLRAAVMTPYMNKAENFDYFAPKIKQAMQEKLEAIYEDRK

SEQ ID NO: 97 - DNA, 1863 bp, Artificial sequence
  Engineered sequence
atgagcaacaccagtttcagcgcaaaagataccgatctgagtgcactgtttatcggtgacaaagcagaaaatggtcagctgtataaggacctgctgggcaaactggttgatgaacatctgggttggcgccagaattatatgccgcaggatccgccgatgatcagcgccgaacatcagaccagcccggaatttcgtggtaccgtgaataatatgaaggacgttctggatgagctgagcagtcgcctgcgtagtcagagcgttccgtggcataatgccggtcgttattggggccacatgaatagcgaaaccctgatgccggcaattctggcctataattatgcaatgctgtggaatggtaacaacgtggcctatgaaagcagcccggcaaccagccagatggaagaagaagttggtctggaatttgccaccctgatgggctataccaatggttggggccatattgttgcagatggtagcctggcaaatctggaaggcctgtggtatgcacgcaatattaagagcctgccgtttgccatgaaagccgttgatccgaccattgttgccggcaaaaccgattgggaactgagtaatatgagcaccaaagaaatcatggacctggttgaagccaatggtgacaaaattgatgagatcaaggccaaaagcgcccgcggcggtaaagatctggataaactgggtaaatggctggttccgcagaccaaacattatagttggctgaaagccgcagatattatcggcattggcctggatcaggttattccggttccggttgatagcaattatcgtatggatatcaacgagctggagaaaattatccgcgaactggcaagtaccgaaaccccgattctgggcgttgtgggcgttgtgggtagtaccgaagaaggtgccgttgatggcattaatgaaattgcagaactgcgtaacaagctggtgaaagaaggtatctatttctacttccacatcgacgccgcctatggtggctatggtcgcgcaattctgctggatgaagataataagctgatcccgtataaggaccttcagagtaaattcgccgaatataacgtgttcaccgaagaagaaaacctggtgagtgaacatacctataacgcctatgccgcatttccggaagccgaaagtgttaccattgatccgcataaaatgggctatatcccgtatagtgcaggcggcattgccattcaggatattcgcatgcgtgatgttatcagctatttcgcaacctatgtgttcgaaaagggcgcagatattccggcactgctgggtgcttatattctggaaggcagtaaagcaggcgcaaccgcagccagtgtttgggcagcacataaaaccctgccgctgaatgttaccggttatggtaaactggttggtgcaagcattgaaggcgcccgccgtttttataattttctgagcggcctggaattcaaggtgggcgataaaaccattgaagttcatccgctgaccgatccggattttaatatggttgattacgtgttccaggagaagggcaataataatctggtggaaatgaacgagctgaaccatgaattttacaaccaggcaagctacgttaccggtagcatctatggcaatgaatatctgaccagccataccgatttcgcaattccggattatggtaatagcccgtttaagtttgtgaacaacctgggcgtgaccgaagaaggctggaaagaagcaggtaaagtgaccgttctgcgcgccgctgtgatgacaccttatatgaataaggcagagaacttcgactacttcgccccgaaaattaagcaggccatgcaggaaaaactggaagccatctatgaagatcgtaag

SEQ ID NO: 98 - protein, 621 aa, Artificial sequence
  Engineered sequence
MSNTSFSAKDTDLSALFIGDKAENGQLYKDLLGKLVDEHLGWRQNYMPQDPPMISAEHQTSPEFRGTVNNMKDVLDELSSRLRSQSVPWHNAGRYWGHMNSETLMPAILAYNYAMLWNGNNVAYESSPATSQMEEEVGLEFATLMGYTNGWGHIVADGSLANLEGLWYARNIKSLPFAMKAVDPTIVAGKTDWELSNMSTKEIMDLVEANGDKIDEIKAKSARGGKDLDKLGKWLVPQTKHYSWLKAADIIGIGLDQVIPVPVDSNYRMDINELEKIIRELASTETPILGVVGVVGSTEEGAVDGINEIAELRNKLVKEGIYFYFHIDAAYGGYGRAILLDEDNKLIPYKDLQSKFAEYNVFTEEENLVSEHTYNAYAAFPEAESVTIDPHKMGYIPYSAGGIAIQDIRMRDVISYFATYVFEKGADIPALLGAYILEGSKAGATAASVWAAHKTLPLNVTGYGKLVGASIEGARRFYNFLSGLEFKVGDKTIEVHPLTDPDFNMVDYVFQEKGNNNLVEMNELNHEFYNQASYVTGSIYGNEYLTSHTDFAIPDYGNSPFKFVNNLGVTEEGWKEAGKVTVLRAAVMTPYMNKAENFDYFAPKIKQAMQEKLEAIYEDRK

SEQ ID NO: 99 - DNA, 1863 bp, Artificial sequence
  Engineered sequence
atgagcaacaccagtttcagcgcaaaagataccgatctgagtgcactgtttatcggtgacaaagcagaaaatggtcagctgtataaggacctgctgggcaaactggttgatgaacatctgggttggcgccagaattatatgccgcaggatccgccgatgatcagcgccgaacagcagaccagcccggaatttcgtggtaccgtgaataatatgaaggacgttctggatgagctgagcagtcgcctgcgtagtcagagcgttccgtggcataatgccggtcgttattggggccacatgaatagcgaaaccctgatgccggcaattctggcctataattatgcaatgctgtggaatggtaacaacgtggcctatgaaagcagcccggcaaccagccagatggaagaagaagttggtctggaatttgccaccctgatgggctttaccaatggttggggccatattgttgcagatggtagcctggcaaatctggaaggcctgtggtatgcacgcaatattaagagcctgccgtttgccatgaaagccgttgatccgaccattgttgccggcaaaaccgattgggaactgagtaatatgagcaccaaagaaatcatggacctggttgaagccaatggtgacaaaattgatgagatcaaggccaaaagcgcccgcggcggtaaagatctggataaactgggtaaatggctggttccgcagaccaaacattatagttggctgaaagccgcagatattatcggcattggcctggatcaggttattccggttccggttgatagcaattatcgtatggatatcaacgagctggagaaaattatccgcgaactggcaagtaccgaaaccccgattctgggcgttgtgggcgttgtgggtagtaccgaagaaggtgccgttgatggcattaatgaaattgcagaactgcgtaacaagctggtgaaagaaggtatctatttctacttccacatcgacgccgcctatggtggctatggtcgcgcaattctgctggatgaagataataagctgatcccgtataaggaccttcagagtaaattcgccgaatataacgtgttcaccgaagaagaaaacctggtgagtgaacatacctataacgcctatgccgcatttccggaagccgaaagtgttaccattgatccgcataaaatgggctatatcccgtatagtgcaggcggcattgccattcaggatattcgcatgcgtgatgttatcagctatttcgcaacctatgtgttcgaaaagggcgcagatattccggcactgctgggtgcttatattctggaaggcagtaaagcaggcgcaaccgcagccagtgtttgggcagcacataaaaccctgccgctgaatgttaccggttatggtaaactggttggtgcaagcattgaaggcgcccgccgtttttataattttctgagcggcctggaattcaaggtgggcgataaaaccattgaagttcatccgctgaccgatccggattttaatatggttgattacgtgttccaggagaagggcaataataatctggtggaaatgaacgagctgaaccatgaattttacaaccaggcaagctacgttaccggtagcatctatggcaatgaatatctgaccagccataccgatttcgcaattccggattatggtaatagcccgtttaagtttgtgaacaacctgggcgtgaccgaagaaggctggaaagaagcaggtaaagtgaccgttctgcgcgccgctgtgatgacaccttatatgaataaggcagagaacttcgactacttcgccccgaaaattaagcaggccatgcaggaaaaactggaagccatctatgaagatcgtaag

SEQ ID NO: 100 - protein, 621 aa, Artificial sequence
  Engineered sequence
MSNTSFSAKDTDLSALFIGDKAENGQLYKDLLGKLVDEHLGWRQNYMPQDPPMISAEQQTSPEFRGTVNNMKDVLDELSSRLRSQSVPWHNAGRYWGHMNSETLMPAILAYNYAMLWNGNNVAYESSPATSQMEEEVGLEFATLMGFTNGWGHIVADGSLANLEGLWYARNIKSLPFAMKAVDPTIVAGKTDWELSNMSTKEIMDLVEANGDKIDEIKAKSARGGKDLDKLGKWLVPQTKHYSWLKAADIIGIGLDQVIPVPVDSNYRMDINELEKIIRELASTETPILGVVGVVGSTEEGAVDGINEIAELRNKLVKEGIYFYFHIDAAYGGYGRAILLDEDNKLIPYKDLQSKFAEYNVFTEEENLVSEHTYNAYAAFPEAESVTIDPHKMGYIPYSAGGIAIQDIRMRDVISYFATYVFEKGADIPALLGAYILEGSKAGATAASVWAAHKTLPLNVTGYGKLVGASIEGARRFYNFLSGLEFKVGDKTIEVHPLTDPDFNMVDYVFQEKGNNNLVEMNELNHEFYNQASYVTGSIYGNEYLTSHTDFAIPDYGNSPFKFVNNLGVTEEGWKEAGKVTVLRAAVMTPYMNKAENFDYFAPKIKQAMQEKLEAIYEDRK

SEQ ID NO: 101 - DNA, 1863 bp, Artificial sequence
  Engineered sequence
atgagcaacaccagtttcagcgcaaaagataccgatctgagtgcactgtttatcggtgacaaagcagaaaatggtcagctgtataaggacctgctgggcaaactggttgatgaacatctgggttggcgccagaattatatgccgcaggatccgccgatgatcagcgccgaacagcagaccagcccggaatttcgtggtaccgtgaataatatgaaggacgttctggatgagctgagcagtcgcctgcgtagtcagagcgttccgtggcataatgccggtcgttattggggccacatgaatagcgaaaccctgatgccggcaattctggcctataattatgcaatgctgtggaatggtaacaacgtggcctatgaaagcagcccggcaaccagccagatggaagaagaagttggtctggaatttgccaccctgatgggctataccaatggttggggccatattgttgcagatggtagcctggcaaatctggaaggcctgtggtatgcacgcaatattaagagcctgccgtttgccatgaaagccgttgatccgaccattgttgccggcaaaaccgattgggaactgagtaatatgagcaccaaagaaatcatggacctggttgaagccaatggtgacaaaattgatgagatcaaggccaaaagcgcccgcggcggtaaagatctggataaactgggtaaatggctggttccgcagaccaaacattatagttggctgaaagccgcagatattatcggcattggcctggatcaggttattccggttccggttgatagcaattatcgtatggatatcaacgagctggagaaaattatccgcgaactggcaagtaccgaaaccccgattctgggcgttgtgggcgttgtgggtagtaccgaagaaggtgccgttgatggcattaatgaaattgcagaactgcgtaacaagctggtgaaagaaggtatctatttctacttccacatcgacgccgcctatggtggctatggtcgcgcaattctgctggatgaagataataagctgatcccgtataaggaccttcagagtaaattcgccgaatataacgtgttcaccgaagaagaaaacctggtgagtgaacatacctataacgcctatgccgcatttccggaagccgaaagtgttaccattgatccgcataaaatgggctatatcccgtatagtgcaggcggcattgccattcaggatattcgcatgcgtgatgttatcagctatttcgcaacctatgtgttcgaaaagggcgcagatattccggcactgctgggtgcttatattctggaaggcagtaaagcaggcgcaaccgcagccagtgtttgggcagcacataaaaccctgccgctgaatgttaccggttatggtttgctggttggtgcaagcattgaaggcgcccgccgtttttataattttctgagcggcctggaattcaaggtgggcgataaaaccattgaagttcatccgctgaccgatccggattttaatatggttgattacgtgttccaggagaagggcaataataatctggtggaaatgaacgagctgaaccatgaattttacaaccaggcaagctacgttaccggtagcatctatggcaatgaatatctgaccagccataccgatttcgcaattccggattatggtaatagcccgtttaagtttgtgaacaacctgggcgtgaccgaagaaggctggaaagaagcaggtaaagtgaccgttctgcgcgccgctgtgatgacaccttatatgaataaggcagagaacttcgactacttcgccccgaaaattaagcaggccatgcaggaaaaactggaagccatctatgaagatcgtaag

SEQ ID NO: 102 - protein, 621 aa, Artificial sequence
  Engineered sequence
MSNTSFSAKDTDLSALFIGDKAENGQLYKDLLGKLVDEHLGWRQNYMPQDPPMISAEQQTSPEFRGTVNNMKDVLDELSSRLRSQSVPWHNAGRYWGHMNSETLMPAILAYNYAMLWNGNNVAYESSPATSQMEEEVGLEFATLMGYTNGWGHIVADGSLANLEGLWYARNIKSLPFAMKAVDPTIVAGKTDWELSNMSTKEIMDLVEANGDKIDEIKAKSARGGKDLDKLGKWLVPQTKHYSWLKAADIIGIGLDQVIPVPVDSNYRMDINELEKIIRELASTETPILGVVGVVGSTEEGAVDGINEIAELRNKLVKEGIYFYFHIDAAYGGYGRAILLDEDNKLIPYKDLQSKFAEYNVFTEEENLVSEHTYNAYAAFPEAESVTIDPHKMGYIPYSAGGIAIQDIRMRDVISYFATYVFEKGADIPALLGAYILEGSKAGATAASVWAAHKTLPLNVTGYGLLVGASIEGARRFYNFLSGLEFKVGDKTIEVHPLTDPDFNMVDYVFQEKGNNNLVEMNELNHEFYNQASYVTGSIYGNEYLTSHTDFAIPDYGNSPFKFVNNLGVTEEGWKEAGKVTVLRAAVMTPYMNKAENFDYFAPKIKQAMQEKLEAIYEDRK

SEQ ID NO: 103 - DNA, 1863 bp, Artificial sequence
  Engineered sequence
atgagcaacaccagtttcagcgcaaaagataccgatctgagtgcactgtttatcggtgacaaagcagaaaatggtcagctgtataaggacctgctgggcaaactggttgatgaacatctgggttggcgccagaattatatgccgcaggatccgccgatgatcagcgccgaacagcagaccagcccggaatttcgtggtaccgtgaataatatgaaggacgttctggatgagctgagcagtcgcctgcgtagtcagagcgttccgtggcataatgccggtcgttattggggccacatgaatagcgaaaccctgatgccggcaattctggcctataattatgcaatgctgtggaatggtaacaacgtggcctatgaaagcagcccggcaaccagccagatggaagaagaagttggtctggaatttgccaccctgatgggctataccaatggttggggccatattgttgcagatggtagcctggcaaatctggaaggcctgtggtatgcacgcaatattaagagcctgccgtttgccatgaaagccgttgatccgaccattgttgccggcaaaaccgattgggaactgagtaatatgagcaccaaagaaatcatggacctggttgaagccaatggtgacaaaattgatgagatcaaggccaaaagcgcccgcggcggtaaagatctggataaactgggtaaatggctggttccgcagaccaaacattatagttggctgaaagccgcagatattatcggcattggcctggatcaggttattccggttccggttgatagcaattatcgtatggatatcaacgagctggagaaaattatccgcgaactggcaagtaccgaaaccccgattctgggcgttgtgggcgttgtgggtagtaccgaagaaggtgccgttgatggcattaatgaaattgcagaactgcgtaacaagctggtgaaagaaggtatctatttctacttccacatcgacgccgcctatggtggctatggtcgcgcaattctgctggatgaagataataagctgatcccgtataaggaccttcagagtaaattcgccgaatataacgtgttcaccgaagaagaaaacctggtgagtgaacatacctataacgcctatgccgcatttccggaagccgaaagtgttaccattgatccgcataaaatgggctatatcccgtatagtgcaggcggcattgccattcaggatattcgcatgcgtgatgttatcagctatttcgcaacctatgtgttcgaaaagggcgcagatattccggcactgctgggtgcttatattctggaaggcagtaaagcaggcgcaaccgcagccagtgtttgggcagcacataaaaccctgccgctgaatgttaccggttatggtggtctggttggtgcaagcattgaaggcgcccgccgtttttataattttctgagcggcctggaattcaaggtgggcgataaaaccattgaagttcatccgctgaccgatccggattttaatatggttgattacgtgttccaggagaagggcaataataatctggtggaaatgaacgagctgaaccatgaattttacaaccaggcaagctacgttaccggtagcatctatggcaatgaatatctgaccagccataccgatttcgcaattccggattatggtaatagcccgtttaagtttgtgaacaacctgggcgtgaccgaagaaggctggaaagaagcaggtaaagtgaccgttctgcgcgccgctgtgatgacaccttatatgaataaggcagagaacttcgactacttcgccccgaaaattaagcaggccatgcaggaaaaactggaagccatctatgaagatcgtaag

SEQ ID NO: 104 - protein, 621 aa, Artificial sequence
  Engineered sequence
MSNTSFSAKDTDLSALFIGDKAENGQLYKDLLGKLVDEHLGWRQNYMPQDPPMISAEQQTSPEFRGTVNNMKDVLDELSSRLRSQSVPWHNAGRYWGHMNSETLMPAILAYNYAMLWNGNNVAYESSPATSQMEEEVGLEFATLMGYTNGWGHIVADGSLANLEGLWYARNIKSLPFAMKAVDPTIVAGKTDWELSNMSTKEIMDLVEANGDKIDEIKAKSARGGKDLDKLGKWLVPQTKHYSWLKAADIIGIGLDQVIPVPVDSNYRMDINELEKIIRELASTETPILGVVGVVGSTEEGAVDGINEIAELRNKLVKEGIYFYFHIDAAYGGYGRAILLDEDNKLIPYKDLQSKFAEYNVFTEEENLVSEHTYNAYAAFPEAESVTIDPHKMGYIPYSAGGIAIQDIRMRDVISYFATYVFEKGADIPALLGAYILEGSKAGATAASVWAAHKTLPLNVTGYGGLVGASIEGARRFYNFLSGLEFKVGDKTIEVHPLTDPDFNMVDYVFQEKGNNNLVEMNELNHEFYNQASYVTGSIYGNEYLTSHTDFAIPDYGNSPFKFVNNLGVTEEGWKEAGKVTVLRAAVMTPYMNKAENFDYFAPKIKQAMQEKLEAIYEDRK